European Patent Application EP 4 772 637 A1, published July 8, 2026. Title: RasGRP4のアンチセンスオリゴヌクレオチド. Applicant: 日産化学株式会社. The sequence listing filed with the application follows.

SEQUENCE LISTING (363 sequences)

SEQ ID NO: 1 - RNA, 3132 nt, Homo sapiens
  source 1..3132: mol_type = mRNA
ctctttccttcccaagcaccgaggaggccccagctccctaggggctgagaagctggagtcctgggcaaggggaggagctgagccctactcttgcaagacccccggcctcctcaccccacgcgggaagcatgaacagaaaagacagtaagaggaagtcccaccaggaatgcaccggaaaaataggagggcgaggccggccccgccaagtgcgccgccacaagacatgccccagccctcgggaaatcagcaaggtcatggcttccatgaacctgggcctgctgagtgagggcggctgcagcgaagatgagctgctggagaaatgcatccagtccttcgattcagctggcagcctgtgccacgaggaccacatgctcaacatggtgctggccatgcacagctgggtgctgccgtccgccgacctggctgcccgcctgctgacctcataccagaaggccacaggggacacccaggagctgagacggctgcagatctgtcacctggtcaggtactggctgatgcgacaccctgaggtgatgcaccaggatccccagctagaagaagtcataggtcgtttctgggccaccgtggcccgggagggcaactcagcccagagaagactgggagactcttctgacctcctgagccctggtggccctggccccccactcccaatgagcagcccaggcctgggcaaaaagcgcaaagtgtccttgcttttcgaccacttggagacgggggagctggctcagcacctcacctacctggagttccggtccttccaggctatcacgccccaggacctgcggagctacgttttgcagggctcagtacgaggctgcccggccctggagggctccgtaggtctcagcaacagcgtgtcccgctgggtgcaggtgatggtgctgagccgtcccgggcccctacagcgtgcacaggtgctggacaagttcattcacgtggcacagaggctccaccagctgcagaatttcaacacgctgatggcagtcacagggggcctgtgtcacagtgccatctccagactcaaggactcccatgcccacctgagccctgacagcaccaaggccctcctggagctcactgagctccttgcctcccacaacaactacgcccgctaccgccgcacctgggctggctgcgcgggtttccggctgcctgtactgggcgtgcacctcaaggacctggtgtccctgcatgaggcacagcccgacaggttgcctgacggccgcctgcacctacccaagctgaacaacctctacctgcggctgcaggagctggtggccctccaagggcagcatccaccctgcagcgccaatgaggatctgctgcacctgctcacgctctccctggacctcttctacacggaagacgagatctatgagctttcttatgcccgggagccgcgttgtcccaagagcctgccaccctcccccttcaatgcacctctggtggtggagtgggcccctggtgtgacacccaagccggacagggtcacactgggtcggcatgtggagcagctggtggagtctgtgttcaagaattatgaccctgaaggccgaggaacaatctctcaggaggactttgagcgactctcgggcaattttcccttcgcctgccatgggcttcacccacccccacgccaggggagaggatccttcagcagagaggagctgacagggtacctgctccgggccagcgccatctgctccaagttgggcctggccttcctgcacaccttccatgaggtcaccttccgaaagcctaccttctgcgacagctgcagtggcttcctctggggtgtcaccaagcaaggctaccgctgtcgggagtgcgggctgtgttgccacaaacactgcagagaccaggtgaaggtagaatgtaagaagaggccaggggccaagggcgatgcaggaccccccggagctcctgtcccatccacaccagctccccatgccagctgtggctccgaggaaaatcactcctacacgctatccctggagcctgagactgggtgccagcttcgccatgcctggacccagactgaatccccacacccttcctgggaaacagatacggtcccctgcccggtgatggacccaccatcaactgcatcctccaagctggattcctagacatctcttggtctcctctcttcctcactcccttcccccagtcagtcctgagtcctgccgtcagactctggcagggctcccagaggtaggcctccagaggcatccgccttcccatccacactgcctttagtggtacgtccgtcatctttttccctggaagtgactttcctcttttgcatcctggtggatgctaatcctgctccctttccctgcacttagtatctgtgcggctgtgtgttggatacatttagactcaggcctcattctaccaactccctacatctccatttctttttttttttgagacagagtcttgctctgtcacccaggctggagtgcaatgatgcaatctcagctcactgcaacttccgcctcctgggttcaagtgattcttctgcctcagcctcccaagtagctgggattacaggcacgcgccaccatgcccggctaatttttgtatttttagtagagacggggtttccccatgttggccaagatggtctcaaactcctgacctcatgatccaccagcctcagcctcccaaagtgctgggaatacaggcgtgagccaccacgcccagctcctgtttttctgcatagaatgtgctccctctgacagcctatactttttccctctttatctcgttgaacgtctgtctttcctcaacaggagcatcaactccaggagaacagggatttctatcaatgtcattcactgctgcatccccagtgcctagaacagggctggcaggtggtaggcgcctgacagatgcttgtctgatgcctgaatgtctccttacccatgcccacggcacaggatagatgtgctatagggcaaagaactttgagggtcgagcagcaggggcccattcagtcccagggagcagagacccccccaaccccttcacaaaccccaacacccctgacttggcccccacagagagaggtcctacagctgtcataaattaaatttattctctgga

SEQ ID NO: 2 - DNA, 18455 bp, Homo sapiens
  source 1..18455: mol_type = genomic DNA
ttttgtagagacggggttttgtcacgttgttcaagctggtctcaaactcttagactcaagcgatccgcctgccttggcctcccaaagtgctggatgacaggcgtgagcccctgtgagcccccgtgcctggtccggtatgtaattttttttaaggtaacagtggattgtgtgaggattaaatgagttaatatttttaaagtccttacagcagtgtgtggtacacagtaggtgctatgtggaggtttgttacaataaagtcagaaagtgaaaatgttttccagggtacaaatggtatcacttaaactaggaataagagacgcctatgaagaaatatacaaaatactatgtcttgtgagtttccattcaaaccttcatgaattatatatatgaatatgtccttctagacagacagacttatctttttgagtgagtgtgtgtgtttttacataaatatcagtcatgctttaaaaagaaaagccccttcttttattgaagtatgacagtgacgggtctcgacaccgaaagatgggggagatagagagcccgccggggagcttgagggtgggagagccagcgatgccggaaacctcagcagaagggatccccgtgtgggggaggggggccttcggtctctccccagcctcttccttccccctggcctgagggtgggtggggaggggcagttcctctttccttcccaagcaccgaggaggccccagctccctaggggctgagaagctggagtcctgggcaaggggaggagctgagccctactcttgcaagacccccggcctcctcaccccacgcgggaagcatgaacagaaaagacagtaagaggtgagaggaccctccccagggagcccggcagcaccctgaggcctccctctgcatgggagggctggggagatcactcgccagggtggcaggattcctgacttctttgggatcaggcgcaggggggccaggtggatgcttcagggagtctggagccagctacggctgcagtcgcttgtatgtggcatctgtaccgtgttgtccctggagtttgagctgctccgtgccccttttccactcctcatcaccccacctccatccctggcctgggctgagtgtctctgccctccctgggggcttcctggttccccatccccgtggactggaaactccaggctcctgcagggcctggcccaggagaggggagtgtggcacagggcaaggcgactcccctgcctcttaaaccactcctggctgttccagacccctacagggggctgcaggacagggcctagtggctggctgtgcggccggttctggaatgggcttcatctcctgggcaagctggcccttctgtccccacagaggcagatggtgggtggctccctagcctgggtaactcctcctgccacccccagcaccactctgatgggcaaagggctttcctccccacccagcagtttagtggtagactcctggctgcctaatttcctagctgtgtgaccttaggtaagtcacttaactgctctgtgtctcgggtttttcttctgtcagtagaacaatcatatcctctacctcggagaggcctgtaagtactcaatgagacactctagaccagtggttctcaaactggagcgagcctcagaactgtctggagggcttgtaaaatacaggttgctgggcttacctttaaagtgtttggtttttttttttttgttttttttttttgagacggagtctcgctctgccgccaggctggagtgcagtggcacaatcttggctcactgcaacctctgcctcccgggttcaagcgatcatcctgcctcagcctcccaagtagctgggactacaggtgtgcaccaccacacccagctacttttttgtatttttagtagagatggggtttcaccatgttgggcaggatggtctcgatctcttgacctcgtgatccacccacctcggcctcccaaagtgctgggattagaggcatgagccaccacccttagccttaaagtgtttgattttgtaggtctgggttgggacctgagaatctgtattgatatccagttcccaggtgatgcttttggtactagctgggtgcccacacttagggaaatgctgacttagttagaatgctccttccttagcctaggacatatataatactttaaaatgtcccttctagtaacgatggctcatgcctctaatcccagcactttgggaggataagacaaggagaacttgaagccaggagttctagaccagcctgagaaatatagtgagacccccccccccattgacacacacccaaacacacacacaaaattagctgggtatggtcgtgcacacctgtagtcccagctacctgggagactaaggcaggaggatcactcgagtccaggagttcaaggttacaatgagctttgattgcacaactgtgctccagcctgggagacagagcaagaccctgtctgaaaaagggtagaggtgggagcctggcgtgatggctcacacctgtaatcccagcactttcagaggcaaaggtgggaggatcagttgggcccaggagtttgaaaccagcctggccaacatggtgaaaccccatttctactaaaaatacaaaaattagctcggcgtggtggcacgtgcctgtagtcccaactacttgggaggctgaggcaggagaattgcttgaacccgggaggtggaggttgcagtgagctgagatcgcaccactgcactccagcctgggtgacagagtgagaccctgtctccaaaaaaagaaagaaagaaagaaaaaagaaatccctggagaaggtccaaggactatcctcatttttccttcgaggaaattgagccccagagaaattaagtgactaacacgaagtcacaacagctggcaaaaatttctggattctactttcgtctgaagcttggattcagcagcctccctgctcccaccatccttgtctctccattaccctcttcccctatcaggaacagcagcctctgggaggcaccaggcagagggagaattattattactattattactattattattattattattttgagactaagactcgctctgttgcccaggctggagtgcagtggcacgatctcggctcactgcaacctccgcctcctgggttcaagcaagtcttctgcctcagcctcctgagtagctgggattacaggagcccaccaccacgcctggctaatttttgtatttttaatagagatggggtttcaccatgttggccaggctggtctcgaactcctgacctcaagtgatccacccacctcagcctcccaaagtgctgggactacaggcgtgagccactgtgactggcctctctttttaatttttttattattatttttgaaacagaaatcactctgtcacccaggttggagcacagtgatgcagttccggctcactgcagcctccacctcctgggttcaagcgaccctcctgcctcagcctcctgagtagctgggattacaggcgcccgccatcacgcctgaccaatttttgcatttttagtagcgatgggggtttcaccatgttggccggggtggtctcgaactcctggcctcaagtgatccacccaccttggcctcccaaagctttgggattacaggcgtgagccatcacactggtccaagagccttgctctcttgagggctgtgggaggaaggaggggagggtgttagagaccaaacgggagccctgaggaggcaattcctgaaggcaggtcctcccatgcctctgcctggggaggacagaagagattccaggggtcttctcccgagtccctggtaggccaggagtaatcctgggatctgccaaaaggaagtctcttccaggatgccctggaagcagtcaagaggaagttgggggcaatgcctggggaaggagttcttatgattccctgaggggtcttgagtggtcccaggggtcttctactgtgattccctgggagattcagagcagtcctgagcggcggtccccaggctttttggcatcagggaccagttttgtggaagggggtggggatggtgtggggatgattcaagttaattacatgtatcctgtgctttatttttattattattacattgtaatatataatgaaatagttacgcagctcaccataatggagaatcagtgggagccctgagcttgttttcctgcaactggatgctcccatctgggggtgatgagagacagtgacagatcatcaggcattaggcatcaggcatcataaacagcacgcagcctagatcatcaggcatcataaacagcacgcagcctagatccctcgcatgtgaagttcacaatagggttcatgctcctaagagagtctaatgccccagctgatctgacaggaggtggagctcaggcgggggtgcttgcttgcccgctggttcctaacaggccacggactggtacctgtctgtgtcccaggggctggggacccctggtcttgaggatcttcctctctgattccctgaagggagcaggaatatccctgggagtttgcttgtgggagagggctcccatgattcccccagggatctggaatattcctggggattctctctagagtccctggtaggtcaggggtaaccctggggctttgcctttaggaagcctctcccgtggtgccttggggcattagagtcaaaaggaattctagggtctgtccgaaagaaggtgctcccatgactccttgggggctgtgcccacaggaagtcccaccaggaatgcaccggaaaaataggagggcgaggccggccccgccaagtgcgccgccacaagacatgccccagccctcgggaaatcagcaaggtcatggcttccatgaacctgggcctgctgagtgagggcggctgcagcgaagatgagctgctggagaaatgcatccagtccttcggtaagtgtcctctccccagcagcctccctggccctaacctcgggctcagcactcgcttctctccacctcagtttttggaggtaaaatgagaacagggctgggtggaatgaaactcaatcactacattagagataacagaaacacctgcatttcttctttcctgaaatggaaatatatacatttatatatatatataatatatgtgtatattatatatatttatataaatcttttttcttttcttttctttttcttttgagacagagtctcgctctgttacccaggctggagtgcagtggcctgatctcagctcactgcaacccccacctcctgggttcaagagattctcctgcctcagcttcccgagtagctaggattacaggcacatgccaccaggcccagctaatttttgtgtttttagtagaaacggtgtttcaccatgttggccagacttgtcccgaactcctggcctcatatgatccgcccgattcagcctcccaaagtgctgggattacaggtgtgagccactgtgcccggccagtctggtgctatttcaatcttcagcaagacttgccaggggtgatgctgccccatgcacaatacagataaggaaactgaggcacaggaggttaggttgcctgtccaaggtcatgctggggatcaccgttagagctggtctttgaaccaggtggtccggcaggatctggagctacgctctgcattgcttgagggccattctgtcacagagtacccctccttccaccccagattcagctggcagcctgtgccacgaggaccacatgctcaacatggtgctggccatgcacagctgggtgctgccgtccgccgacctggctgcccgcctgctgacctcatatcctccaggactgtgagctatgggtggagggcagagggcagagtcgtgagaacctgggcaatgggaatggggagcaggcaggtcatggatcctggaaaacagagccttgaccagaactcaaataccagaaggccacaggggacacccaggagctgagacggctgcagatctgtcacctggtcaggtagggctgggccgagatccccactctcaggacccacgacttccatcctgcttccccctcaaaaaacattcctcagagaatccccaggccagttcccacagacccaaccagccccacaggccaaaatcccacttctgagacacctgtagcttggttcctaagaccctcttagttccgttccttagaacccccacttcctagagacccccctcaccaaccagatcccatagaccctcctagctggtgcccagagacctccaactctgatccccaaaatctctacctcccacagaccccagcctagcccataagaccccctcattctgtccctccaaaaatttcacccccggaagcccccagtctagttcctaggacgctccacgatcttgcttcccaataatcccacttccaagtgactccccggtctgtttcccacagatccccccagtctctgttaagagacccccatcctactccagagattctccaagcctggtgcccctccaaaccccaaccctccagggacccccacacacatttagagaccccctagctcagcacctagaaattcctcagcccaaaataccccttgtagagaccttcgccacccccggcctcatctcaccatctccaaaccactctcaggtactggctgatgcgacaccctgaggtgatgcaccaggatccccagctagaagaagtcataggtcgtttctgggccaccgtggcccgggagggcaactcagcccagagaagactgggagactcttctgacctgtgagtcagccctgtgctcccctcttccctgccccatcgccattctgccatctccctctatatccccaagccctcaactgtgagccactccaataccctgcccctcttggcccccagcctgagccctggtggccctggccccccactcccaatgagcagcccaggcctgggcaaaaagcgcaaagtgtccttgcttttcgaccacttggagacgggggagctggctcagcacctcacctacctggagttccggtccttccaggctatcacggtgaggaccccctcccatccccgtcccaagcaggggagacactggggtaggggagggattggctgggggaaggtaggactgagaggacacctgcatggtcattcggcagagatctcaaagtcttaaactcaaacctgtatgctagaaggtccaggaaaatgagttaaagaggccaaggcaggcagatcgcctgaggtcaggagtttgagaccagcctggccaacatggtgaaaccccatctctactaaaaatacaaaaattatccaggtgtggtggtgcatgcctgtaatcccagctacttgggagggtgaggcaggagaatcacttgaacctcaggaggcggagattacagtgagctgagatcacaccactgcactccagcctgggcgacagagcgagattctgtctcgaaaaacaacaacaacaaaaaagtaaaataaataaataaaaggcttattgcagcgactggcacttagtaagtgctcaaaatattttatcatttattcaacaagcatttaaattcatggtgcctcagtttcctcatctgtaaaaaggggatatgcacagttcctgccttgcaggaacagtgcctggtccagggtaaatgctatctgcttgaaccatttgaaattgtcatatattacctacccaaggatcagtttcatgtgcttcaacatatatatgcattagcttttgccatctggacatcatcatttcaagggaaggtggggatctgtttccttcatgtgaaactgtcccgattgtatgtgtgtgttgtgtgtgtgagtgtgtatgcaaatatactcagtgtagtggatgtgggtatgaaatgaacactccttgggcagaacagatagaggttgatttcaattcatcttccccagccttccctttgcttactgtataccagtcaggtgtacagttaagagcatatagacgcccaccctgactcacacctgtgtgaccctgggcaaattacctatcctctatgtgcctcaactgtctcacctctaaaatggaatgatactcacctcatagagttatgaggattaaattatttaatatgattacttgtcaaatatagtgcctggctatattgaaacatgcctcctcagatgggagaggagcatggtgacgttaaggacatgtagcagcctgagggttgggggacagatgacaaaggtcactccggctagaccaggctaggacatcagagatcgtgactgctagttggatgccatggaagggcagggcctgagcgccacggcccaccttgacacccacctcgctcccagccccaggacctgcggagctacgttttgcagggctcagtacgaggctgcccggccctggagggctccgtaggtctcagcaacagcgtgtcccgctgggtgcaggtgatggtgctgagccgtcccgggcccctacagcgtgcacaggtgctggacaagttcattcacgtggcacaggtgaggcccgccccttggggctgcgaactccactgcacgcagccacctggtccttccccttccagaccctcgaccccacagggtcatcccggcggtgacgtcacgcatctcccggccccgcccccgaggccacagcctgggcattccaaccaaggaccgtaacttcttctttggccttgatgtcaccgcgtcgcacccaccgtggccccaccccttggccctagacgtgacaggctcccaagccctatgcccgaatattctatccccaggtcaatgagagtgtctcttccatgcccccacctttgtggggcatggaagcccgaggcttcaatccccagtccccaggccccagcggtcgcttcgggattgtgcatcgctccccattgcgtccgggctctccccgccccgccccattgtgttacgcccttctcttcccctcccttccccctcctttccggacaccttctcgcccttctggggaaaagggaagccctacggccccgctgtggccgcgcccccttgcgtatttccacgcagaccacgcccttcctctggtgtcttccctggcttgcttactcctgcagggcccctgagacctgggggtctcgacgtccgcctggggtgtccttagtctgagcattttccattcctccctggccccactctctccacagcaacctctgccgaaatttgtcaaaaggagggcaagggaattccccagctgccctggtggccccacacctgtctagcatctgtctgactcctccatatctctctggccctattcacctctgcctggctcccagctcctgcccagagcctgcaccttcttgcctccccgcacctgtgtgactctcagagcagtcagacccccagatggctgacaccctgacatgtctgaagcctcctccacctgacacacacctgtctattccccaaatccgcccaacttctcgtacttcctgtctccccagattttctaacctcgtatcagtcaatcacttgcttgaccctcccggctcagatagccatctgacacccctgtgaggcccacacatggcatgtcccactcttgccgcacacacccgccttctctcacctgtctgatccccacattggtccacacatgcctgggaccccacctcaactgggatgctgtcatctgaactcctgacttgccctccctcccgtgacggccctgtgtgcatgcttctcttcctagaggctccaccagctgcagaatttcaacacgctgatggcagtcacagggggcctgtgtcacagtgccatctccagactcaaggactcccatgcccacctgagccctgacagcaccaaggtgaatcccactaccctccccaaagctccaagtggtcagctgtcttgagcccccacacctaattccccaagccctgtccattcctgcccaggggtcctggtaccacatgaagtccttgctcctccaaatcccagacccccaggctctgccagcattcctcctccctgtcatccatccactcatggtgctgatccctctctgctttcagtgtgtctggtccggagctggactgtgagggagacagatgggagacaggctagcagagaactttgcagtccccatggggaggactggctgaggtcagaaagtggcaggaaattaagccgaagatgccctgggaagatcctatagcgccttgtaagatgggctaagctagggaagttttgagagtgatgacacacccttgataaaatctgggtttttaagaaataattataggctgggtacagtgtggctcacacttgtaatcccagcgttttgggaggccaagattggaggatcactttagcccaggtgtttcagaccagcctgggcaacatagcgagaccccatctccagaaatttttttttttttttttttttttttttgagacagagtctcgctcttgtcgcccaggctggagtgcagtggtgcaatctcggctcactgcaacctctgcctcccggattcaggtaattctcctgccccagcctcccgaatagctgggattacaggggtgcaccaccatgccctgctaattttgtatttttagtagagacagggttttaccatgttggccaggctggtctcaaactcctgacctaaggcgatccacccaccttggcctccaaaagtgctgggattacaggtgtgagcctccgcgcctggctgaaaaaaaatttaaaaataaattagccagggatggtggcccatgcctgtagtcccagctacttgggaggctgagggggaggactgctggagcctccccctcagccttttcattgttgttttttgagacagagtctcactctatctcccaggctggagtacagtgtcgaaatcttggctcactgaagcctccacctcccaggttcaagcgattcgcctgcctcagactcccgagtagctgggattacaggcctgcaccaccagacccagttaatttttgtatttttagtagagacaggtttttaccatgttgcccaggctgttctcgaactcctgacctcagatgatccgcctgcctcggcctctcaaaatgctgggattacaggtgtgagccaccgtgcccagccatcaagctcaggagtttaaggctgcaatgagctgtgatcatgacactgtactccagcctgggtgacagagtgagaccctagcctaaaaaataaataaataaaaaggccggtcttgatggctaacgcctgtaatcccaacactttgggaggccgaggcaggcagatcacctgaggtgaggagtttgagaccagcctggccaacatggtaaaaccctgtctctactaaaaatacaaaattagcctggcgtggtggctcaatgcctgtaatcccagcttcttgggaggctgaggcaggagaatcgcttgaacccaggaggtggaggtggcagtaagccgagatcacgccactgcactctagcctgggcaagacagcaaaactccatctcaaaaaaaaaaaaaaaaaaatcaaaaagaaagaaagataaaagaaatcattttagccaaagaatgggggattgtggaacttctctgagatggggacccaagaggaagagcagtttgggggagatgctgagaccggcatgggatatggaagggctccagaggtttccacaatgccactgggtccctgaaggcctagagcccacacaggaggctgctcaggggatgggactgtcctgataacgccccaatcccatgtccctcctccccaggccctcctggagctcactgagctccttgcctcccacaacaactacgcccgctaccgccgcacctgggctggctgcgcgggtttccggctgcctgtactgggcgtgcacctcaaggacctggtgtccctgcatgaggcacagcccgacaggttgcctgacggccgcctgcacctacccaagctgaacaacctctacctgcggctgcaggagctggtggccctccaagggcagcatccaccctgcagcgccaatgaggatctgctgcacctgctcacggtgagcccccctggccccgcccaggctgggcttccaagggtactgagatatagggtcctgggtgtgtgagtgtctccaggaccaggatagaaaagtgctggagtgcatgggttttgaagccagaacttctaggtttttttctagctgcgtgatcttgggcaagtcactgaacccttaagcctcagtttccttatccacaaaatgggaataataaaaggacccagccgggcgcagtggctcacgcctgtgatcccaacactttgggacgctgaggtgggcagatcacctgaggtcaggagttcgagaccagcctgaccaacatggagaaaccccgtctctactaaaaatacaaaattagccaggagtggtggtgcgtgcctgtaatcccagctacttgggaggctgaggcaggagaattgcttgaacccgggaggtggaggttgcagtgagctgagattgcgccattgcgccattgcaccccagcctgggcaagaagagcgaaactccttctcaaaataaataaataaataaaaataaaataaaataaaaggacccacttcagagggtggttgaggagagacagccaatgacatcgttcaaagaatgtctttaagacagtgtctagccgggcgcagtggctcatgcctctaatcctagcactttgggaggctgaggtaggcggattgcctgaggagtttgagaccagcctaggcaacatggtgaaaccccatctctactaaaaatacaaaaaattagcctggcatagtggcacacgcctgtaatcccagctacttgggaggctgaggcatgagaatcgcttgaacctgggaggcggaggttgcagtgagccaagatcgtaccactacactccagcctgggtgacagagcaagactctgtctcaaaaaacgacagtatatggagcagagtgagctctgtattctatttaagtaacatgttttttccccacttcctccaatgactcaagtatccattgatctgagctctggaattgctttggggttcacattcttaaactccaaggttctgagcttctcatgctgatagcccaaaatctcaagctttgacatatccaagaatctaagcaaaaggctactaacagttattgatcattgactgtgtgccaggtacctcattccaccttacaaccctatgaggtcgggacccttactgtgcccattctgtagattgggaaactgaggcccagagaggtgaggtcccttgcccactgtcccacagcagtaatgccaggatttgaacccaggaggggctttgggaagagcctgcgagtgggtgtgggggtctggggcagggctatagatgggaggatccgtaacacccctgtctgctccagctctccctggacctcttctacacggaagacgagatctatgagctttcttatgcccgggagccgcgttgtcccaagagcctggtgagacccaacccctggcctcggactcccccaattacctcgaaccccccctaagcctatgcagtgactaactgtgctcctctgtccccgccccagccaccctcccccttcaatgcacctctggtggtggagtgggcccctggtgtgacacccaagccggacagggtcacactgggtcggcatgtggagcagctggtggaggtaaggaggggagggtggcccggccgccagcagccaggagggaagacatctgtagaaccctgagcctggaggtggggacttatggccatggggatcatatttcgacaactgggccttatctgcttccccacactcctctgaagtctgtgttcaagaattatgaccctgaaggccgaggaacaatctctcaggaggactttgagcgactctcgggcaattttcccttcgcctgccatgggcttcacccacccccacgccaggggtaagtggttgtgactcctggatcctccgaagatgaggacactggggttgcctggactcctgggtctggaggacgttggggcaggtcatgctgaggctcagtttctgcccccaggagaggatccttcagcagagaggagctgacagggtacctgctccgggccagcgccatctgctccaagttgggcctggccttcctgcacaccttccatgaggtcaccttccgaaagcctaccttctgcgacagctgcagtggcttcgtgagcaccccaccccatcaccacccttaggttccatctgtcctgaagccggcagtccgcaaaccccagataacccccaaattccagaaatcctccagcttcaaatcatcctgtttcatataaaccctaaacaccagacattccctatatcctggataatctccaaatgccagataatcccaaaatcccagataatgtccaccccagacaattgctgaaccatggataatacctaaaactctagataggaggccaggagtggtggctcacgcctgtaatcccagcacttggggaggctgaggtgggcggattgcttgagctcaagagttcaagaccagcctagggaacatagcaagagagaccccgtctctactaaaaatacaaaaattagctgcatgtggtggtgcatacctgtgatcccagctactcaggaggctgaggcacgagaattgcttgaacccaggaggtggaggttgcatgagccaagatcgcagcactgcactccagcttgggtgacagagcgagattctgtctcaaaaacaacaacaacaacaacaacaacaacaacaacaacaacaacaacaacaaacctggataatctccaaaccgggtagattatgttcaaacagaatcatcctccaaatctctagactccagatcattcaaactctgaataacttccaaattcaagagatcctcaaactctggctagtggatcaatctctcaacctataacccgagactaattcacaaaccttggattacttcccacattcatttattcattcatgaaatatttactgagcacctcctgtgtgccaggtaatcctaggccctggggttacagcaggaatacagcagacaactcttgcccatagaatttgcattttagtaactctaaattttacctaaatctaatatctgaggtgattatctaaacttgagataatctccaagtttcctttatttattttgttaagagatgggtcttgctctattacccaggctggagtgccgtggtacgatcatggttcattgcagcctccaatcctgagctcaagcgatcctcccaccttggcctcccaacctcccaccttggcgtctcaaagtgctgggattactggcatgagccactgtaccccacccacattcctttaattccagttaaatctctagccttgagaatttcaaaacctgggtagcttccacacttccactccccagctgccctgccaatccacagccctccctctcctaggatgggtaaccttttctcctttctcttcccagctctggggtgtcaccaagcaaggctaccgctgtcggggtgagtggggtgtcagtgagtgggagggaagccttggcccgcaggctggaagaatggatgacacagatcggacccctgccgctgccttcccccagagtgcgggctgtgttgccacaaacactgcagagaccaggtgaaggtagaatgtaagaagaggccaggggccaagggcgatgcaggaccccccggagctcctgtcccatccacaccagctccccatgccagctgtggtaagacctagagcacaccggtgctgggaaggggcctgggggaaaggggttgagtccaaggtcaagaagaggtccttcccatcagacccacatcccttccatccacccacaaacaggctccgaggaaaatcactcctacacgctatccctggagcctgagactgggtgccagcttcgccatgcctggacccagactgaatccccacacccttcctgggaaacagatacggtgaggagaaaccgcccctacccccaagtggatacaggggacacaggccattggcgtggggaagactggacagatttggagacccatagaaagtacaaatatgcagaagtccttgactgctggggtaggagggtatggatactggttactttttaatattgatagaaaaataggctgggtgtggtggctcatgcttgtaatcccaggacttcggggaggctgaggtgggaggatcacttgaggtcagaagttcgagatcagcctggccaacgtgataaaaccctatctctactaaaaatacaaaaattagccaagtgtgatggcgggtgcctgtagtcccagctacacgggaggctgaggcaggagaatcacttgagcccgggaggcagaggctgtagtgagctgagattgtgccactgcacaccagcctaggtgacagagcaagaccctgtctcaaaaaaaaaaaaaaaagaaaaatagaagtttcaacatgttgggggtagggtggggacaataaccactaggagaacagaaaaaaggattctagccaataagatagcaagaataaggccaaatatatcaggagctactgtacgggttaatggagtaaacgccactatttgagggcagagactctcagattgggttacaaaaaggattccacaggggacgttcattcatccacttaccagtctgggcagggaagtgttcctggcagtgaagcgtctcctagacatcatatgctccccacatcatctgtcatctttcttcctcccttcctccttccaggtcccctgcccggtgatggacccaccatcaactgcatcctccaagctggattcctagacatctcttggtctcctctcttcctcactcccttcccccagtcagtcctgagtcctgccgtcagactctggcagggctcccagaggtaggcctccagaggcatccgccttcccatccacactgcctttagtggtacgtccgtcatctttttccctggaagtgactttcctcttttgcatcctggtggatgctaatcctgctccctttccctgcacttagtatctgtgcggctgtgtgttggatacatttagactcaggcctcattctaccaactccctacatctccatttctttttttttttgagacagagtcttgctctgtcacccaggctggagtgcaatgatgcaatctcagctcactgcaacttccgcctcctgggttcaagtgattcttctgcctcagcctcccaagtagctgggattacaggcacgcgccaccatgcccggctaatttttgtatttttagtagagacggggtttccccatgttggccaagatggtctcaaactcctgacctcatgatccaccagcctcagcctcccaaagtgctgggaatacaggcgtgagccaccacgcccagctcctgtttttctgcatagaatgtgctccctctgacagcctatactttttccctctttatctcgttgaacgtctgtctttcctcaacaggagcatcaactccaggagaacagggatttctatcaatgtcattcactgctgcatccccagtgcctagaacagggctggcaggtggtaggcgcctgacagatgcttgtctgatgcctgaatgtctccttacccatgcccacggcacaggatagatgtgctatagggcaaagaactttgagggtcgagcagcaggggcccattcagtcccagggagcagagacccccccaaccccttcacaaaccccaacacccctgacttggcccccacagagagaggtcctacagctgtcataaattaaatttattctctggagaacatggttcttggtattgacgtgaatgggagcagggcatttggggactcaggaataggagatggggggcttgggtgccaaataccaaggaaagccttaaacggactccccagagattaccgatagcattagcatctcatggaggaccccccgcccccgaccaccagtccccctttacttcttcttcttcttcttgcgaccccaacactgggggcctccatcctctcttcggctcctccaggtgggcatgggaggctccagctcatttgggcggcccccccggtctggaacgttgcccataagcacctgagagtttatgagatttgagttgcagagaaaaaaagtatcttggacaagggggccagagagcgaagggaacagcatgaggctgaagaagaaacagcagatgttgactatttgagtacagtggctgggggaggggggactgaactggtggaagatactagcatgagctttcttttttcttttcttttttttgagacggagtctcactctgttgcccaggctggagtgcagtggtgtgatctcagctcactgcaacctccacctaccgggttcaagagattctcctgcctcagcctccca

SEQ ID NO: 3 - DNA, 16 bp, synthetic construct
  source 1..16: mol_type = other DNA
tggggcatgtcttgtg

SEQ ID NO: 4 - DNA, 16 bp, synthetic construct
  source 1..16: mol_type = other DNA
ccttgctgatttcccg

SEQ ID NO: 5 - DNA, 16 bp, synthetic construct
  source 1..16: mol_type = other DNA
tcagccagtacctgac

SEQ ID NO: 6 - DNA, 16 bp, synthetic construct
  source 1..16: mol_type = other DNA
ctttttgcccaggcct

SEQ ID NO: 7 - DNA, 16 bp, synthetic construct
  source 1..16: mol_type = other DNA
actccaggtaggtgag

SEQ ID NO: 8 - DNA, 16 bp, synthetic construct
  source 1..16: mol_type = other DNA
tgatagcctggaagga

SEQ ID NO: 9 - DNA, 16 bp, synthetic construct
  source 1..16: mol_type = other DNA
tcagcaccatcacctg

SEQ ID NO: 10 - DNA, 16 bp, synthetic construct
  source 1..16: mol_type = other DNA
gaatgaacttgtccag

SEQ ID NO: 11 - DNA, 16 bp, synthetic construct
  source 1..16: mol_type = other DNA
gaaattctgcagctgg

SEQ ID NO: 12 - DNA, 16 bp, synthetic construct
  source 1..16: mol_type = other DNA
gtgttgaaattctgca

SEQ ID NO: 13 - DNA, 16 bp, synthetic construct
  source 1..16: mol_type = other DNA
tccttgagtctggaga

SEQ ID NO: 14 - DNA, 16 bp, synthetic construct
  source 1..16: mol_type = other DNA
gggagtccttgagtct

SEQ ID NO: 15 - DNA, 16 bp, synthetic construct
  source 1..16: mol_type = other DNA
gcgtagttgttgtggg

SEQ ID NO: 16 - DNA, 16 bp, synthetic construct
  source 1..16: mol_type = other DNA
aggtccttgaggtgca

SEQ ID NO: 17 - DNA, 16 bp, synthetic construct
  source 1..16: mol_type = other DNA
ttcagcttgggtaggt

SEQ ID NO: 18 - DNA, 16 bp, synthetic construct
  source 1..16: mol_type = other DNA
gcagcagatcctcatt

SEQ ID NO: 19 - DNA, 16 bp, synthetic construct
  source 1..16: mol_type = other DNA
tgtagaagaggtccag

SEQ ID NO: 20 - DNA, 16 bp, synthetic construct
  source 1..16: mol_type = other DNA
tccgtgtagaagaggt

SEQ ID NO: 21 - DNA, 16 bp, synthetic construct
  source 1..16: mol_type = other DNA
ccgggcataagaaagc

SEQ ID NO: 22 - DNA, 16 bp, synthetic construct
  source 1..16: mol_type = other DNA
gtgcattgaaggggga

SEQ ID NO: 23 - DNA, 16 bp, synthetic construct
  source 1..16: mol_type = other DNA
accagctgctccacat

SEQ ID NO: 24 - DNA, 16 bp, synthetic construct
  source 1..16: mol_type = other DNA
gaacacagactccacc

SEQ ID NO: 25 - DNA, 16 bp, synthetic construct
  source 1..16: mol_type = other DNA
cgctcaaagtcctcct

SEQ ID NO: 26 - DNA, 16 bp, synthetic construct
  source 1..16: mol_type = other DNA
ctctgctgaaggatcc

SEQ ID NO: 27 - DNA, 16 bp, synthetic construct
  source 1..16: mol_type = other DNA
ccaacttggagcagat

SEQ ID NO: 28 - DNA, 16 bp, synthetic construct
  source 1..16: mol_type = other DNA
ttcggaaggtgacctc

SEQ ID NO: 29 - DNA, 16 bp, synthetic construct
  source 1..16: mol_type = other DNA
agccttgcttggtgac

SEQ ID NO: 30 - DNA, 16 bp, synthetic construct
  source 1..16: mol_type = other DNA
ggcctcttcttacatt

SEQ ID NO: 31 - DNA, 16 bp, synthetic construct
  source 1..16: mol_type = other DNA
ggattcagtctgggtc

SEQ ID NO: 32 - DNA, 16 bp, synthetic construct
  source 1..16: mol_type = other DNA
gggggaaggaagaggc

SEQ ID NO: 33 - DNA, 16 bp, synthetic construct
  source 1..16: mol_type = other DNA
ggaaagaggaactgcc

SEQ ID NO: 34 - DNA, 16 bp, synthetic construct
  source 1..16: mol_type = other DNA
ctccctgaagcatcca

SEQ ID NO: 35 - DNA, 16 bp, synthetic construct
  source 1..16: mol_type = other DNA
agctcaaactccaggg

SEQ ID NO: 36 - DNA, 16 bp, synthetic construct
  source 1..16: mol_type = other DNA
aggagtggtttaagag

SEQ ID NO: 37 - DNA, 16 bp, synthetic construct
  source 1..16: mol_type = other DNA
agtgacttacctaagg

SEQ ID NO: 38 - DNA, 16 bp, synthetic construct
  source 1..16: mol_type = other DNA
gccatgaccttgctga

SEQ ID NO: 39 - DNA, 16 bp, synthetic construct
  source 1..16: mol_type = other DNA
catgaccttggacagg

SEQ ID NO: 40 - DNA, 16 bp, synthetic construct
  source 1..16: mol_type = other DNA
ggatatgaggtcagca

SEQ ID NO: 41 - DNA, 16 bp, synthetic construct
  source 1..16: mol_type = other DNA
gagttctggtcaaggc

SEQ ID NO: 42 - DNA, 16 bp, synthetic construct
  source 1..16: mol_type = other DNA
ttggaagtgggattat

SEQ ID NO: 43 - DNA, 16 bp, synthetic construct
  source 1..16: mol_type = other DNA
gtgctgagctaggggg

SEQ ID NO: 44 - DNA, 16 bp, synthetic construct
  source 1..16: mol_type = other DNA
tcagccagtacctgag

SEQ ID NO: 45 - DNA, 16 bp, synthetic construct
  source 1..16: mol_type = other DNA
ggctgactcacaggtc

SEQ ID NO: 46 - DNA, 16 bp, synthetic construct
  source 1..16: mol_type = other DNA
ggctgctcattgggag

SEQ ID NO: 47 - DNA, 16 bp, synthetic construct
  source 1..16: mol_type = other DNA
accgtgatagcctgga

SEQ ID NO: 48 - DNA, 16 bp, synthetic construct
  source 1..16: mol_type = other DNA
tggcctctttaactca

SEQ ID NO: 49 - DNA, 16 bp, synthetic construct
  source 1..16: mol_type = other DNA
agcaccatcacctgca

SEQ ID NO: 50 - DNA, 16 bp, synthetic construct
  source 1..16: mol_type = other DNA
ctctgagagtcacaca

SEQ ID NO: 51 - DNA, 16 bp, synthetic construct
  source 1..16: mol_type = other DNA
ttggggaatagacagg

SEQ ID NO: 52 - DNA, 16 bp, synthetic construct
  source 1..16: mol_type = other DNA
aggcatgtgtggacca

SEQ ID NO: 53 - DNA, 16 bp, synthetic construct
  source 1..16: mol_type = other DNA
agctggtggagcctct

SEQ ID NO: 54 - DNA, 16 bp, synthetic construct
  source 1..16: mol_type = other DNA
ctgcagctggtggagc

SEQ ID NO: 55 - DNA, 16 bp, synthetic construct
  source 1..16: mol_type = other DNA
tctgcagctggtggag

SEQ ID NO: 56 - DNA, 16 bp, synthetic construct
  source 1..16: mol_type = other DNA
ttctgcagctggtgga

SEQ ID NO: 57 - DNA, 16 bp, synthetic construct
  source 1..16: mol_type = other DNA
attctgcagctggtgg

SEQ ID NO: 58 - DNA, 16 bp, synthetic construct
  source 1..16: mol_type = other DNA
aattctgcagctggtg

SEQ ID NO: 59 - DNA, 16 bp, synthetic construct
  source 1..16: mol_type = other DNA
ttgaaattctgcagct

SEQ ID NO: 60 - DNA, 16 bp, synthetic construct
  source 1..16: mol_type = other DNA
gttgaaattctgcagc

SEQ ID NO: 61 - DNA, 16 bp, synthetic construct
  source 1..16: mol_type = other DNA
tgttgaaattctgcag

SEQ ID NO: 62 - DNA, 16 bp, synthetic construct
  source 1..16: mol_type = other DNA
cgtgttgaaattctgc

SEQ ID NO: 63 - DNA, 16 bp, synthetic construct
  source 1..16: mol_type = other DNA
gcgtgttgaaattctg

SEQ ID NO: 64 - DNA, 16 bp, synthetic construct
  source 1..16: mol_type = other DNA
agcgtgttgaaattct

SEQ ID NO: 65 - DNA, 16 bp, synthetic construct
  source 1..16: mol_type = other DNA
gagtccttgagtctgg

SEQ ID NO: 66 - DNA, 16 bp, synthetic construct
  source 1..16: mol_type = other DNA
ggagtccttgagtctg

SEQ ID NO: 67 - DNA, 16 bp, synthetic construct
  source 1..16: mol_type = other DNA
tgggagtccttgagtc

SEQ ID NO: 68 - DNA, 16 bp, synthetic construct
  source 1..16: mol_type = other DNA
atgggagtccttgagt

SEQ ID NO: 69 - DNA, 16 bp, synthetic construct
  source 1..16: mol_type = other DNA
catgggagtccttgag

SEQ ID NO: 70 - DNA, 16 bp, synthetic construct
  source 1..16: mol_type = other DNA
ttggagctttggggag

SEQ ID NO: 71 - DNA, 16 bp, synthetic construct
  source 1..16: mol_type = other DNA
tgggtaggtgcaggcg

SEQ ID NO: 72 - DNA, 16 bp, synthetic construct
  source 1..16: mol_type = other DNA
ttgggtaggtgcaggc

SEQ ID NO: 73 - DNA, 16 bp, synthetic construct
  source 1..16: mol_type = other DNA
cttgggtaggtgcagg

SEQ ID NO: 74 - DNA, 16 bp, synthetic construct
  source 1..16: mol_type = other DNA
gcttgggtaggtgcag

SEQ ID NO: 75 - DNA, 16 bp, synthetic construct
  source 1..16: mol_type = other DNA
agcttgggtaggtgca

SEQ ID NO: 76 - DNA, 16 bp, synthetic construct
  source 1..16: mol_type = other DNA
cagcttgggtaggtgc

SEQ ID NO: 77 - DNA, 16 bp, synthetic construct
  source 1..16: mol_type = other DNA
tcagcttgggtaggtg

SEQ ID NO: 78 - DNA, 16 bp, synthetic construct
  source 1..16: mol_type = other DNA
gttcagcttgggtagg

SEQ ID NO: 79 - DNA, 16 bp, synthetic construct
  source 1..16: mol_type = other DNA
ccgtgtagaagaggtc

SEQ ID NO: 80 - DNA, 16 bp, synthetic construct
  source 1..16: mol_type = other DNA
cataagaaagctcata

SEQ ID NO: 81 - DNA, 16 bp, synthetic construct
  source 1..16: mol_type = other DNA
gcataagaaagctcat

SEQ ID NO: 82 - DNA, 16 bp, synthetic construct
  source 1..16: mol_type = other DNA
ggcataagaaagctca

SEQ ID NO: 83 - DNA, 16 bp, synthetic construct
  source 1..16: mol_type = other DNA
gggcataagaaagctc

SEQ ID NO: 84 - DNA, 16 bp, synthetic construct
  source 1..16: mol_type = other DNA
cgggcataagaaagct

SEQ ID NO: 85 - DNA, 16 bp, synthetic construct
  source 1..16: mol_type = other DNA
cccgggcataagaaag

SEQ ID NO: 86 - DNA, 16 bp, synthetic construct
  source 1..16: mol_type = other DNA
cagctgctccacatgc

SEQ ID NO: 87 - DNA, 16 bp, synthetic construct
  source 1..16: mol_type = other DNA
caccagctgctccaca

SEQ ID NO: 88 - DNA, 16 bp, synthetic construct
  source 1..16: mol_type = other DNA
ccaccagctgctccac

SEQ ID NO: 89 - DNA, 16 bp, synthetic construct
  source 1..16: mol_type = other DNA
tccaccagctgctcca

SEQ ID NO: 90 - DNA, 16 bp, synthetic construct
  source 1..16: mol_type = other DNA
gaacacagacttcaga

SEQ ID NO: 91 - DNA, 16 bp, synthetic construct
  source 1..16: mol_type = other DNA
aaagtcctcctgagag

SEQ ID NO: 92 - DNA, 16 bp, synthetic construct
  source 1..16: mol_type = other DNA
caaagtcctcctgaga

SEQ ID NO: 93 - DNA, 16 bp, synthetic construct
  source 1..16: mol_type = other DNA
tcaaagtcctcctgag

SEQ ID NO: 94 - DNA, 16 bp, synthetic construct
  source 1..16: mol_type = other DNA
ctcaaagtcctcctga

SEQ ID NO: 95 - DNA, 16 bp, synthetic construct
  source 1..16: mol_type = other DNA
gctcaaagtcctcctg

SEQ ID NO: 96 - DNA, 16 bp, synthetic construct
  source 1..16: mol_type = other DNA
tcgctcaaagtcctcc

SEQ ID NO: 97 - DNA, 16 bp, synthetic construct
  source 1..16: mol_type = other DNA
gtcgctcaaagtcctc

SEQ ID NO: 98 - DNA, 16 bp, synthetic construct
  source 1..16: mol_type = other DNA
ctctctgctgaaggat

SEQ ID NO: 99 - DNA, 16 bp, synthetic construct
  source 1..16: mol_type = other DNA
tggaaggtgtgcagga

SEQ ID NO: 100 - DNA, 16 bp, synthetic construct
  source 1..16: mol_type = other DNA
gtgacctcatggaagg

SEQ ID NO: 101 - DNA, 16 bp, synthetic construct
  source 1..16: mol_type = other DNA
ggtgacctcatggaag

SEQ ID NO: 102 - DNA, 16 bp, synthetic construct
  source 1..16: mol_type = other DNA
aaggtgacctcatgga

SEQ ID NO: 103 - DNA, 16 bp, synthetic construct
  source 1..16: mol_type = other DNA
gaaggtgacctcatgg

SEQ ID NO: 104 - DNA, 16 bp, synthetic construct
  source 1..16: mol_type = other DNA
ggaaggtgacctcatg

SEQ ID NO: 105 - DNA, 16 bp, synthetic construct
  source 1..16: mol_type = other DNA
cggaaggtgacctcat

SEQ ID NO: 106 - DNA, 16 bp, synthetic construct
  source 1..16: mol_type = other DNA
tcggaaggtgacctca

SEQ ID NO: 107 - DNA, 16 bp, synthetic construct
  source 1..16: mol_type = other DNA
tagagatttggaggat

SEQ ID NO: 108 - DNA, 16 bp, synthetic construct
  source 1..16: mol_type = other DNA
tgcttggtgacacccc

SEQ ID NO: 109 - DNA, 16 bp, synthetic construct
  source 1..16: mol_type = other DNA
ttgcttggtgacaccc

SEQ ID NO: 110 - DNA, 16 bp, synthetic construct
  source 1..16: mol_type = other DNA
cttgcttggtgacacc

SEQ ID NO: 111 - DNA, 16 bp, synthetic construct
  source 1..16: mol_type = other DNA
ccttgcttggtgacac

SEQ ID NO: 112 - DNA, 16 bp, synthetic construct
  source 1..16: mol_type = other DNA
gccttgcttggtgaca

SEQ ID NO: 113 - DNA, 16 bp, synthetic construct
  source 1..16: mol_type = other DNA
tagccttgcttggtga

SEQ ID NO: 114 - DNA, 16 bp, synthetic construct
  source 1..16: mol_type = other DNA
gtagccttgcttggtg

SEQ ID NO: 115 - DNA, 16 bp, synthetic construct
  source 1..16: mol_type = other DNA
ggtagccttgcttggt

SEQ ID NO: 116 - DNA, 16 bp, synthetic construct
  source 1..16: mol_type = other DNA
cggtagccttgcttgg

SEQ ID NO: 117 - DNA, 16 bp, synthetic construct
  source 1..16: mol_type = other DNA
gcggtagccttgcttg

SEQ ID NO: 118 - DNA, 16 bp, synthetic construct
  source 1..16: mol_type = other DNA
ctaggtcttaccacag

SEQ ID NO: 119 - DNA, 16 bp, synthetic construct
  source 1..16: mol_type = other DNA
ctgggtccaggcatgg

SEQ ID NO: 120 - DNA, 16 bp, synthetic construct
  source 1..16: mol_type = other DNA
attcagtctgggtcca

SEQ ID NO: 121 - DNA, 16 bp, synthetic construct
  source 1..16: mol_type = other DNA
gattcagtctgggtcc

SEQ ID NO: 122 - DNA, 16 bp, synthetic construct
  source 1..16: mol_type = other DNA
tggccttattcttgct

SEQ ID NO: 123 - DNA, 16 bp, synthetic construct
  source 1..16: mol_type = other DNA
caggggtgttggggtt

SEQ ID NO: 124 - DNA, 16 bp, synthetic construct
  source 1..16: mol_type = other DNA
  modified_base 1..16: mod_base = OTHER; note = phosphorothioate bond
  modified_base 1: mod_base = OTHER; note = 2'-O-[2-(N-methylcarbamoyl)ethyl]-5-methyluridine
  modified_base 2..3: mod_base = OTHER; note = modified LNA monomer with guanine base
  modified_base 6: mod_base = m5c
  modified_base 11: mod_base = m5c
  modified_base 14: mod_base = OTHER; note = modified LNA monomer with guanine base
  modified_base 15: mod_base = OTHER; note = modified LNA monomer with thymine base
  modified_base 16: mod_base = OTHER; note = 2'-O-[2-(N-methylcarbamoyl)ethyl]guanosine
tggggcatgtcttgtg

SEQ ID NO: 125 - DNA, 16 bp, synthetic construct
  source 1..16: mol_type = other DNA
  modified_base 1: mod_base = OTHER; note = 2'-O-(2-(N-methylcarbamoyl)ethyl)-5-methylcytidine
  modified_base 2: mod_base = OTHER; note = modified LNA monomer with 5-methylcytosine base
  modified_base 3: mod_base = OTHER; note = modified LNA monomer with thymine base
  modified_base 6: mod_base = m5c
  modified_base 13: mod_base = m5c
  modified_base 14..15: mod_base = OTHER; note = modified LNA monomer with 5-methylcytosine base
  modified_base 16: mod_base = OTHER; note = 2'-O-(2-(N-methylcarbamoyl)ethyl)guanosine
  modified_base 1..16: mod_base = OTHER; note = phosphorothioate bond
ccttgctgatttcccg

SEQ ID NO: 126 - DNA, 16 bp, synthetic construct
  source 1..16: mol_type = other DNA
  modified_base 1..16: mod_base = OTHER; note = phosphorothioate bond
  modified_base 1: mod_base = OTHER; note = 2'-O-[2-(N-methylcarbamoyl)ethyl]-5-methyluridine
  modified_base 2: mod_base = OTHER; note = modified LNA monomer with 5-methylcytosine base
  modified_base 3: mod_base = OTHER; note = modified LNA monomer with adenine base
  modified_base 5..6: mod_base = m5c
  modified_base 11..12: mod_base = m5c
  modified_base 14: mod_base = OTHER; note = modified LNA monomer with guanine base
  modified_base 15: mod_base = OTHER; note = modified LNA monomer with adenine base
  modified_base 16: mod_base = OTHER; note = 2'-O-(2-(N-methylcarbamoyl)ethyl)-5-methylcytidine
tcagccagtacctgac

SEQ ID NO: 127 - DNA, 16 bp, synthetic construct
  source 1..16: mol_type = other DNA
  modified_base 1..16: mod_base = OTHER; note = phosphorothioate bond
  modified_base 1: mod_base = OTHER; note = 2'-O-(2-(N-methylcarbamoyl)ethyl)-5-methylcytidine
  modified_base 2..3: mod_base = OTHER; note = modified LNA monomer with thymine base
  modified_base 8..10: mod_base = m5c
  modified_base 14..15: mod_base = OTHER; note = modified LNA monomer with 5-methylcytosine base
  modified_base 16: mod_base = OTHER; note = 2'-O-[2-(N-methylcarbamoyl)ethyl]-5-methyluridine
ctttttgcccaggcct

SEQ ID NO: 128 - DNA, 16 bp, synthetic construct
  source 1..16: mol_type = other DNA
  modified_base 1..16: mod_base = OTHER; note = phosphorothioate bond
  modified_base 1: mod_base = OTHER; note = 2'-O-[2-(N-methylcarbamoyl)ethyl]adenosine
  modified_base 2: mod_base = OTHER; note = modified LNA monomer with 5-methylcytosine base
  modified_base 3: mod_base = OTHER; note = modified LNA monomer with thymine base
  modified_base 4..5: mod_base = m5c
  modified_base 14: mod_base = OTHER; note = modified LNA monomer with guanine base
  modified_base 15: mod_base = OTHER; note = modified LNA monomer with adenine base
  modified_base 16: mod_base = OTHER; note = 2'-O-[2-(N-methylcarbamoyl)ethyl]guanosine
actccaggtaggtgag

SEQ ID NO: 129 - DNA, 16 bp, synthetic construct
  source 1..16: mol_type = other DNA
  modified_base 1..16: mod_base = OTHER; note = phosphorothioate bond
  modified_base 1: mod_base = OTHER; note = 2'-O-[2-(N-methylcarbamoyl)ethyl]-5-methyluridine
  modified_base 2: mod_base = OTHER; note = modified LNA monomer with guanine base
  modified_base 3: mod_base = OTHER; note = modified LNA monomer with adenine base
  modified_base 7..8: mod_base = m5c
  modified_base 14..15: mod_base = OTHER; note = modified LNA monomer with guanine base
  modified_base 16: mod_base = OTHER; note = 2'-O-[2-(N-methylcarbamoyl)ethyl]adenosine
tgatagcctggaagga

SEQ ID NO: 130 - DNA, 16 bp, synthetic construct
  source 1..16: mol_type = other DNA
  modified_base 1..16: mod_base = OTHER; note = phosphorothioate bond
  modified_base 1: mod_base = OTHER; note = 2'-O-[2-(N-methylcarbamoyl)ethyl]-5-methyluridine
  modified_base 2: mod_base = OTHER; note = modified LNA monomer with 5-methylcytosine base
  modified_base 3: mod_base = OTHER; note = modifi ed LNA monomer with adenine base
  modified_base 5: mod_base = m5c
  modified_base 7..8: mod_base = m5c
  modified_base 11: mod_base = m5c
  modified_base 13: mod_base = m5c
  modified_base 14: mod_base = OTHER; note = modified LNA monomer with 5-methylcytosine base
  modified_base 15: mod_base = OTHER; note = modified LNA monomer with thymine base
  modified_base 16: mod_base = OTHER; note = 2'-O-(2-(N-methylcarbamoyl)ethyl)guanosine
tcagcaccatcacctg

SEQ ID NO: 131 - DNA, 16 bp, synthetic construct
  source 1..16: mol_type = other DNA
  modified_base 1..16: mod_base = OTHER; note = phosphorothioate bond
  modified_base 1: mod_base = OTHER; note = 2'-O-(2-(N-methylcarbamoyl)ethyl)guanosine
  modified_base 2..3: mod_base = OTHER; note = modified LNA monomer with adenine base
  modified_base 8: mod_base = m5c
  modified_base 13: mod_base = m5c
  modified_base 14: mod_base = OTHER; note = modified LNA monomer with 5-methylcytosine base
  modified_base 15: mod_base = OTHER; note = modified LNA monomer with adenine base
  modified_base 16: mod_base = OTHER; note = 2'-O-(2-(N-methylcarbamoyl)ethyl)guanosine
gaatgaacttgtccag

SEQ ID NO: 132 - DNA, 16 bp, synthetic construct
  source 1..16: mol_type = other DNA
  modified_base 1..16: mod_base = OTHER; note = phosphorothioate bond
  modified_base 1: mod_base = OTHER; note = 2'-O-(2-(N-methylcarbamoyl)ethyl)guanosine
  modified_base 2..3: mod_base = OTHER; note = modified LNA monomer with adenine base
  modified_base 7: mod_base = m5c
  modified_base 10: mod_base = m5c
  modified_base 13: mod_base = m5c
  modified_base 14: mod_base = OTHER; note = modified LNA monomer with thymine base
  modified_base 15: mod_base = OTHER; note = modified LNA monomer with guanine base
  modified_base 16: mod_base = OTHER; note = 2'-O-(2-(N-methylcarbamoyl)ethyl)guanosine
gaaattctgcagctgg

SEQ ID NO: 133 - DNA, 16 bp, synthetic construct
  source 1..16: mol_type = other DNA
  modified_base 1..16: mod_base = OTHER; note = phosphorothioate bond
  modified_base 1: mod_base = OTHER; note = 2'-O-[2-(N-methylcarbamoyl)ethyl]guanosine
  modified_base 2: mod_base = OTHER; note = modified LNA monomer with thymine base
  modified_base 3: mod_base = OTHER; note = modified LNA monomer with guanine base
  modified_base 12: mod_base = m5c
  modified_base 14: mod_base = OTHER; note = modified LNA monomer with guanine base
  modified_base 15: mod_base = OTHER; note = modified LNA monomer with 5-methylcytosine base
  modified_base 16: mod_base = OTHER; note = 2'-O-[2-(N-methylcarbamoyl)ethyl]adenosine
gtgttgaaattctgca

SEQ ID NO: 134 - DNA, 16 bp, synthetic construct
  source 1..16: mol_type = other DNA
  modified_base 1..16: mod_base = OTHER; note = phosphorothioate bond
  modified_base 1: mod_base = OTHER; note = 2'-O-[2-(N-methylcarbamoyl)ethyl]-5-methyluridine
  modified_base 2..3: mod_base = OTHER; note = modified LNA monomer with 5-methylcytosine base
  modified_base 10: mod_base = m5c
  modified_base 15: mod_base = OTHER; note = modified LNA monomer with guanine base
  modified_base 14: mod_base = OTHER; note = modified LNA monomer with adenine base
  modified_base 16: mod_base = OTHER; note = 2'-O-(2-(N-methylcarbamoyl)ethyl)adenosine
tccttgagtctggaga

SEQ ID NO: 135 - DNA, 16 bp, synthetic construct
  source 1..16: mol_type = other DNA
  modified_base 1..16: mod_base = OTHER; note = phosphorothioate bond
  modified_base 1: mod_base = OTHER; note = 2'-O-[2-(N-methylcarbamoyl)ethyl]guanosine
  modified_base 2..3: mod_base = OTHER; note = modified LNA monomer with guanine base
  modified_base 7..8: mod_base = m5c
  modified_base 14: mod_base = OTHER; note = modified LNA monomer with thymine base
  modified_base 15: mod_base = OTHER; note = modified LNA monomer with 5-methylcytosine base
  modified_base 16: mod_base = OTHER; note = 2'-O-[2-(N-methylcarbamoyl)ethyl]-5-methyluridine
gggagtccttgagtct

SEQ ID NO: 136 - DNA, 16 bp, synthetic construct
  source 1..16: mol_type = other DNA
  modified_base 1..16: mod_base = OTHER; note = phosphorothioate bond
  modified_base 1: mod_base = OTHER; note = 2'-O-[2-(N-methylcarbamoyl)ethyl]guanosine
  modified_base 2: mod_base = OTHER; note = modified LNA monomer with 5-methylcytosine base
  modified_base 3: mod_base = OTHER; note = modified LNA monomer with guanine base
  modified_base 14..15: mod_base = OTHER; note = modified LNA monomer with guanine base
  modified_base 16: mod_base = OTHER; note = 2'-O-[2-(N-methylcarbamoyl)ethyl]guanosine
gcgtagttgttgtggg

SEQ ID NO: 137 - DNA, 16 bp, synthetic construct
  source 1..16: mol_type = other DNA
  modified_base 1..16: mod_base = OTHER; note = phosphorothioate bond
  modified_base 1: mod_base = OTHER; note = 2'-O-[2-(N-methylcarbamoyl)ethyl]adenosine
  modified_base 2..3: mod_base = OTHER; note = modified LNA monomer with guanine base
  modified_base 5..6: mod_base = m5c
  modified_base 14: mod_base = OTHER; note = modified LNA monomer with guanine base
  modified_base 15: mod_base = OTHER; note = modified LNA monomer with 5-methylcytosine base
  modified_base 16: mod_base = OTHER; note = 2'-O-[2-(N-methylcarbamoyl)ethyl]adenosine
aggtccttgaggtgca

SEQ ID NO: 138 - DNA, 16 bp, synthetic construct
  source 1..16: mol_type = other DNA
  modified_base 1..16: mod_base = OTHER; note = phosphorothioate bond
  modified_base 1: mod_base = OTHER; note = 2'-O-[2-(N-methylcarbamoyl)ethyl]-5-methyluridine
  modified_base 3: mod_base = OTHER; note = modified LNA monomer with 5-methylcytosine base
  modified_base 2: mod_base = OTHER; note = modifi ed LNA monomer with thymine base
  modified_base 6: mod_base = m5c
  modified_base 14..15: mod_base = OTHER; note = modified LNA monomer with guanine base
  modified_base 16: mod_base = OTHER; note = 2'-O-[2-(N-methylcarbamoyl)ethyl]-5-methyluridine
ttcagcttgggtaggt

SEQ ID NO: 139 - DNA, 16 bp, synthetic construct
  source 1..16: mol_type = other DNA
  modified_base 1..16: mod_base = OTHER; note = phosphorothioate bond
  modified_base 1: mod_base = OTHER; note = 2'-O-[2-(N-methylcarbamoyl)ethyl]guanosine
  modified_base 2: mod_base = OTHER; note = modified LNA monomer with 5-methylcytosine base
  modified_base 3: mod_base = OTHER; note = modifi ed LNA monomer with adenine base
  modified_base 5: mod_base = m5c
  modified_base 10..11: mod_base = m5c
  modified_base 13: mod_base = m5c
  modified_base 14: mod_base = OTHER; note = modified LNA monomer with adenine base
  modified_base 15: mod_base = OTHER; note = modified LNA monomer with thymine base
  modified_base 16: mod_base = OTHER; note = 2'-O-[2-(N-methylcarbamoyl)ethyl]-5-methyluridine
gcagcagatcctcatt

SEQ ID NO: 140 - DNA, 16 bp, synthetic construct
  source 1..16: mol_type = other DNA
  modified_base 1..16: mod_base = OTHER; note = phosphorothioate bond
  modified_base 1: mod_base = OTHER; note = 2'-O-[2-(N-methylcarbamoyl)ethyl]-5-methyluridine
  modified_base 2: mod_base = OTHER; note = modified LNA monomer with guanine base
  modified_base 3: mod_base = OTHER; note = modifi ed LNA monomer with thymine base
  modified_base 13: mod_base = m5c
  modified_base 14: mod_base = OTHER; note = modified LNA monomer with 5-methylcytosine base
  modified_base 15: mod_base = OTHER; note = modified LNA monomer with adenine base
  modified_base 16: mod_base = OTHER; note = 2'-O-[2-(N-methylcarbamoyl)ethyl]guanosine
tgtagaagaggtccag

SEQ ID NO: 141 - DNA, 16 bp, synthetic construct
  source 1..16: mol_type = other DNA
  modified_base 1..16: mod_base = OTHER; note = phosphorothioate bond
  modified_base 1: mod_base = OTHER; note = 2'-O-[2-(N-methylcarbamoyl)ethyl]-5-methyluridine
  modified_base 16: mod_base = OTHER; note = 2'-O-[2-(N-methylcarbamoyl)ethyl]-5-methyluridine
  modified_base 14..15: mod_base = OTHER; note = modified LNA monomer with guanine base
  modified_base 2..3: mod_base = OTHER; note = modified LNA monomer with 5-methylcytosine base
tccgtgtagaagaggt

SEQ ID NO: 142 - DNA, 16 bp, synthetic construct
  source 1..16: mol_type = other DNA
  modified_base 1: mod_base = OTHER; note = 2'-O-(2-(N-methylcarbamoyl)ethyl)-5-methylcytidine
  modified_base 2: mod_base = OTHER; note = modified LNA monomer with 5-methylcytosine base
  modified_base 3: mod_base = OTHER; note = modified LNA monomer with guanine base
  modified_base 6: mod_base = m5c
  modified_base 14: mod_base = OTHER; note = modified LNA monomer with adenine base
  modified_base 15: mod_base = OTHER; note = modified LNA monomer with guanine base
  modified_base 16: mod_base = OTHER; note = 2'-O-(2-(N-methylcarbamoyl)ethyl)-5-methylcytidine
  modified_base 1..16: mod_base = OTHER; note = phosphorothioate bond
ccgggcataagaaagc

SEQ ID NO: 143 - DNA, 16 bp, synthetic construct
  source 1..16: mol_type = other DNA
  modified_base 1..16: mod_base = OTHER; note = phosphorothioate bond
  modified_base 1: mod_base = OTHER; note = 2'-O-[2-(N-methylcarbamoyl)ethyl]guanosine
  modified_base 2: mod_base = OTHER; note = modified LNA monomer with thymine base
  modified_base 3: mod_base = OTHER; note = modified LNA monomer with guanine base
  modified_base 4: mod_base = m5c
  modified_base 14..15: mod_base = OTHER; note = modified LNA monomer with guanine base
  modified_base 16: mod_base = OTHER; note = 2'-O-[2-(N-methylcarbamoyl)ethyl]adenosine
gtgcattgaaggggga

SEQ ID NO: 144 - DNA, 16 bp, synthetic construct
  source 1..16: mol_type = other DNA
  modified_base 1..16: mod_base = OTHER; note = phosphorothioate bond
  modified_base 1: mod_base = OTHER; note = 2'-O-[2-(N-methylcarbamoyl)ethyl]adenosine
  modified_base 2..3: mod_base = OTHER; note = modified LNA monomer with 5-methylcytosine base
  modified_base 6: mod_base = m5c
  modified_base 14: mod_base = OTHER; note = modified LNA monomer with 5-methylcytosine base
  modified_base 15: mod_base = OTHER; note = modified LNA monomer with adenine base
  modified_base 16: mod_base = OTHER; note = 2'-O-[2-(N-methylcarbamoyl)ethyl]-5-methyluridine
  modified_base 9: mod_base = m5c
  modified_base 11..12: mod_base = m5c
accagctgctccacat

SEQ ID NO: 145 - DNA, 16 bp, synthetic construct
  source 1..16: mol_type = other DNA
  modified_base 1..16: mod_base = OTHER; note = phosphorothioate bond
  modified_base 1: mod_base = OTHER; note = 2'-O-(2-(N-methylcarbamoyl)ethyl)guanosine
  modified_base 2..3: mod_base = OTHER; note = modified LNA monomer with adenine base
  modified_base 6: mod_base = m5c
  modified_base 10: mod_base = m5c
  modified_base 12..13: mod_base = m5c
  modified_base 14: mod_base = OTHER; note = modified LNA monomer with adenine base
  modified_base 15: mod_base = OTHER; note = modified LNA monomer with 5-methylcytosine base
  modified_base 16: mod_base = OTHER; note = 2'-O-(2-(N-methylcarbamoyl)ethyl)-5-methylcytidine
  modified_base 4: mod_base = m5c
gaacacagactccacc

SEQ ID NO: 146 - DNA, 16 bp, synthetic construct
  source 1..16: mol_type = other DNA
  modified_base 1..16: mod_base = OTHER; note = phosphorothioate bond
  modified_base 1: mod_base = OTHER; note = 2'-O-(2-(N-methylcarbamoyl)ethyl)-5-methylcytidine
  modified_base 2: mod_base = OTHER; note = modified LNA monomer with guanine base
  modified_base 11..12: mod_base = m5c
  modified_base 14..15: mod_base = OTHER; note = modified LNA monomer with 5-methylcytosine base
  modified_base 16: mod_base = OTHER; note = 2'-O-[2-(N-methylcarbamoyl)ethyl]-5-methyluridine
  modified_base 3: mod_base = OTHER; note = modified LNA monomer with 5-methylcytosine base
  modified_base 5: mod_base = m5c
cgctcaaagtcctcct

SEQ ID NO: 147 - DNA, 16 bp, synthetic construct
  source 1..16: mol_type = other DNA
  modified_base 1: mod_base = OTHER; note = 2'-O-(2-(N-methylcarbamoyl)ethyl)-5-methylcytidine
  modified_base 3: mod_base = OTHER; note = modified LNA monomer with 5-methylcytosine base
  modified_base 2: mod_base = OTHER; note = modified LNA monomer with thymine base
  modified_base 6: mod_base = m5c
  modified_base 15: mod_base = OTHER; note = modified LNA monomer with 5-methylcytosine base
  modified_base 16: mod_base = OTHER; note = 2'-O-(2-(N-methylcarbamoyl)ethyl)-5-methylcytidine
  modified_base 1..16: mod_base = OTHER; note = phosphorothioate bond
  modified_base 14: mod_base = OTHER; note = modified LNA monomer with thymine base
ctctgctgaaggatcc

SEQ ID NO: 148 - DNA, 16 bp, synthetic construct
  source 1..16: mol_type = other DNA
  modified_base 1: mod_base = OTHER; note = 2'-O-(2-(N-methylcarbamoyl)ethyl)-5-methylcytidine
  modified_base 2: mod_base = OTHER; note = modified LNA monomer with 5-methylcytosine base
  modified_base 3: mod_base = OTHER; note = modified LNA monomer with adenine base
  modified_base 5: mod_base = m5c
  modified_base 15: mod_base = OTHER; note = modified LNA monomer with adenine base
  modified_base 14: mod_base = OTHER; note = modified LNA monomer with guanine base
  modified_base 16: mod_base = OTHER; note = 2'-O-(2-(N-methylcarbamoyl)ethyl)-5-methyluridine
  modified_base 1..16: mod_base = OTHER; note = phosphorothioate bond
  modified_base 12: mod_base = m5c
ccaacttggagcagat

SEQ ID NO: 149 - DNA, 16 bp, synthetic construct
  source 1..16: mol_type = other DNA
  modified_base 1..16: mod_base = OTHER; note = phosphorothioate bond
  modified_base 1: mod_base = OTHER; note = 2'-O-[2-(N-methylcarbamoyl)ethyl]-5-methyluridine
  modified_base 3: mod_base = OTHER; note = modified LNA monomer with 5-methylcytosine base
  modified_base 2: mod_base = OTHER; note = modifi ed LNA monomer with thymine base
  modified_base 13: mod_base = m5c
  modified_base 14: mod_base = OTHER; note = modified LNA monomer with 5-methylcytosine base
  modified_base 16: mod_base = OTHER; note = 2'-O-[2-(N-methylcarbamoyl)ethyl]-5-methylcytidine
  modified_base 15: mod_base = OTHER; note = modified LNA monomer with thymine base
ttcggaaggtgacctc

SEQ ID NO: 150 - DNA, 16 bp, synthetic construct
  source 1..16: mol_type = other DNA
  modified_base 1..16: mod_base = OTHER; note = phosphorothioate bond
  modified_base 1: mod_base = OTHER; note = 2'-O-[2-(N-methylcarbamoyl)ethyl]adenosine
  modified_base 2: mod_base = OTHER; note = modified LNA monomer with guanine base
  modified_base 3: mod_base = OTHER; note = modified LNA monomer with 5-methylcytosine base
  modified_base 4: mod_base = m5c
  modified_base 8: mod_base = m5c
  modified_base 14: mod_base = OTHER; note = modified LNA monomer with guanine base
  modified_base 15: mod_base = OTHER; note = modified LNA monomer with adenine base
  modified_base 16: mod_base = OTHER; note = 2'-O-[2-(N-methylcarbamoyl)ethyl]-5-methylcytidine
agccttgcttggtgac

SEQ ID NO: 151 - DNA, 16 bp, synthetic construct
  source 1..16: mol_type = other DNA
  modified_base 1..16: mod_base = OTHER; note = phosphorothioate bond
  modified_base 1: mod_base = OTHER; note = 2'-O-[2-(N-methylcarbamoyl)ethyl]guanosine
  modified_base 2: mod_base = OTHER; note = modified LNA monomer with guanine base
  modified_base 3: mod_base = OTHER; note = modified LNA monomer with 5-methylcytosine base
  modified_base 4: mod_base = m5c
  modified_base 6: mod_base = m5c
  modified_base 9: mod_base = m5c
  modified_base 13: mod_base = m5c
  modified_base 14: mod_base = OTHER; note = modified LNA monomer with adenine base
  modified_base 15: mod_base = OTHER; note = modified LNA monomer with thymine base
  modified_base 16: mod_base = OTHER; note = 2'-O-[2-(N-methylcarbamoyl)ethyl]-5-methyluridine
ggcctcttcttacatt

SEQ ID NO: 152 - DNA, 16 bp, synthetic construct
  source 1..16: mol_type = other DNA
  modified_base 1..16: mod_base = OTHER; note = phosphorothioate bond
  modified_base 1: mod_base = OTHER; note = 2'-O-[2-(N-methylcarbamoyl)ethyl]guanosine
  modified_base 2: mod_base = OTHER; note = modified LNA monomer with guanine base
  modified_base 3: mod_base = OTHER; note = modified LNA monomer with adenine base
  modified_base 6: mod_base = m5c
  modified_base 10: mod_base = m5c
  modified_base 14: mod_base = OTHER; note = modified LNA monomer with guanine base
  modified_base 15: mod_base = OTHER; note = modified LNA monomer with thymine base
  modified_base 16: mod_base = OTHER; note = 2'-O-[2-(N-methylcarbamoyl)ethyl]-5-methylcytidine
ggattcagtctgggtc

SEQ ID NO: 153 - DNA, 16 bp, synthetic construct
  source 1..16: mol_type = other DNA
  modified_base 1..16: mod_base = OTHER; note = phosphorothioate bond
  modified_base 1: mod_base = OTHER; note = 2'-O-[2-(N-methylcarbamoyl)ethyl]guanosine
  modified_base 2..3: mod_base = OTHER; note = modified LNA monomer with guanine base
  modified_base 14..15: mod_base = OTHER; note = modified LNA monomer with guanine base
  modified_base 16: mod_base = OTHER; note = 2'-O-(2-(N-methylcarbamoyl)ethyl)-5-methylcytidine
gggggaaggaagaggc

SEQ ID NO: 154 - DNA, 16 bp, synthetic construct
  source 1..16: mol_type = other DNA
  modified_base 1..16: mod_base = OTHER; note = phosphorothioate bond
  modified_base 1: mod_base = OTHER; note = 2'-O-[2-(N-methylcarbamoyl)ethyl]guanosine
  modified_base 2: mod_base = OTHER; note = modified LNA monomer with guanine base
  modified_base 3: mod_base = OTHER; note = modified LNA monomer with adenine base
  modified_base 12: mod_base = m5c
  modified_base 14: mod_base = OTHER; note = modified LNA monomer with guanine base
  modified_base 15: mod_base = OTHER; note = modified LNA monomer with 5-methylcytosine base
  modified_base 16: mod_base = OTHER; note = 2'-O-[2-(N-methylcarbamoyl)ethyl]-5-methylcytidine
ggaaagaggaactgcc

SEQ ID NO: 155 - DNA, 16 bp, synthetic construct
  source 1..16: mol_type = other DNA
  modified_base 1..16: mod_base = OTHER; note = phosphorothioate bond
  modified_base 1: mod_base = OTHER; note = 2'-O-[2-(N-methylcarbamoyl)ethyl]-5-methylcytidine
  modified_base 2: mod_base = OTHER; note = modified LNA monomer with thymine base
  modified_base 3: mod_base = OTHER; note = modified LNA monomer with 5-methylcytosine base
  modified_base 4..5: mod_base = m5c
  modified_base 11: mod_base = m5c
  modified_base 14..15: mod_base = OTHER; note = modified LNA monomer with 5-methylcytosine base
  modified_base 16: mod_base = OTHER; note = 2'-O-[2-(N-methylcarbamoyl)ethyl]adenosine
ctccctgaagcatcca

SEQ ID NO: 156 - DNA, 16 bp, synthetic construct
  source 1..16: mol_type = other DNA
  modified_base 1..16: mod_base = OTHER; note = phosphorothioate bond
  modified_base 1: mod_base = OTHER; note = 2'-O-[2-(N-methylcarbamoyl)ethyl]adenosine
  modified_base 2: mod_base = OTHER; note = modified LNA monomer with guanine base
  modified_base 3: mod_base = OTHER; note = modified LNA monomer with 5-methylcytosine base
  modified_base 5: mod_base = m5c
  modified_base 9: mod_base = m5c
  modified_base 11..12: mod_base = m5c
  modified_base 14..15: mod_base = OTHER; note = modified LNA monomer with guanine base
  modified_base 16: mod_base = OTHER; note = 2'-O-[2-(N-methylcarbamoyl)ethyl]guanosine
agctcaaactccaggg

SEQ ID NO: 157 - DNA, 16 bp, synthetic construct
  source 1..16: mol_type = other DNA
  modified_base 1..16: mod_base = OTHER; note = phosphorothioate bond
  modified_base 1: mod_base = OTHER; note = 2'-O-[2-(N-methylcarbamoyl)ethyl]adenosine
  modified_base 2..3: mod_base = OTHER; note = modified LNA monomer with guanine base
  modified_base 14: mod_base = OTHER; note = modified LNA monomer with guanine base
  modified_base 15: mod_base = OTHER; note = modified LNA monomer with adenine base
  modified_base 16: mod_base = OTHER; note = 2'-O-[2-(N-methylcarbamoyl)ethyl]guanosine
aggagtggtttaagag

SEQ ID NO: 158 - DNA, 16 bp, synthetic construct
  source 1..16: mol_type = other DNA
  modified_base 1..16: mod_base = OTHER; note = phosphorothioate bond
  modified_base 1: mod_base = OTHER; note = 2'-O-[2-(N-methylcarbamoyl)ethyl]adenosine
  modified_base 2: mod_base = OTHER; note = modified LNA monomer with guanine base
  modified_base 3: mod_base = OTHER; note = modified LNA monomer with thymine base
  modified_base 6: mod_base = m5c
  modified_base 10..11: mod_base = m5c
  modified_base 14: mod_base = OTHER; note = modified LNA monomer with adenine base
  modified_base 15: mod_base = OTHER; note = modified LNA monomer with guanine base
  modified_base 16: mod_base = OTHER; note = 2'-O-[2-(N-methylcarbamoyl)ethyl]guanosine
agtgacttacctaagg

SEQ ID NO: 159 - DNA, 16 bp, synthetic construct
  source 1..16: mol_type = other DNA
  modified_base 1..16: mod_base = OTHER; note = phosphorothioate bond
  modified_base 1: mod_base = OTHER; note = 2'-O-[2-(N-methylcarbamoyl)ethyl]guanosine
  modified_base 2..3: mod_base = OTHER; note = modified LNA monomer with 5-methylcytosine base
  modified_base 8..9: mod_base = m5c
  modified_base 13: mod_base = m5c
  modified_base 14: mod_base = OTHER; note = modified LNA monomer with thymine base
  modified_base 15: mod_base = OTHER; note = modified LNA monomer with guanine base
  modified_base 16: mod_base = OTHER; note = 2'-O-[2-(N-methylcarbamoyl)ethyl]adenosine
gccatgaccttgctga

SEQ ID NO: 160 - DNA, 16 bp, synthetic construct
  source 1..16: mol_type = other DNA
  modified_base 1..16: mod_base = OTHER; note = phosphorothioate bond
  modified_base 1: mod_base = OTHER; note = 2'-O-[2-(N-methylcarbamoyl)ethyl]-5-methylcytidine
  modified_base 2: mod_base = OTHER; note = modified LNA monomer with adenine base
  modified_base 3: mod_base = OTHER; note = modified LNA monomer with thymine base
  modified_base 6..7: mod_base = m5c
  modified_base 13: mod_base = m5c
  modified_base 14: mod_base = OTHER; note = modified LNA monomer with adenine base
  modified_base 15: mod_base = OTHER; note = modified LNA monomer with guanine base
  modified_base 16: mod_base = OTHER; note = 2'-O-[2-(N-methylcarbamoyl)ethyl]guanosine
catgaccttggacagg

SEQ ID NO: 161 - DNA, 16 bp, synthetic construct
  source 1..16: mol_type = other DNA
  modified_base 1..16: mod_base = OTHER; note = phosphorothioate bond
  modified_base 1: mod_base = OTHER; note = 2'-O-[2-(N-methylcarbamoyl)ethyl]guanosine
  modified_base 2: mod_base = OTHER; note = modified LNA monomer with guanine base
  modified_base 3: mod_base = OTHER; note = modified LNA monomer with adenine base
  modified_base 12: mod_base = m5c
  modified_base 14: mod_base = OTHER; note = modified LNA monomer with guanine base
  modified_base 15: mod_base = OTHER; note = modified LNA monomer with 5-methylcytosine base
  modified_base 16: mod_base = OTHER; note = 2'-O-[2-(N-methylcarbamoyl)ethyl]adenosine
ggatatgaggtcagca

SEQ ID NO: 162 - DNA, 16 bp, synthetic construct
  source 1..16: mol_type = other DNA
  modified_base 1..16: mod_base = OTHER; note = phosphorothioate bond
  modified_base 1: mod_base = OTHER; note = 2'-O-[2-(N-methylcarbamoyl)ethyl]guanosine
  modified_base 2: mod_base = OTHER; note = modified LNA monomer with adenine base
  modified_base 3: mod_base = OTHER; note = modified LNA monomer with guanine base
  modified_base 6: mod_base = m5c
  modified_base 11: mod_base = m5c
  modified_base 14..15: mod_base = OTHER; note = modified LNA monomer with guanine base
  modified_base 16: mod_base = OTHER; note = 2'-O-[2-(N-methylcarbamoyl)ethyl]-5-methylcytidine
gagttctggtcaaggc

SEQ ID NO: 163 - DNA, 16 bp, synthetic construct
  source 1..16: mol_type = other DNA
  modified_base 1..16: mod_base = OTHER; note = phosphorothioate bond
  modified_base 1: mod_base = OTHER; note = 2'-O-[2-(N-methylcarbamoyl)ethyl]-5-methyluridine
  modified_base 2: mod_base = OTHER; note = modified LNA monomer with thymine base
  modified_base 3: mod_base = OTHER; note = modified LNA monomer with guanine base
  modified_base 14: mod_base = OTHER; note = modified LNA monomer with thymine base
  modified_base 15: mod_base = OTHER; note = modified LNA monomer with adenine base
  modified_base 16: mod_base = OTHER; note = 2'-O-[2-(N-methylcarbamoyl)ethyl]-5-methyluridine
ttggaagtgggattat

SEQ ID NO: 164 - DNA, 16 bp, synthetic construct
  source 1..16: mol_type = other DNA
  modified_base 1..16: mod_base = OTHER; note = phosphorothioate bond
  modified_base 1: mod_base = OTHER; note = 2'-O-[2-(N-methylcarbamoyl)ethyl]guanosine
  modified_base 2: mod_base = OTHER; note = modified LNA monomer with thymine base
  modified_base 3: mod_base = OTHER; note = modified LNA monomer with guanine base
  modified_base 4: mod_base = m5c
  modified_base 9: mod_base = m5c
  modified_base 14..15: mod_base = OTHER; note = modified LNA monomer with guanine base
  modified_base 16: mod_base = OTHER; note = 2'-O-[2-(N-methylcarbamoyl)ethyl]guanosine
gtgctgagctaggggg

SEQ ID NO: 165 - DNA, 16 bp, synthetic construct
  source 1..16: mol_type = other DNA
  modified_base 1..16: mod_base = OTHER; note = phosphorothioate bond
  modified_base 1: mod_base = OTHER; note = 2'-O-[2-(N-methylcarbamoyl)ethyl]-5-methyluridine
  modified_base 2: mod_base = OTHER; note = modified LNA monomer with 5-methylcytosine base
  modified_base 3: mod_base = OTHER; note = modified LNA monomer with adenine base
  modified_base 5..6: mod_base = m5c
  modified_base 11..12: mod_base = m5c
  modified_base 14: mod_base = OTHER; note = modified LNA monomer with guanine base
  modified_base 15: mod_base = OTHER; note = modified LNA monomer with adenine base
  modified_base 16: mod_base = OTHER; note = 2'-O-[2-(N-methylcarbamoyl)ethyl]guanosine
tcagccagtacctgag

SEQ ID NO: 166 - DNA, 16 bp, synthetic construct
  source 1..16: mol_type = other DNA
  modified_base 1..16: mod_base = OTHER; note = phosphorothioate bond
  modified_base 1: mod_base = OTHER; note = 2'-O-[2-(N-methylcarbamoyl)ethyl]guanosine
  modified_base 2: mod_base = OTHER; note = modified LNA monomer with guanine base
  modified_base 3: mod_base = OTHER; note = modified LNA monomer with 5-methylcytosine base
  modified_base 7: mod_base = m5c
  modified_base 9: mod_base = m5c
  modified_base 11: mod_base = m5c
  modified_base 14: mod_base = OTHER; note = modified LNA monomer with guanine base
  modified_base 15: mod_base = OTHER; note = modified LNA monomer with thymine base
  modified_base 16: mod_base = OTHER; note = 2'-O-[2-(N-methylcarbamoyl)ethyl]-5-methylcytidine
ggctgactcacaggtc

SEQ ID NO: 167 - DNA, 16 bp, synthetic construct
  source 1..16: mol_type = other DNA
  modified_base 1..16: mod_base = OTHER; note = phosphorothioate bond
  modified_base 1: mod_base = OTHER; note = 2'-O-[2-(N-methylcarbamoyl)ethyl]guanosine
  modified_base 2: mod_base = OTHER; note = modified LNA monomer with guanine base
  modified_base 3: mod_base = OTHER; note = modified LNA monomer with 5-methylcytosine base
  modified_base 6: mod_base = m5c
  modified_base 8: mod_base = m5c
  modified_base 14: mod_base = OTHER; note = modified LNA monomer with guanine base
  modified_base 15: mod_base = OTHER; note = modified LNA monomer with adenine base
  modified_base 16: mod_base = OTHER; note = 2'-O-[2-(N-methylcarbamoyl)ethyl]guanosine
ggctgctcattgggag

SEQ ID NO: 168 - DNA, 16 bp, synthetic construct
  source 1..16: mol_type = other DNA
  modified_base 1..16: mod_base = OTHER; note = phosphorothioate bond
  modified_base 1: mod_base = OTHER; note = 2'-O-[2-(N-methylcarbamoyl)ethyl]adenosine
  modified_base 2..3: mod_base = OTHER; note = modified LNA monomer with 5-methylcytosine base
  modified_base 11..12: mod_base = m5c
  modified_base 14..15: mod_base = OTHER; note = modified LNA monomer with guanine base
  modified_base 16: mod_base = OTHER; note = 2'-O-[2-(N-methylcarbamoyl)ethyl]adenosine
accgtgatagcctgga

SEQ ID NO: 169 - DNA, 16 bp, synthetic construct
  source 1..16: mol_type = other DNA
  modified_base 1..16: mod_base = OTHER; note = phosphorothioate bond
  modified_base 1: mod_base = OTHER; note = 2'-O-[2-(N-methylcarbamoyl)ethyl]-5-methyluridine
  modified_base 2..3: mod_base = OTHER; note = modified LNA monomer with guanine base
  modified_base 4..5: mod_base = m5c
  modified_base 7: mod_base = m5c
  modified_base 13: mod_base = m5c
  modified_base 14: mod_base = OTHER; note = modified LNA monomer with thymine base
  modified_base 15: mod_base = OTHER; note = modified LNA monomer with 5-methylcytosine base
  modified_base 16: mod_base = OTHER; note = 2'-O-[2-(N-methylcarbamoyl)ethyl]adenosine
tggcctctttaactca

SEQ ID NO: 170 - DNA, 16 bp, synthetic construct
  source 1..16: mol_type = other DNA
  modified_base 1..16: mod_base = OTHER; note = phosphorothioate bond
  modified_base 1: mod_base = OTHER; note = 2'-O-[2-(N-methylcarbamoyl)ethyl]adenosine
  modified_base 2: mod_base = OTHER; note = modified LNA monomer with guanine base
  modified_base 3: mod_base = OTHER; note = modified LNA monomer with 5-methylcytosine base
  modified_base 5..6: mod_base = m5c
  modified_base 9: mod_base = m5c
  modified_base 11..12: mod_base = m5c
  modified_base 14: mod_base = OTHER; note = modified LNA monomer with guanine base
  modified_base 15: mod_base = OTHER; note = modified LNA monomer with 5-methylcytosine base
  modified_base 16: mod_base = OTHER; note = 2'-O-[2-(N-methylcarbamoyl)ethyl]adenosine
agcaccatcacctgca

SEQ ID NO: 171 - DNA, 16 bp, synthetic construct
  source 1..16: mol_type = other DNA
  modified_base 1..16: mod_base = OTHER; note = phosphorothioate bond
  modified_base 1: mod_base = OTHER; note = 2'-O-[2-(N-methylcarbamoyl)ethyl]-5-methylcytidine
  modified_base 2: mod_base = OTHER; note = modified LNA monomer with thymine base
  modified_base 3: mod_base = OTHER; note = modified LNA monomer with 5-methylcytosine base
  modified_base 11: mod_base = m5c
  modified_base 13: mod_base = m5c
  modified_base 14: mod_base = OTHER; note = modified LNA monomer with adenine base
  modified_base 15: mod_base = OTHER; note = modified LNA monomer with 5-methylcytosine base
  modified_base 16: mod_base = OTHER; note = 2'-O-[2-(N-methylcarbamoyl)ethyl]adenosine
ctctgagagtcacaca

SEQ ID NO: 172 - DNA, 16 bp, synthetic construct
  source 1..16: mol_type = other DNA
  modified_base 1..16: mod_base = OTHER; note = phosphorothioate bond
  modified_base 1: mod_base = OTHER; note = 2'-O-[2-(N-methylcarbamoyl)ethyl]-5-methyluridine
  modified_base 2: mod_base = OTHER; note = modified LNA monomer with thymine base
  modified_base 3: mod_base = OTHER; note = modified LNA monomer with guanine base
  modified_base 13: mod_base = m5c
  modified_base 14: mod_base = OTHER; note = modified LNA monomer with adenine base
  modified_base 15: mod_base = OTHER; note = modified LNA monomer with guanine base
  modified_base 16: mod_base = OTHER; note = 2'-O-[2-(N-methylcarbamoyl)ethyl]guanosine
ttggggaatagacagg

SEQ ID NO: 173 - DNA, 16 bp, synthetic construct
  source 1..16: mol_type = other DNA
  modified_base 1..16: mod_base = OTHER; note = phosphorothioate bond
  modified_base 1: mod_base = OTHER; note = 2'-O-[2-(N-methylcarbamoyl)ethyl]adenosine
  modified_base 2..3: mod_base = OTHER; note = modified LNA monomer with guanine base
  modified_base 4: mod_base = m5c
  modified_base 14..15: mod_base = OTHER; note = modified LNA monomer with 5-methylcytosine base
  modified_base 16: mod_base = OTHER; note = 2'-O-[2-(N-methylcarbamoyl)ethyl]adenosine
aggcatgtgtggacca

SEQ ID NO: 174 - DNA, 16 bp, synthetic construct
  source 1..16: mol_type = other DNA
  modified_base 1..16: mod_base = OTHER; note = phosphorothioate bond
  modified_base 1: mod_base = OTHER; note = 2'-O-[2-(N-methylcarbamoyl)ethyl]adenosine
  modified_base 2: mod_base = OTHER; note = modified LNA monomer with guanine base
  modified_base 3: mod_base = OTHER; note = modified LNA monomer with 5-methylcytosine base
  modified_base 12..13: mod_base = m5c
  modified_base 14: mod_base = OTHER; note = modified LNA monomer with thymine base
  modified_base 15: mod_base = OTHER; note = modified LNA monomer with 5-methylcytosine base
  modified_base 16: mod_base = OTHER; note = 2'-O-[2-(N-methylcarbamoyl)ethyl]-5-methyluridine
agctggtggagcctct

SEQ ID NO: 175 - DNA, 16 bp, synthetic construct
  source 1..16: mol_type = other DNA
  modified_base 1..16: mod_base = OTHER; note = phosphorothioate bond
  modified_base 1: mod_base = OTHER; note = 2'-O-[2-(N-methylcarbamoyl)ethyl]-5-methylcytidine
  modified_base 2: mod_base = OTHER; note = modified LNA monomer with thymine base
  modified_base 3: mod_base = OTHER; note = modified LNA monomer with guanine base
  modified_base 4: mod_base = m5c
  modified_base 7: mod_base = m5c
  modified_base 14: mod_base = OTHER; note = modified LNA monomer with adenine base
  modified_base 15: mod_base = OTHER; note = modified LNA monomer with guanine base
  modified_base 16: mod_base = OTHER; note = 2'-O-[2-(N-methylcarbamoyl)ethyl]-5-methylcytidine
ctgcagctggtggagc

SEQ ID NO: 176 - DNA, 16 bp, synthetic construct
  source 1..16: mol_type = other DNA
  modified_base 1..16: mod_base = OTHER; note = phosphorothioate bond
  modified_base 1: mod_base = OTHER; note = 2'-O-[2-(N-methylcarbamoyl)ethyl]-5-methyluridine
  modified_base 2: mod_base = OTHER; note = modified LNA monomer with 5-methylcytosine base
  modified_base 3: mod_base = OTHER; note = modified LNA monomer with thymine base
  modified_base 5: mod_base = m5c
  modified_base 8: mod_base = m5c
  modified_base 14: mod_base = OTHER; note = modified LNA monomer with guanine base
  modified_base 15: mod_base = OTHER; note = modified LNA monomer with adenine base
  modified_base 16: mod_base = OTHER; note = 2'-O-[2-(N-methylcarbamoyl)ethyl]guanosine
tctgcagctggtggag

SEQ ID NO: 177 - DNA, 16 bp, synthetic construct
  source 1..16: mol_type = other DNA
  modified_base 1..16: mod_base = OTHER; note = phosphorothioate bond
  modified_base 1: mod_base = OTHER; note = 2'-O-[2-(N-methylcarbamoyl)ethyl]-5-methyluridine
  modified_base 2: mod_base = OTHER; note = modified LNA monomer with thymine base
  modified_base 3: mod_base = OTHER; note = modified LNA monomer with 5-methylcytosine base
  modified_base 6: mod_base = m5c
  modified_base 9: mod_base = m5c
  modified_base 14..15: mod_base = OTHER; note = modified LNA monomer with guanine base
  modified_base 16: mod_base = OTHER; note = 2'-O-[2-(N-methylcarbamoyl)ethyl]adenosine
ttctgcagctggtgga

SEQ ID NO: 178 - DNA, 16 bp, synthetic construct
  source 1..16: mol_type = other DNA
  modified_base 1..16: mod_base = OTHER; note = phosphorothioate bond
  modified_base 1: mod_base = OTHER; note = 2'-O-[2-(N-methylcarbamoyl)ethyl]adenosine
  modified_base 2..3: mod_base = OTHER; note = modified LNA monomer with thymine base
  modified_base 4: mod_base = m5c
  modified_base 7: mod_base = m5c
  modified_base 10: mod_base = m5c
  modified_base 14: mod_base = OTHER; note = modified LNA monomer with thymine base
  modified_base 15: mod_base = OTHER; note = modified LNA monomer with guanine base
  modified_base 16: mod_base = OTHER; note = 2'-O-[2-(N-methylcarbamoyl)ethyl]guanosine
attctgcagctggtgg

SEQ ID NO: 179 - DNA, 16 bp, synthetic construct
  source 1..16: mol_type = other DNA
  modified_base 1..16: mod_base = OTHER; note = phosphorothioate bond
  modified_base 1: mod_base = OTHER; note = 2'-O-[2-(N-methylcarbamoyl)ethyl]adenosine
  modified_base 2: mod_base = OTHER; note = modified LNA monomer with adenine base
  modified_base 3: mod_base = OTHER; note = modified LNA monomer with thymine base
  modified_base 5: mod_base = m5c
  modified_base 8: mod_base = m5c
  modified_base 11: mod_base = m5c
  modified_base 14: mod_base = OTHER; note = modified LNA monomer with guanine base
  modified_base 15: mod_base = OTHER; note = modified LNA monomer with thymine base
  modified_base 16: mod_base = OTHER; note = 2'-O-[2-(N-methylcarbamoyl)ethyl]guanosine
aattctgcagctggtg

SEQ ID NO: 180 - DNA, 16 bp, synthetic construct
  source 1..16: mol_type = other DNA
  modified_base 1: mod_base = OTHER; note = 2'-O-[2-(N-methylcarbamoyl)ethyl]-5-methyluridine
  modified_base 1..16: mod_base = OTHER; note = phosphorothioate bond
  modified_base 2: mod_base = OTHER; note = modified LNA monomer with thymine base
  modified_base 3: mod_base = OTHER; note = modified LNA monomer with guanine base
  modified_base 9: mod_base = m5c
  modified_base 12: mod_base = m5c
  modified_base 14: mod_base = OTHER; note = modified LNA monomer with guanine base
  modified_base 15: mod_base = OTHER; note = modified LNA monomer with 5-methylcytosine base
  modified_base 16: mod_base = OTHER; note = 2'-O-[2-(N-methylcarbamoyl)ethyl]-5-methyluridine
ttgaaattctgcagct

SEQ ID NO: 181 - DNA, 16 bp, synthetic construct
  source 1..16: mol_type = other DNA
  modified_base 1..16: mod_base = OTHER; note = phosphorothioate bond
  modified_base 1: mod_base = OTHER; note = 2'-O-[2-(N-methylcarbamoyl)ethyl]guanosine
  modified_base 2..3: mod_base = OTHER; note = modified LNA monomer with thymine base
  modified_base 10: mod_base = m5c
  modified_base 13: mod_base = m5c
  modified_base 14: mod_base = OTHER; note = modified LNA monomer with adenine base
  modified_base 15: mod_base = OTHER; note = modified LNA monomer with guanine base
  modified_base 16: mod_base = OTHER; note = 2'-O-[2-(N-methylcarbamoyl)ethyl]-5-methylcytidine
gttgaaattctgcagc

SEQ ID NO: 182 - DNA, 16 bp, synthetic construct
  source 1..16: mol_type = other DNA
  modified_base 1..16: mod_base = OTHER; note = phosphorothioate bond
  modified_base 1: mod_base = OTHER; note = 2'-O-[2-(N-methylcarbamoyl)ethyl]-5-methyluridine
  modified_base 2: mod_base = OTHER; note = modified LNA monomer with guanine base
  modified_base 3: mod_base = OTHER; note = modified LNA monomer with thymine base
  modified_base 11: mod_base = m5c
  modified_base 14: mod_base = OTHER; note = modified LNA monomer with 5-methylcytosine base
  modified_base 15: mod_base = OTHER; note = modified LNA monomer with adenine base
  modified_base 16: mod_base = OTHER; note = 2'-O-[2-(N-methylcarbamoyl)ethyl]guanosine
tgttgaaattctgcag

SEQ ID NO: 183 - DNA, 16 bp, synthetic construct
  source 1..16: mol_type = other DNA
  modified_base 1..16: mod_base = OTHER; note = phosphorothioate bond
  modified_base 1: mod_base = OTHER; note = 2'-O-[2-(N-methylcarbamoyl)ethyl]-5-methylcytidine
  modified_base 2: mod_base = OTHER; note = modified LNA monomer with guanine base
  modified_base 3: mod_base = OTHER; note = modified LNA monomer with thymine base
  modified_base 13: mod_base = m5c
  modified_base 14: mod_base = OTHER; note = modified LNA monomer with thymine base
  modified_base 15: mod_base = OTHER; note = modified LNA monomer with guanine base
  modified_base 16: mod_base = OTHER; note = 2'-O-[2-(N-methylcarbamoyl)ethyl]-5-methylcytidine
cgtgttgaaattctgc

SEQ ID NO: 184 - DNA, 16 bp, synthetic construct
  source 1..16: mol_type = other DNA
  modified_base 1..16: mod_base = OTHER; note = phosphorothioate bond
  modified_base 1: mod_base = OTHER; note = 2'-O-[2-(N-methylcarbamoyl)ethyl]guanosine
  modified_base 2: mod_base = OTHER; note = modified LNA monomer with 5-methylcytosine base
  modified_base 3: mod_base = OTHER; note = modified LNA monomer with guanine base
  modified_base 14: mod_base = OTHER; note = modified LNA monomer with 5-methylcytosine base
  modified_base 15: mod_base = OTHER; note = modified LNA monomer with thymine base
  modified_base 16: mod_base = OTHER; note = 2'-O-[2-(N-methylcarbamoyl)ethyl]guanosine
gcgtgttgaaattctg

SEQ ID NO: 185 - DNA, 16 bp, synthetic construct
  source 1..16: mol_type = other DNA
  modified_base 1..16: mod_base = OTHER; note = phosphorothioate bond
  modified_base 1: mod_base = OTHER; note = 2'-O-[2-(N-methylcarbamoyl)ethyl]adenosine
  modified_base 2: mod_base = OTHER; note = modified LNA monomer with guanine base
  modified_base 3: mod_base = OTHER; note = modified LNA monomer with 5-methylcytosine base
  modified_base 14: mod_base = OTHER; note = modified LNA monomer with thymine base
  modified_base 15: mod_base = OTHER; note = modified LNA monomer with 5-methylcytosine base
  modified_base 16: mod_base = OTHER; note = 2'-O-[2-(N-methylcarbamoyl)ethyl]-5-methyluridine
agcgtgttgaaattct

SEQ ID NO: 186 - DNA, 16 bp, synthetic construct
  source 1..16: mol_type = other DNA
  modified_base 1..16: mod_base = OTHER; note = phosphorothioate bond
  modified_base 1: mod_base = OTHER; note = 2'-O-[2-(N-methylcarbamoyl)ethyl]guanosine
  modified_base 2: mod_base = OTHER; note = modified LNA monomer with adenine base
  modified_base 3: mod_base = OTHER; note = modified LNA monomer with guanine base
  modified_base 5..6: mod_base = m5c
  modified_base 13: mod_base = m5c
  modified_base 14: mod_base = OTHER; note = modified LNA monomer with thymine base
  modified_base 15: mod_base = OTHER; note = modified LNA monomer with guanine base
  modified_base 16: mod_base = OTHER; note = 2'-O-[2-(N-methylcarbamoyl)ethyl]guanosine
gagtccttgagtctgg

SEQ ID NO: 187 - DNA, 16 bp, synthetic construct
  source 1..16: mol_type = other DNA
  modified_base 1..16: mod_base = OTHER; note = phosphorothioate bond
  modified_base 1: mod_base = OTHER; note = 2'-O-[2-(N-methylcarbamoyl)ethyl]guanosine
  modified_base 2: mod_base = OTHER; note = modified LNA monomer with guanine base
  modified_base 3: mod_base = OTHER; note = modified LNA monomer with adenine base
  modified_base 6..7: mod_base = m5c
  modified_base 14: mod_base = OTHER; note = modified LNA monomer with 5-methylcytosine base
  modified_base 15: mod_base = OTHER; note = modified LNA monomer with thymine base
  modified_base 16: mod_base = OTHER; note = 2'-O-[2-(N-methylcarbamoyl)ethyl]guanosine
ggagtccttgagtctg

SEQ ID NO: 188 - DNA, 16 bp, synthetic construct
  source 1..16: mol_type = other DNA
  modified_base 1..16: mod_base = OTHER; note = phosphorothioate bond
  modified_base 1: mod_base = OTHER; note = 2'-O-[2-(N-methylcarbamoyl)ethyl]-5-methyluridine
  modified_base 2..3: mod_base = OTHER; note = modified LNA monomer with guanine base
  modified_base 8..9: mod_base = m5c
  modified_base 14: mod_base = OTHER; note = modified LNA monomer with guanine base
  modified_base 15: mod_base = OTHER; note = modified LNA monomer with thymine base
  modified_base 16: mod_base = OTHER; note = 2'-O-[2-(N-methylcarbamoyl)ethyl]-5-methylcytidine
tgggagtccttgagtc

SEQ ID NO: 189 - DNA, 16 bp, synthetic construct
  source 1..16: mol_type = other DNA
  modified_base 1..16: mod_base = OTHER; note = phosphorothioate bond
  modified_base 1: mod_base = OTHER; note = 2'-O-[2-(N-methylcarbamoyl)ethyl]adenosine
  modified_base 2: mod_base = OTHER; note = modified LNA monomer with thymine base
  modified_base 3: mod_base = OTHER; note = modified LNA monomer with guanine base
  modified_base 9..10: mod_base = m5c
  modified_base 14: mod_base = OTHER; note = modified LNA monomer with adenine base
  modified_base 15: mod_base = OTHER; note = modified LNA monomer with guanine base
  modified_base 16: mod_base = OTHER; note = 2'-O-[2-(N-methylcarbamoyl)ethyl]-5-methyluridine
atgggagtccttgagt

SEQ ID NO: 190 - DNA, 16 bp, synthetic construct
  source 1..16: mol_type = other DNA
  modified_base 1..16: mod_base = OTHER; note = phosphorothioate bond
  modified_base 1: mod_base = OTHER; note = 2'-O-[2-(N-methylcarbamoyl)ethyl]-5-methylcytidine
  modified_base 2: mod_base = OTHER; note = modified LNA monomer with adenine base
  modified_base 3: mod_base = OTHER; note = modified LNA monomer with thymine base
  modified_base 10..11: mod_base = m5c
  modified_base 14: mod_base = OTHER; note = modified LNA monomer with guanine base
  modified_base 15: mod_base = OTHER; note = modified LNA monomer with adenine base
  modified_base 16: mod_base = OTHER; note = 2'-O-[2-(N-methylcarbamoyl)ethyl]guanosine
catgggagtccttgag

SEQ ID NO: 191 - DNA, 16 bp, synthetic construct
  source 1..16: mol_type = other DNA
  modified_base 1..16: mod_base = OTHER; note = phosphorothioate bond
  modified_base 1: mod_base = OTHER; note = 2'-O-[2-(N-methylcarbamoyl)ethyl]-5-methyluridine
  modified_base 2: mod_base = OTHER; note = modified LNA monomer with thymine base
  modified_base 3: mod_base = OTHER; note = modified LNA monomer with guanine base
  modified_base 7: mod_base = m5c
  modified_base 14: mod_base = OTHER; note = modified LNA monomer with guanine base
  modified_base 15: mod_base = OTHER; note = modified LNA monomer with adenine base
  modified_base 16: mod_base = OTHER; note = 2'-O-[2-(N-methylcarbamoyl)ethyl]guanosine
ttggagctttggggag

SEQ ID NO: 192 - DNA, 16 bp, synthetic construct
  source 1..16: mol_type = other DNA
  modified_base 1..16: mod_base = OTHER; note = phosphorothioate bond
  modified_base 1: mod_base = OTHER; note = 2'-O-[2-(N-methylcarbamoyl)ethyl]-5-methyluridine
  modified_base 2..3: mod_base = OTHER; note = modified LNA monomer with guanine base
  modified_base 11: mod_base = m5c
  modified_base 14: mod_base = OTHER; note = modified LNA monomer with guanine base
  modified_base 15: mod_base = OTHER; note = modified LNA monomer with 5-methylcytosine base
  modified_base 16: mod_base = OTHER; note = 2'-O-[2-(N-methylcarbamoyl)ethyl]guanosine
tgggtaggtgcaggcg

SEQ ID NO: 193 - DNA, 16 bp, synthetic construct
  source 1..16: mol_type = other DNA
  modified_base 1..16: mod_base = OTHER; note = phosphorothioate bond
  modified_base 1: mod_base = OTHER; note = 2'-O-[2-(N-methylcarbamoyl)ethyl]-5-methyluridine
  modified_base 2: mod_base = OTHER; note = modified LNA monomer with thymine base
  modified_base 3: mod_base = OTHER; note = modified LNA monomer with guanine base
  modified_base 12: mod_base = m5c
  modified_base 14..15: mod_base = OTHER; note = modified LNA monomer with guanine base
  modified_base 16: mod_base = OTHER; note = 2'-O-[2-(N-methylcarbamoyl)ethyl]-5-methylcytidine
ttgggtaggtgcaggc

SEQ ID NO: 194 - DNA, 16 bp, synthetic construct
  source 1..16: mol_type = other DNA
  modified_base 1..16: mod_base = OTHER; note = phosphorothioate bond
  modified_base 1: mod_base = OTHER; note = 2'-O-[2-(N-methylcarbamoyl)ethyl]-5-methylcytidine
  modified_base 2..3: mod_base = OTHER; note = modified LNA monomer with thymine base
  modified_base 13: mod_base = m5c
  modified_base 14: mod_base = OTHER; note = modified LNA monomer with adenine base
  modified_base 15: mod_base = OTHER; note = modified LNA monomer with guanine base
  modified_base 16: mod_base = OTHER; note = 2'-O-[2-(N-methylcarbamoyl)ethyl]guanosine
cttgggtaggtgcagg

SEQ ID NO: 195 - DNA, 16 bp, synthetic construct
  source 1..16: mol_type = other DNA
  modified_base 1..16: mod_base = OTHER; note = phosphorothioate bond
  modified_base 1: mod_base = OTHER; note = 2'-O-[2-(N-methylcarbamoyl)ethyl]guanosine
  modified_base 2: mod_base = OTHER; note = modified LNA monomer with 5-methylcytosine base
  modified_base 3: mod_base = OTHER; note = modified LNA monomer with thymine base
  modified_base 14: mod_base = OTHER; note = modified LNA monomer with 5-methylcytosine base
  modified_base 15: mod_base = OTHER; note = modified LNA monomer with adenine base
  modified_base 16: mod_base = OTHER; note = 2'-O-[2-(N-methylcarbamoyl)ethyl]guanosine
gcttgggtaggtgcag

SEQ ID NO: 196 - DNA, 16 bp, synthetic construct
  source 1..16: mol_type = other DNA
  modified_base 1..16: mod_base = OTHER; note = phosphorothioate bond
  modified_base 1: mod_base = OTHER; note = 2'-O-[2-(N-methylcarbamoyl)ethyl]adenosine
  modified_base 2: mod_base = OTHER; note = modified LNA monomer with guanine base
  modified_base 3: mod_base = OTHER; note = modified LNA monomer with 5-methylcytosine base
  modified_base 14: mod_base = OTHER; note = modified LNA monomer with guanine base
  modified_base 15: mod_base = OTHER; note = modified LNA monomer with 5-methylcytosine base
  modified_base 16: mod_base = OTHER; note = 2'-O-[2-(N-methylcarbamoyl)ethyl]adenosine
agcttgggtaggtgca

SEQ ID NO: 197 - DNA, 16 bp, synthetic construct
  source 1..16: mol_type = other DNA
  modified_base 1..16: mod_base = OTHER; note = phosphorothioate bond
  modified_base 1: mod_base = OTHER; note = 2'-O-[2-(N-methylcarbamoyl)ethyl]-5-methylcytidine
  modified_base 2: mod_base = OTHER; note = modified LNA monomer with adenine base
  modified_base 3: mod_base = OTHER; note = modified LNA monomer with guanine base
  modified_base 4: mod_base = m5c
  modified_base 14: mod_base = OTHER; note = modified LNA monomer with thymine base
  modified_base 15: mod_base = OTHER; note = modified LNA monomer with guanine base
  modified_base 16: mod_base = OTHER; note = 2'-O-[2-(N-methylcarbamoyl)ethyl]-5-methylcytidine
cagcttgggtaggtgc

SEQ ID NO: 198 - DNA, 16 bp, synthetic construct
  source 1..16: mol_type = other DNA
  modified_base 1..16: mod_base = OTHER; note = phosphorothioate bond
  modified_base 1: mod_base = OTHER; note = 2'-O-[2-(N-methylcarbamoyl)ethyl]-5-methyluridine
  modified_base 2: mod_base = OTHER; note = modified LNA monomer with 5-methylcytosine base
  modified_base 3: mod_base = OTHER; note = modified LNA monomer with adenine base
  modified_base 5: mod_base = m5c
  modified_base 14: mod_base = OTHER; note = modified LNA monomer with guanine base
  modified_base 15: mod_base = OTHER; note = modified LNA monomer with thymine base
  modified_base 16: mod_base = OTHER; note = 2'-O-[2-(N-methylcarbamoyl)ethyl]guanosine
tcagcttgggtaggtg

SEQ ID NO: 199 - DNA, 16 bp, synthetic construct
  source 1..16: mol_type = other DNA
  modified_base 1..16: mod_base = OTHER; note = phosphorothioate bond
  modified_base 1: mod_base = OTHER; note = 2'-O-[2-(N-methylcarbamoyl)ethyl]guanosine
  modified_base 2..3: mod_base = OTHER; note = modified LNA monomer with thymine base
  modified_base 4: mod_base = m5c
  modified_base 7: mod_base = m5c
  modified_base 14: mod_base = OTHER; note = modified LNA monomer with adenine base
  modified_base 15: mod_base = OTHER; note = modified LNA monomer with guanine base
  modified_base 16: mod_base = OTHER; note = 2'-O-[2-(N-methylcarbamoyl)ethyl]guanosine
gttcagcttgggtagg

SEQ ID NO: 200 - DNA, 16 bp, synthetic construct
  source 1..16: mol_type = other DNA
  modified_base 1..16: mod_base = OTHER; note = phosphorothioate bond
  modified_base 1: mod_base = OTHER; note = 2'-O-[2-(N-methylcarbamoyl)ethyl]-5-methylcytidine
  modified_base 2: mod_base = OTHER; note = modified LNA monomer with 5-methylcytosine base
  modified_base 3: mod_base = OTHER; note = modified LNA monomer with guanine base
  modified_base 14: mod_base = OTHER; note = modified LNA monomer with guanine base
  modified_base 15: mod_base = OTHER; note = modified LNA monomer with thymine base
  modified_base 16: mod_base = OTHER; note = 2'-O-[2-(N-methylcarbamoyl)ethyl]-5-methylcytidine
ccgtgtagaagaggtc

SEQ ID NO: 201 - DNA, 16 bp, synthetic construct
  source 1..16: mol_type = other DNA
  modified_base 1..16: mod_base = OTHER; note = phosphorothioate bond
  modified_base 1: mod_base = OTHER; note = 2'-O-[2-(N-methylcarbamoyl)ethyl]-5-methylcytidine
  modified_base 2: mod_base = OTHER; note = modified LNA monomer with adenine base
  modified_base 3: mod_base = OTHER; note = modified LNA monomer with thymine base
  modified_base 11: mod_base = m5c
  modified_base 13: mod_base = m5c
  modified_base 14: mod_base = OTHER; note = modified LNA monomer with adenine base
  modified_base 15: mod_base = OTHER; note = modified LNA monomer with thymine base
  modified_base 16: mod_base = OTHER; note = 2'-O-[2-(N-methylcarbamoyl)ethyl]adenosine
cataagaaagctcata

SEQ ID NO: 202 - DNA, 16 bp, synthetic construct
  source 1..16: mol_type = other DNA
  modified_base 1..16: mod_base = OTHER; note = phosphorothioate bond
  modified_base 1: mod_base = OTHER; note = 2'-O-[2-(N-methylcarbamoyl)ethyl]guanosine
  modified_base 2: mod_base = OTHER; note = modified LNA monomer with 5-methylcytosine base
  modified_base 3: mod_base = OTHER; note = modified LNA monomer with adenine base
  modified_base 12: mod_base = m5c
  modified_base 14: mod_base = OTHER; note = modified LNA monomer with 5-methylcytosine base
  modified_base 15: mod_base = OTHER; note = modified LNA monomer with adenine base
  modified_base 16: mod_base = OTHER; note = 2'-O-[2-(N-methylcarbamoyl)ethyl]-5-methyluridine
gcataagaaagctcat

SEQ ID NO: 203 - DNA, 16 bp, synthetic construct
  source 1..16: mol_type = other DNA
  modified_base 1..16: mod_base = OTHER; note = phosphorothioate bond
  modified_base 1: mod_base = OTHER; note = 2'-O-[2-(N-methylcarbamoyl)ethyl]guanosine
  modified_base 2: mod_base = OTHER; note = modified LNA monomer with guanine base
  modified_base 3: mod_base = OTHER; note = modified LNA monomer with 5-methylcytosine base
  modified_base 13: mod_base = m5c
  modified_base 14: mod_base = OTHER; note = modified LNA monomer with thymine base
  modified_base 15: mod_base = OTHER; note = modified LNA monomer with 5-methylcytosine base
  modified_base 16: mod_base = OTHER; note = 2'-O-[2-(N-methylcarbamoyl)ethyl]adenosine
ggcataagaaagctca

SEQ ID NO: 204 - DNA, 16 bp, synthetic construct
  source 1..16: mol_type = other DNA
  modified_base 1..16: mod_base = OTHER; note = phosphorothioate bond
  modified_base 1: mod_base = OTHER; note = 2'-O-[2-(N-methylcarbamoyl)ethyl]guanosine
  modified_base 2..3: mod_base = OTHER; note = modified LNA monomer with guanine base
  modified_base 4: mod_base = m5c
  modified_base 14: mod_base = OTHER; note = modified LNA monomer with 5-methylcytosine base
  modified_base 15: mod_base = OTHER; note = modified LNA monomer with thymine base
  modified_base 16: mod_base = OTHER; note = 2'-O-[2-(N-methylcarbamoyl)ethyl]-5-methylcytidine
gggcataagaaagctc

SEQ ID NO: 205 - DNA, 16 bp, synthetic construct
  source 1..16: mol_type = other DNA
  modified_base 1..16: mod_base = OTHER; note = phosphorothioate bond
  modified_base 1: mod_base = OTHER; note = 2'-O-[2-(N-methylcarbamoyl)ethyl]-5-methylcytidine
  modified_base 2..3: mod_base = OTHER; note = modified LNA monomer with guanine base
  modified_base 5: mod_base = m5c
  modified_base 14: mod_base = OTHER; note = modified LNA monomer with guanine base
  modified_base 15: mod_base = OTHER; note = modified LNA monomer with 5-methylcytosine base
  modified_base 16: mod_base = OTHER; note = 2'-O-[2-(N-methylcarbamoyl)ethyl]-5-methyluridine
cgggcataagaaagct

SEQ ID NO: 206 - DNA, 16 bp, synthetic construct
  source 1..16: mol_type = other DNA
  modified_base 1..16: mod_base = OTHER; note = phosphorothioate bond
  modified_base 1: mod_base = OTHER; note = 2'-O-[2-(N-methylcarbamoyl)ethyl]-5-methylcytidine
  modified_base 2..3: mod_base = OTHER; note = modified LNA monomer with 5-methylcytosine base
  modified_base 7: mod_base = m5c
  modified_base 14..15: mod_base = OTHER; note = modified LNA monomer with adenine base
  modified_base 16: mod_base = OTHER; note = 2'-O-[2-(N-methylcarbamoyl)ethyl]guanosine
cccgggcataagaaag

SEQ ID NO: 207 - DNA, 16 bp, synthetic construct
  source 1..16: mol_type = other DNA
  modified_base 1..16: mod_base = OTHER; note = phosphorothioate bond
  modified_base 1: mod_base = OTHER; note = 2'-O-[2-(N-methylcarbamoyl)ethyl]-5-methylcytidine
  modified_base 2: mod_base = OTHER; note = modified LNA monomer with adenine base
  modified_base 3: mod_base = OTHER; note = modified LNA monomer with guanine base
  modified_base 4: mod_base = m5c
  modified_base 7: mod_base = m5c
  modified_base 9..10: mod_base = m5c
  modified_base 12: mod_base = m5c
  modified_base 14: mod_base = OTHER; note = modified LNA monomer with thymine base
  modified_base 15: mod_base = OTHER; note = modified LNA monomer with guanine base
  modified_base 16: mod_base = OTHER; note = 2'-O-[2-(N-methylcarbamoyl)ethyl]-5-methylcytidine
cagctgctccacatgc

SEQ ID NO: 208 - DNA, 16 bp, synthetic construct
  source 1..16: mol_type = other DNA
  modified_base 1..16: mod_base = OTHER; note = phosphorothioate bond
  modified_base 1: mod_base = OTHER; note = 2'-O-[2-(N-methylcarbamoyl)ethyl]-5-methylcytidine
  modified_base 2: mod_base = OTHER; note = modified LNA monomer with adenine base
  modified_base 3: mod_base = OTHER; note = modified LNA monomer with 5-methylcytosine base
  modified_base 4: mod_base = m5c
  modified_base 7: mod_base = m5c
  modified_base 10: mod_base = m5c
  modified_base 12..13: mod_base = m5c
  modified_base 14: mod_base = OTHER; note = modified LNA monomer with adenine base
  modified_base 15: mod_base = OTHER; note = modified LNA monomer with 5-methylcytosine base
  modified_base 16: mod_base = OTHER; note = 2'-O-[2-(N-methylcarbamoyl)ethyl]adenosine
caccagctgctccaca

SEQ ID NO: 209 - DNA, 16 bp, synthetic construct
  source 1..16: mol_type = other DNA
  modified_base 1..16: mod_base = OTHER; note = phosphorothioate bond
  modified_base 1: mod_base = OTHER; note = 2'-O-[2-(N-methylcarbamoyl)ethyl]-5-methylcytidine
  modified_base 2: mod_base = OTHER; note = modified LNA monomer with 5-methylcytosine base
  modified_base 3: mod_base = OTHER; note = modified LNA monomer with adenine base
  modified_base 4..5: mod_base = m5c
  modified_base 8: mod_base = m5c
  modified_base 11: mod_base = m5c
  modified_base 13: mod_base = m5c
  modified_base 14: mod_base = OTHER; note = modified LNA monomer with 5-methylcytosine base
  modified_base 15: mod_base = OTHER; note = modified LNA monomer with adenine base
  modified_base 16: mod_base = OTHER; note = 2'-O-[2-(N-methylcarbamoyl)ethyl]-5-methylcytidine
ccaccagctgctccac

SEQ ID NO: 210 - DNA, 16 bp, synthetic construct
  source 1..16: mol_type = other DNA
  modified_base 1..16: mod_base = OTHER; note = phosphorothioate bond
  modified_base 1: mod_base = OTHER; note = 2'-O-[2-(N-methylcarbamoyl)ethyl]-5-methyluridine
  modified_base 2..3: mod_base = OTHER; note = modified LNA monomer with 5-methylcytosine base
  modified_base 5..6: mod_base = m5c
  modified_base 9: mod_base = m5c
  modified_base 12: mod_base = m5c
  modified_base 14..15: mod_base = OTHER; note = modified LNA monomer with 5-methylcytosine base
  modified_base 16: mod_base = OTHER; note = 2'-O-[2-(N-methylcarbamoyl)ethyl]adenosine
tccaccagctgctcca

SEQ ID NO: 211 - DNA, 16 bp, synthetic construct
  source 1..16: mol_type = other DNA
  modified_base 1..16: mod_base = OTHER; note = phosphorothioate bond
  modified_base 1: mod_base = OTHER; note = 2'-O-[2-(N-methylcarbamoyl)ethyl]guanosine
  modified_base 2..3: mod_base = OTHER; note = modified LNA monomer with adenine base
  modified_base 4: mod_base = m5c
  modified_base 6: mod_base = m5c
  modified_base 10: mod_base = m5c
  modified_base 13: mod_base = m5c
  modified_base 14: mod_base = OTHER; note = modified LNA monomer with adenine base
  modified_base 15: mod_base = OTHER; note = modified LNA monomer with guanine base
  modified_base 16: mod_base = OTHER; note = 2'-O-[2-(N-methylcarbamoyl)ethyl]adenosine
gaacacagacttcaga

SEQ ID NO: 212 - DNA, 16 bp, synthetic construct
  source 1..16: mol_type = other DNA
  modified_base 1..16: mod_base = OTHER; note = phosphorothioate bond
  modified_base 1: mod_base = OTHER; note = 2'-O-[2-(N-methylcarbamoyl)ethyl]adenosine
  modified_base 2..3: mod_base = OTHER; note = modified LNA monomer with adenine base
  modified_base 6..7: mod_base = m5c
  modified_base 9..10: mod_base = m5c
  modified_base 14: mod_base = OTHER; note = modified LNA monomer with guanine base
  modified_base 15: mod_base = OTHER; note = modified LNA monomer with adenine base
  modified_base 16: mod_base = OTHER; note = 2'-O-[2-(N-methylcarbamoyl)ethyl]guanosine
aaagtcctcctgagag

SEQ ID NO: 213 - DNA, 16 bp, synthetic construct
  source 1..16: mol_type = other DNA
  modified_base 1..16: mod_base = OTHER; note = phosphorothioate bond
  modified_base 1: mod_base = OTHER; note = 2'-O-[2-(N-methylcarbamoyl)ethyl]-5-methylcytidine
  modified_base 2..3: mod_base = OTHER; note = modified LNA monomer with adenine base
  modified_base 7..8: mod_base = m5c
  modified_base 10..11: mod_base = m5c
  modified_base 14: mod_base = OTHER; note = modified LNA monomer with adenine base
  modified_base 15: mod_base = OTHER; note = modified LNA monomer with guanine base
  modified_base 16: mod_base = OTHER; note = 2'-O-[2-(N-methylcarbamoyl)ethyl]adenosine
caaagtcctcctgaga

SEQ ID NO: 214 - DNA, 16 bp, synthetic construct
  source 1..16: mol_type = other DNA
  modified_base 1..16: mod_base = OTHER; note = phosphorothioate bond
  modified_base 1: mod_base = OTHER; note = 2'-O-[2-(N-methylcarbamoyl)ethyl]-5-methyluridine
  modified_base 2: mod_base = OTHER; note = modified LNA monomer with 5-methylcytosine base
  modified_base 3: mod_base = OTHER; note = modified LNA monomer with adenine base
  modified_base 8..9: mod_base = m5c
  modified_base 11..12: mod_base = m5c
  modified_base 14: mod_base = OTHER; note = modified LNA monomer with guanine base
  modified_base 15: mod_base = OTHER; note = modified LNA monomer with adenine base
  modified_base 16: mod_base = OTHER; note = 2'-O-[2-(N-methylcarbamoyl)ethyl]guanosine
tcaaagtcctcctgag

SEQ ID NO: 215 - DNA, 16 bp, synthetic construct
  source 1..16: mol_type = other DNA
  modified_base 1..16: mod_base = OTHER; note = phosphorothioate bond
  modified_base 1: mod_base = OTHER; note = 2'-O-[2-(N-methylcarbamoyl)ethyl]-5-methylcytidine
  modified_base 2: mod_base = OTHER; note = modified LNA monomer with thymine base
  modified_base 3: mod_base = OTHER; note = modified LNA monomer with 5-methylcytosine base
  modified_base 9..10: mod_base = m5c
  modified_base 12..13: mod_base = m5c
  modified_base 14: mod_base = OTHER; note = modified LNA monomer with thymine base
  modified_base 15: mod_base = OTHER; note = modified LNA monomer with guanine base
  modified_base 16: mod_base = OTHER; note = 2'-O-[2-(N-methylcarbamoyl)ethyl]adenosine
ctcaaagtcctcctga

SEQ ID NO: 216 - DNA, 16 bp, synthetic construct
  source 1..16: mol_type = other DNA
  modified_base 1..16: mod_base = OTHER; note = phosphorothioate bond
  modified_base 1: mod_base = OTHER; note = 2'-O-[2-(N-methylcarbamoyl)ethyl]guanosine
  modified_base 2: mod_base = OTHER; note = modified LNA monomer with 5-methylcytosine base
  modified_base 3: mod_base = OTHER; note = modified LNA monomer with thymine base
  modified_base 4: mod_base = m5c
  modified_base 10..11: mod_base = m5c
  modified_base 13: mod_base = m5c
  modified_base 14: mod_base = OTHER; note = modified LNA monomer with 5-methylcytosine base
  modified_base 15: mod_base = OTHER; note = modified LNA monomer with thymine base
  modified_base 16: mod_base = OTHER; note = 2'-O-[2-(N-methylcarbamoyl)ethyl]guanosine
gctcaaagtcctcctg

SEQ ID NO: 217 - DNA, 16 bp, synthetic construct
  source 1..16: mol_type = other DNA
  modified_base 1..16: mod_base = OTHER; note = phosphorothioate bond
  modified_base 1: mod_base = OTHER; note = 2'-O-[2-(N-methylcarbamoyl)ethyl]-5-methyluridine
  modified_base 2: mod_base = OTHER; note = modified LNA monomer with 5-methylcytosine base
  modified_base 3: mod_base = OTHER; note = modified LNA monomer with guanine base
  modified_base 4: mod_base = m5c
  modified_base 6: mod_base = m5c
  modified_base 12..13: mod_base = m5c
  modified_base 14: mod_base = OTHER; note = modified LNA monomer with thymine base
  modified_base 15: mod_base = OTHER; note = modified LNA monomer with 5-methylcytosine base
  modified_base 16: mod_base = OTHER; note = 2'-O-[2-(N-methylcarbamoyl)ethyl]-5-methylcytidine
tcgctcaaagtcctcc

SEQ ID NO: 218 - DNA, 16 bp, synthetic construct
  source 1..16: mol_type = other DNA
  modified_base 1..16: mod_base = OTHER; note = phosphorothioate bond
  modified_base 1: mod_base = OTHER; note = 2'-O-[2-(N-methylcarbamoyl)ethyl]guanosine
  modified_base 2: mod_base = OTHER; note = modified LNA monomer with thymine base
  modified_base 3: mod_base = OTHER; note = modified LNA monomer with 5-methylcytosine base
  modified_base 5: mod_base = m5c
  modified_base 7: mod_base = m5c
  modified_base 13: mod_base = m5c
  modified_base 14: mod_base = OTHER; note = modified LNA monomer with 5-methylcytosine base
  modified_base 15: mod_base = OTHER; note = modified LNA monomer with thymine base
  modified_base 16: mod_base = OTHER; note = 2'-O-[2-(N-methylcarbamoyl)ethyl]-5-methylcytidine
gtcgctcaaagtcctc

SEQ ID NO: 219 - DNA, 16 bp, synthetic construct
  source 1..16: mol_type = other DNA
  modified_base 1..16: mod_base = OTHER; note = phosphorothioate bond
  modified_base 1: mod_base = OTHER; note = 2'-O-[2-(N-methylcarbamoyl)ethyl]-5-methylcytidine
  modified_base 2: mod_base = OTHER; note = modified LNA monomer with thymine base
  modified_base 3: mod_base = OTHER; note = modified LNA monomer with 5-methylcytosine base
  modified_base 5: mod_base = m5c
  modified_base 8: mod_base = m5c
  modified_base 14: mod_base = OTHER; note = modified LNA monomer with guanine base
  modified_base 15: mod_base = OTHER; note = modified LNA monomer with adenine base
  modified_base 16: mod_base = OTHER; note = 2'-O-[2-(N-methylcarbamoyl)ethyl]-5-methyluridine
ctctctgctgaaggat

SEQ ID NO: 220 - DNA, 16 bp, synthetic construct
  source 1..16: mol_type = other DNA
  modified_base 1..16: mod_base = OTHER; note = phosphorothioate bond
  modified_base 1: mod_base = OTHER; note = 2'-O-[2-(N-methylcarbamoyl)ethyl]-5-methyluridine
  modified_base 2..3: mod_base = OTHER; note = modified LNA monomer with guanine base
  modified_base 12: mod_base = m5c
  modified_base 14..15: mod_base = OTHER; note = modified LNA monomer with guanine base
  modified_base 16: mod_base = OTHER; note = 2'-O-[2-(N-methylcarbamoyl)ethyl]adenosine
tggaaggtgtgcagga

SEQ ID NO: 221 - DNA, 16 bp, synthetic construct
  source 1..16: mol_type = other DNA
  modified_base 1..16: mod_base = OTHER; note = phosphorothioate bond
  modified_base 1: mod_base = OTHER; note = 2'-O-[2-(N-methylcarbamoyl)ethyl]guanosine
  modified_base 2: mod_base = OTHER; note = modified LNA monomer with thymine base
  modified_base 3: mod_base = OTHER; note = modified LNA monomer with guanine base
  modified_base 5..6: mod_base = m5c
  modified_base 8: mod_base = m5c
  modified_base 14: mod_base = OTHER; note = modified LNA monomer with adenine base
  modified_base 15: mod_base = OTHER; note = modified LNA monomer with guanine base
  modified_base 16: mod_base = OTHER; note = 2'-O-[2-(N-methylcarbamoyl)ethyl]guanosine
gtgacctcatggaagg

SEQ ID NO: 222 - DNA, 16 bp, synthetic construct
  source 1..16: mol_type = other DNA
  modified_base 1: mod_base = OTHER; note = 2'-O-[2-(N-methylcarbamoyl)ethyl]guanosine
  modified_base 1..16: mod_base = OTHER; note = phosphorothioate bond
  modified_base 2: mod_base = OTHER; note = modified LNA monomer with guanine base
  modified_base 3: mod_base = OTHER; note = modified LNA monomer with thymine base
  modified_base 6..7: mod_base = m5c
  modified_base 9: mod_base = m5c
  modified_base 14..15: mod_base = OTHER; note = modified LNA monomer with adenine base
  modified_base 16: mod_base = OTHER; note = 2'-O-[2-(N-methylcarbamoyl)ethyl]guanosine
ggtgacctcatggaag

SEQ ID NO: 223 - DNA, 16 bp, synthetic construct
  source 1..16: mol_type = other DNA
  modified_base 1..16: mod_base = OTHER; note = phosphorothioate bond
  modified_base 1: mod_base = OTHER; note = 2'-O-[2-(N-methylcarbamoyl)ethyl]adenosine
  modified_base 2: mod_base = OTHER; note = modified LNA monomer with adenine base
  modified_base 3: mod_base = OTHER; note = modified LNA monomer with guanine base
  modified_base 8..9: mod_base = m5c
  modified_base 11: mod_base = m5c
  modified_base 14..15: mod_base = OTHER; note = modified LNA monomer with guanine base
  modified_base 16: mod_base = OTHER; note = 2'-O-[2-(N-methylcarbamoyl)ethyl]adenosine
aaggtgacctcatgga

SEQ ID NO: 224 - DNA, 16 bp, synthetic construct
  source 1..16: mol_type = other DNA
  modified_base 1..16: mod_base = OTHER; note = phosphorothioate bond
  modified_base 1: mod_base = OTHER; note = 2'-O-[2-(N-methylcarbamoyl)ethyl]guanosine
  modified_base 2..3: mod_base = OTHER; note = modified LNA monomer with adenine base
  modified_base 9..10: mod_base = m5c
  modified_base 14: mod_base = OTHER; note = modified LNA monomer with thymine base
  modified_base 12: mod_base = m5c
  modified_base 15: mod_base = OTHER; note = modified LNA monomer with guanine base
  modified_base 16: mod_base = OTHER; note = 2'-O-[2-(N-methylcarbamoyl)ethyl]guanosine
gaaggtgacctcatgg

SEQ ID NO: 225 - DNA, 16 bp, synthetic construct
  source 1..16: mol_type = other DNA
  modified_base 1..16: mod_base = OTHER; note = phosphorothioate bond
  modified_base 1: mod_base = OTHER; note = 2'-O-[2-(N-methylcarbamoyl)ethyl]guanosine
  modified_base 2: mod_base = OTHER; note = modified LNA monomer with guanine base
  modified_base 3: mod_base = OTHER; note = modified LNA monomer with adenine base
  modified_base 10..11: mod_base = m5c
  modified_base 13: mod_base = m5c
  modified_base 14: mod_base = OTHER; note = modified LNA monomer with adenine base
  modified_base 15: mod_base = OTHER; note = modified LNA monomer with thymine base
  modified_base 16: mod_base = OTHER; note = 2'-O-[2-(N-methylcarbamoyl)ethyl]guanosine
ggaaggtgacctcatg

SEQ ID NO: 226 - DNA, 16 bp, synthetic construct
  source 1..16: mol_type = other DNA
  modified_base 1..16: mod_base = OTHER; note = phosphorothioate bond
  modified_base 1: mod_base = OTHER; note = 2'-O-[2-(N-methylcarbamoyl)ethyl]-5-methylcytidine
  modified_base 2..3: mod_base = OTHER; note = modified LNA monomer with guanine base
  modified_base 11..12: mod_base = m5c
  modified_base 14: mod_base = OTHER; note = modified LNA monomer with 5-methylcytosine base
  modified_base 15: mod_base = OTHER; note = modified LNA monomer with adenine base
  modified_base 16: mod_base = OTHER; note = 2'-O-[2-(N-methylcarbamoyl)ethyl]-5-methyluridine
cggaaggtgacctcat

SEQ ID NO: 227 - DNA, 16 bp, synthetic construct
  source 1..16: mol_type = other DNA
  modified_base 1..16: mod_base = OTHER; note = phosphorothioate bond
  modified_base 1: mod_base = OTHER; note = 2'-O-[2-(N-methylcarbamoyl)ethyl]-5-methyluridine
  modified_base 2: mod_base = OTHER; note = modified LNA monomer with 5-methylcytosine base
  modified_base 3: mod_base = OTHER; note = modified LNA monomer with guanine base
  modified_base 12..13: mod_base = m5c
  modified_base 14: mod_base = OTHER; note = modified LNA monomer with thymine base
  modified_base 15: mod_base = OTHER; note = modified LNA monomer with 5-methylcytosine base
  modified_base 16: mod_base = OTHER; note = 2'-O-[2-(N-methylcarbamoyl)ethyl]adenosine
tcggaaggtgacctca

SEQ ID NO: 228 - DNA, 16 bp, synthetic construct
  source 1..16: mol_type = other DNA
  modified_base 1..16: mod_base = OTHER; note = phosphorothioate bond
  modified_base 1: mod_base = OTHER; note = 2'-O-[2-(N-methylcarbamoyl)ethyl]-5-methyluridine
  modified_base 2: mod_base = OTHER; note = modified LNA monomer with adenine base
  modified_base 3: mod_base = OTHER; note = modified LNA monomer with guanine base
  modified_base 14: mod_base = OTHER; note = modified LNA monomer with guanine base
  modified_base 15: mod_base = OTHER; note = modified LNA monomer with adenine base
  modified_base 16: mod_base = OTHER; note = 2'-O-[2-(N-methylcarbamoyl)ethyl]-5-methyluridine
tagagatttggaggat

SEQ ID NO: 229 - DNA, 16 bp, synthetic construct
  source 1..16: mol_type = other DNA
  modified_base 1..16: mod_base = OTHER; note = phosphorothioate bond
  modified_base 1: mod_base = OTHER; note = 2'-O-[2-(N-methylcarbamoyl)ethyl]-5-methyluridine
  modified_base 2: mod_base = OTHER; note = modified LNA monomer with guanine base
  modified_base 3: mod_base = OTHER; note = modified LNA monomer with 5-methylcytosine base
  modified_base 11: mod_base = m5c
  modified_base 13: mod_base = m5c
  modified_base 14..15: mod_base = OTHER; note = modified LNA monomer with 5-methylcytosine base
  modified_base 16: mod_base = OTHER; note = 2'-O-[2-(N-methylcarbamoyl)ethyl]-5-methylcytidine
tgcttggtgacacccc

SEQ ID NO: 230 - DNA, 16 bp, synthetic construct
  source 1..16: mol_type = other DNA
  modified_base 1..16: mod_base = OTHER; note = phosphorothioate bond
  modified_base 1: mod_base = OTHER; note = 2'-O-[2-(N-methylcarbamoyl)ethyl]-5-methyluridine
  modified_base 2: mod_base = OTHER; note = modified LNA monomer with thymine base
  modified_base 3: mod_base = OTHER; note = modified LNA monomer with guanine base
  modified_base 4: mod_base = m5c
  modified_base 12: mod_base = m5c
  modified_base 14..15: mod_base = OTHER; note = modified LNA monomer with 5-methylcytosine base
  modified_base 16: mod_base = OTHER; note = 2'-O-[2-(N-methylcarbamoyl)ethyl]-5-methylcytidine
ttgcttggtgacaccc

SEQ ID NO: 231 - DNA, 16 bp, synthetic construct
  source 1..16: mol_type = other DNA
  modified_base 1..16: mod_base = OTHER; note = phosphorothioate bond
  modified_base 1: mod_base = OTHER; note = 2'-O-[2-(N-methylcarbamoyl)ethyl]-5-methylcytidine
  modified_base 2..3: mod_base = OTHER; note = modified LNA monomer with thymine base
  modified_base 5: mod_base = m5c
  modified_base 13: mod_base = m5c
  modified_base 14: mod_base = OTHER; note = modified LNA monomer with adenine base
  modified_base 15: mod_base = OTHER; note = modified LNA monomer with 5-methylcytosine base
  modified_base 16: mod_base = OTHER; note = 2'-O-[2-(N-methylcarbamoyl)ethyl]-5-methylcytidine
cttgcttggtgacacc

SEQ ID NO: 232 - DNA, 16 bp, synthetic construct
  source 1..16: mol_type = other DNA
  modified_base 1..16: mod_base = OTHER; note = phosphorothioate bond
  modified_base 1: mod_base = OTHER; note = 2'-O-[2-(N-methylcarbamoyl)ethyl]-5-methylcytidine
  modified_base 2: mod_base = OTHER; note = modified LNA monomer with 5-methylcytosine base
  modified_base 3: mod_base = OTHER; note = modified LNA monomer with thymine base
  modified_base 6: mod_base = m5c
  modified_base 14: mod_base = OTHER; note = modified LNA monomer with 5-methylcytosine base
  modified_base 15: mod_base = OTHER; note = modified LNA monomer with adenine base
  modified_base 16: mod_base = OTHER; note = 2'-O-[2-(N-methylcarbamoyl)ethyl]-5-methylcytidine
ccttgcttggtgacac

SEQ ID NO: 233 - DNA, 16 bp, synthetic construct
  source 1..16: mol_type = other DNA
  modified_base 1..16: mod_base = OTHER; note = phosphorothioate bond
  modified_base 1: mod_base = OTHER; note = 2'-O-[2-(N-methylcarbamoyl)ethyl]guanosine
  modified_base 2..3: mod_base = OTHER; note = modified LNA monomer with 5-methylcytosine base
  modified_base 7: mod_base = m5c
  modified_base 14: mod_base = OTHER; note = modified LNA monomer with adenine base
  modified_base 15: mod_base = OTHER; note = modified LNA monomer with 5-methylcytosine base
  modified_base 16: mod_base = OTHER; note = 2'-O-[2-(N-methylcarbamoyl)ethyl]adenosine
gccttgcttggtgaca

SEQ ID NO: 234 - DNA, 16 bp, synthetic construct
  source 1..16: mol_type = other DNA
  modified_base 1..16: mod_base = OTHER; note = phosphorothioate bond
  modified_base 1: mod_base = OTHER; note = 2'-O-[2-(N-methylcarbamoyl)ethyl]-5-methyluridine
  modified_base 2: mod_base = OTHER; note = modified LNA monomer with adenine base
  modified_base 3: mod_base = OTHER; note = modified LNA monomer with guanine base
  modified_base 4..5: mod_base = m5c
  modified_base 9: mod_base = m5c
  modified_base 14: mod_base = OTHER; note = modified LNA monomer with thymine base
  modified_base 15: mod_base = OTHER; note = modified LNA monomer with guanine base
  modified_base 16: mod_base = OTHER; note = 2'-O-[2-(N-methylcarbamoyl)ethyl]adenosine
tagccttgcttggtga

SEQ ID NO: 235 - DNA, 16 bp, synthetic construct
  source 1..16: mol_type = other DNA
  modified_base 1..16: mod_base = OTHER; note = phosphorothioate bond
  modified_base 1: mod_base = OTHER; note = 2'-O-[2-(N-methylcarbamoyl)ethyl]guanosine
  modified_base 2: mod_base = OTHER; note = modified LNA monomer with thymine base
  modified_base 3: mod_base = OTHER; note = modified LNA monomer with adenine base
  modified_base 5..6: mod_base = m5c
  modified_base 10: mod_base = m5c
  modified_base 14: mod_base = OTHER; note = modified LNA monomer with guanine base
  modified_base 15: mod_base = OTHER; note = modified LNA monomer with thymine base
  modified_base 16: mod_base = OTHER; note = 2'-O-[2-(N-methylcarbamoyl)ethyl]guanosine
gtagccttgcttggtg

SEQ ID NO: 236 - DNA, 16 bp, synthetic construct
  source 1..16: mol_type = other DNA
  modified_base 1..16: mod_base = OTHER; note = phosphorothioate bond
  modified_base 1: mod_base = OTHER; note = 2'-O-[2-(N-methylcarbamoyl)ethyl]guanosine
  modified_base 2: mod_base = OTHER; note = modified LNA monomer with guanine base
  modified_base 3: mod_base = OTHER; note = modified LNA monomer with thymine base
  modified_base 6..7: mod_base = m5c
  modified_base 11: mod_base = m5c
  modified_base 14..15: mod_base = OTHER; note = modified LNA monomer with guanine base
  modified_base 16: mod_base = OTHER; note = 2'-O-[2-(N-methylcarbamoyl)ethyl]-5-methyluridine
ggtagccttgcttggt

SEQ ID NO: 237 - DNA, 16 bp, synthetic construct
  source 1..16: mol_type = other DNA
  modified_base 1..16: mod_base = OTHER; note = phosphorothioate bond
  modified_base 1: mod_base = OTHER; note = 2'-O-[2-(N-methylcarbamoyl)ethyl]-5-methylcytidine
  modified_base 2..3: mod_base = OTHER; note = modified LNA monomer with guanine base
  modified_base 7..8: mod_base = m5c
  modified_base 12: mod_base = m5c
  modified_base 14: mod_base = OTHER; note = modified LNA monomer with thymine base
  modified_base 15: mod_base = OTHER; note = modified LNA monomer with guanine base
  modified_base 16: mod_base = OTHER; note = 2'-O-[2-(N-methylcarbamoyl)ethyl]guanosine
cggtagccttgcttgg

SEQ ID NO: 238 - DNA, 16 bp, synthetic construct
  source 1..16: mol_type = other DNA
  modified_base 1..16: mod_base = OTHER; note = phosphorothioate bond
  modified_base 1: mod_base = OTHER; note = 2'-O-[2-(N-methylcarbamoyl)ethyl]guanosine
  modified_base 2: mod_base = OTHER; note = modified LNA monomer with 5-methylcytosine base
  modified_base 3: mod_base = OTHER; note = modified LNA monomer with guanine base
  modified_base 8..9: mod_base = m5c
  modified_base 13: mod_base = m5c
  modified_base 14..15: mod_base = OTHER; note = modified LNA monomer with thymine base
  modified_base 16: mod_base = OTHER; note = 2'-O-[2-(N-methylcarbamoyl)ethyl]guanosine
gcggtagccttgcttg

SEQ ID NO: 239 - DNA, 16 bp, synthetic construct
  source 1..16: mol_type = other DNA
  modified_base 1..16: mod_base = OTHER; note = phosphorothioate bond
  modified_base 1: mod_base = OTHER; note = 2'-O-[2-(N-methylcarbamoyl)ethyl]-5-methylcytidine
  modified_base 2: mod_base = OTHER; note = modified LNA monomer with thymine base
  modified_base 3: mod_base = OTHER; note = modified LNA monomer with adenine base
  modified_base 7: mod_base = m5c
  modified_base 11..12: mod_base = m5c
  modified_base 14: mod_base = OTHER; note = modified LNA monomer with 5-methylcytosine base
  modified_base 15: mod_base = OTHER; note = modified LNA monomer with adenine base
  modified_base 16: mod_base = OTHER; note = 2'-O-[2-(N-methylcarbamoyl)ethyl]guanosine
ctaggtcttaccacag

SEQ ID NO: 240 - DNA, 16 bp, synthetic construct
  source 1..16: mol_type = other DNA
  modified_base 1..16: mod_base = OTHER; note = phosphorothioate bond
  modified_base 1: mod_base = OTHER; note = 2'-O-[2-(N-methylcarbamoyl)ethyl]-5-methylcytidine
  modified_base 2: mod_base = OTHER; note = modified LNA monomer with thymine base
  modified_base 3: mod_base = OTHER; note = modified LNA monomer with guanine base
  modified_base 7..8: mod_base = m5c
  modified_base 12: mod_base = m5c
  modified_base 14: mod_base = OTHER; note = modified LNA monomer with thymine base
  modified_base 15: mod_base = OTHER; note = modified LNA monomer with guanine base
  modified_base 16: mod_base = OTHER; note = 2'-O-[2-(N-methylcarbamoyl)ethyl]guanosine
ctgggtccaggcatgg

SEQ ID NO: 241 - DNA, 16 bp, synthetic construct
  source 1..16: mol_type = other DNA
  modified_base 1..16: mod_base = OTHER; note = phosphorothioate bond
  modified_base 1: mod_base = OTHER; note = 2'-O-[2-(N-methylcarbamoyl)ethyl]adenosine
  modified_base 2..3: mod_base = OTHER; note = modified LNA monomer with thymine base
  modified_base 4: mod_base = m5c
  modified_base 8: mod_base = m5c
  modified_base 14..15: mod_base = OTHER; note = modified LNA monomer with 5-methylcytosine base
  modified_base 16: mod_base = OTHER; note = 2'-O-[2-(N-methylcarbamoyl)ethyl]adenosine
attcagtctgggtcca

SEQ ID NO: 242 - DNA, 16 bp, synthetic construct
  source 1..16: mol_type = other DNA
  modified_base 1..16: mod_base = OTHER; note = phosphorothioate bond
  modified_base 1: mod_base = OTHER; note = 2'-O-[2-(N-methylcarbamoyl)ethyl]guanosine
  modified_base 2: mod_base = OTHER; note = modified LNA monomer with adenine base
  modified_base 3: mod_base = OTHER; note = modified LNA monomer with thymine base
  modified_base 5: mod_base = m5c
  modified_base 9: mod_base = m5c
  modified_base 14: mod_base = OTHER; note = modified LNA monomer with thymine base
  modified_base 15: mod_base = OTHER; note = modified LNA monomer with 5-methylcytosine base
  modified_base 16: mod_base = OTHER; note = 2'-O-[2-(N-methylcarbamoyl)ethyl]-5-methylcytidine
gattcagtctgggtcc

SEQ ID NO: 243 - DNA, 16 bp, synthetic construct
  source 1..16: mol_type = other DNA
  modified_base 1..16: mod_base = OTHER; note = phosphorothioate bond
  modified_base 1: mod_base = OTHER; note = 2'-O-[2-(N-methylcarbamoyl)ethyl]-5-methyluridine
  modified_base 2..3: mod_base = OTHER; note = modified LNA monomer with guanine base
  modified_base 4..5: mod_base = m5c
  modified_base 11: mod_base = m5c
  modified_base 14: mod_base = OTHER; note = modified LNA monomer with guanine base
  modified_base 15: mod_base = OTHER; note = modified LNA monomer with 5-methylcytosine base
  modified_base 16: mod_base = OTHER; note = 2'-O-[2-(N-methylcarbamoyl)ethyl]-5-methyluridine
tggccttattcttgct

SEQ ID NO: 244 - DNA, 16 bp, synthetic construct
  source 1..16: mol_type = other DNA
  modified_base 1..16: mod_base = OTHER; note = phosphorothioate bond
  modified_base 1: mod_base = OTHER; note = 2'-O-[2-(N-methylcarbamoyl)ethyl]-5-methylcytidine
  modified_base 2: mod_base = OTHER; note = modified LNA monomer with adenine base
  modified_base 3: mod_base = OTHER; note = modified LNA monomer with guanine base
  modified_base 14: mod_base = OTHER; note = modified LNA monomer with guanine base
  modified_base 15: mod_base = OTHER; note = modified LNA monomer with thymine base
  modified_base 16: mod_base = OTHER; note = 2'-O-[2-(N-methylcarbamoyl)ethyl]-5-methyluridine
caggggtgttggggtt

SEQ ID NO: 245 - DNA, 16 bp, synthetic construct
  source 1..16: mol_type = other DNA
  modified_base 1..16: mod_base = OTHER; note = phosphorothioate bond
  modified_base 1: mod_base = OTHER; note = modified LNA monomer with guanine base
  modified_base 2: mod_base = OTHER; note = modified LNA monomer with thymine base
  modified_base 3: mod_base = OTHER; note = 2'-O-[2-(N-methylcarbamoyl)ethyl]guanosine
  modified_base 12: mod_base = m5c
  modified_base 14: mod_base = OTHER; note = 2'-O-[2-(N-methylcarbamoyl)ethyl]guanosine
  modified_base 15: mod_base = OTHER; note = modified LNA monomer with 5-methylcytosine base
  modified_base 16: mod_base = OTHER; note = modified LNA monomer with adenine base
gtgttgaaattctgca

SEQ ID NO: 246 - DNA, 16 bp, synthetic construct
  source 1..16: mol_type = other DNA
  modified_base 1..16: mod_base = OTHER; note = phosphorothioate bond
  modified_base 1..2: mod_base = OTHER; note = modified LNA monomer with guanine base
  modified_base 3: mod_base = OTHER; note = 2'-O-[2-(N-methylcarbamoyl)ethyl]guanosine
  modified_base 7..8: mod_base = m5c
  modified_base 14: mod_base = OTHER; note = 2'-O-[2-(N-methylcarbamoyl)ethyl]-5-methyluridine
  modified_base 15: mod_base = OTHER; note = modified LNA monomer with 5-methylcytosine base
  modified_base 16: mod_base = OTHER; note = modified LNA monomer with thymine base
gggagtccttgagtct

SEQ ID NO: 247 - DNA, 16 bp, synthetic construct
  source 1..16: mol_type = other DNA
  modified_base 1..16: mod_base = OTHER; note = phosphorothioate bond
  modified_base 1..2: mod_base = OTHER; note = modified LNA monomer with thymine base
  modified_base 3: mod_base = OTHER; note = 2'-O-[2-(N-methylcarbamoyl)ethyl]-5-methylcytidine
  modified_base 13: mod_base = m5c
  modified_base 14: mod_base = OTHER; note = 2'-O-[2-(N-methylcarbamoyl)ethyl]-5-methylcytidine
  modified_base 15: mod_base = OTHER; note = modified LNA monomer with thymine base
  modified_base 16: mod_base = OTHER; note = modified LNA monomer with 5-methylcytosine base
ttcggaaggtgacctc

SEQ ID NO: 248 - DNA, 16 bp, synthetic construct
  source 1..16: mol_type = other DNA
  modified_base 1..16: mod_base = OTHER; note = phosphorothioate bond
  modified_base 1..2: mod_base = OTHER; note = modified LNA monomer with guanine base
  modified_base 3: mod_base = OTHER; note = 2'-O-[2-(N-methylcarbamoyl)ethyl]adenosine
  modified_base 6: mod_base = m5c
  modified_base 10: mod_base = m5c
  modified_base 14: mod_base = OTHER; note = 2'-O-[2-(N-methylcarbamoyl)ethyl]guanosine
  modified_base 15: mod_base = OTHER; note = modified LNA monomer with thymine base
  modified_base 16: mod_base = OTHER; note = modified LNA monomer with 5-methylcytosine base
ggattcagtctgggtc

SEQ ID NO: 249 - DNA, 16 bp, synthetic construct
  source 1..16: mol_type = other DNA
  modified_base 1..16: mod_base = OTHER; note = phosphorothioate bond
  modified_base 1: mod_base = OTHER; note = modified LNA monomer with 5-methylcytosine base
  modified_base 2: mod_base = OTHER; note = modified LNA monomer with guanine base
  modified_base 3: mod_base = OTHER; note = 2'-O-[2-(N-methylcarbamoyl)ethyl]-5-methyluridine
  modified_base 13: mod_base = m5c
  modified_base 14: mod_base = OTHER; note = 2'-O-[2-(N-methylcarbamoyl)ethyl]-5-methyluridine
  modified_base 15: mod_base = OTHER; note = modified LNA monomer with guanine base
  modified_base 16: mod_base = OTHER; note = modified LNA monomer with 5-methylcytosine base
cgtgttgaaattctgc

SEQ ID NO: 250 - DNA, 16 bp, synthetic construct
  source 1..16: mol_type = other DNA
  modified_base 1..16: mod_base = OTHER; note = phosphorothioate bond
  modified_base 1: mod_base = OTHER; note = modified LNA monomer with guanine base
  modified_base 2: mod_base = OTHER; note = modified LNA monomer with 5-methylcytosine base
  modified_base 3: mod_base = OTHER; note = 2'-O-[2-(N-methylcarbamoyl)ethyl]guanosine
  modified_base 14: mod_base = OTHER; note = 2'-O-[2-(N-methylcarbamoyl)ethyl]-5-methylcytidine
  modified_base 15: mod_base = OTHER; note = modified LNA monomer with thymine base
  modified_base 16: mod_base = OTHER; note = modified LNA monomer with guanine base
gcgtgttgaaattctg

SEQ ID NO: 251 - DNA, 16 bp, synthetic construct
  source 1..16: mol_type = other DNA
  modified_base 1..16: mod_base = OTHER; note = phosphorothioate bond
  modified_base 1: mod_base = OTHER; note = modified LNA monomer with guanine base
  modified_base 2: mod_base = OTHER; note = modified LNA monomer with adenine base
  modified_base 3: mod_base = OTHER; note = 2'-O-[2-(N-methylcarbamoyl)ethyl]guanosine
  modified_base 5..6: mod_base = m5c
  modified_base 13: mod_base = m5c
  modified_base 14: mod_base = OTHER; note = 2'-O-[2-(N-methylcarbamoyl)ethyl]-5-methyluridine
  modified_base 15..16: mod_base = OTHER; note = modified LNA monomer with guanine base
gagtccttgagtctgg

SEQ ID NO: 252 - DNA, 16 bp, synthetic construct
  source 1..16: mol_type = other DNA
  modified_base 1..16: mod_base = OTHER; note = phosphorothioate bond
  modified_base 1..2: mod_base = OTHER; note = modified LNA monomer with guanine base
  modified_base 3: mod_base = OTHER; note = 2'-O-[2-(N-methylcarbamoyl)ethyl]adenosine
  modified_base 6..7: mod_base = m5c
  modified_base 14: mod_base = OTHER; note = 2'-O-[2-(N-methylcarbamoyl)ethyl]-5-methylcytidine
  modified_base 15: mod_base = OTHER; note = modified LNA monomer with thymine base
  modified_base 16: mod_base = OTHER; note = modified LNA monomer with guanine base
ggagtccttgagtctg

SEQ ID NO: 253 - DNA, 16 bp, synthetic construct
  source 1..16: mol_type = other DNA
  modified_base 1..16: mod_base = OTHER; note = phosphorothioate bond
  modified_base 1: mod_base = OTHER; note = modified LNA monomer with thymine base
  modified_base 2: mod_base = OTHER; note = modified LNA monomer with guanine base
  modified_base 3: mod_base = OTHER; note = 2'-O-[2-(N-methylcarbamoyl)ethyl]guanosine
  modified_base 8..9: mod_base = m5c
  modified_base 14: mod_base = OTHER; note = 2'-O-[2-(N-methylcarbamoyl)ethyl]guanosine
  modified_base 15: mod_base = OTHER; note = modified LNA monomer with thymine base
  modified_base 16: mod_base = OTHER; note = modified LNA monomer with 5-methylcytosine base
tgggagtccttgagtc

SEQ ID NO: 254 - DNA, 16 bp, synthetic construct
  source 1..16: mol_type = other DNA
  modified_base 1..16: mod_base = OTHER; note = phosphorothioate bond
  modified_base 1: mod_base = OTHER; note = modified LNA monomer with guanine base
  modified_base 2: mod_base = OTHER; note = modified LNA monomer with thymine base
  modified_base 3: mod_base = OTHER; note = 2'-O-[2-(N-methylcarbamoyl)ethyl]-5-methyluridine
  modified_base 4: mod_base = m5c
  modified_base 7: mod_base = m5c
  modified_base 14: mod_base = OTHER; note = 2'-O-[2-(N-methylcarbamoyl)ethyl]adenosine
  modified_base 15..16: mod_base = OTHER; note = modified LNA monomer with guanine base
gttcagcttgggtagg

SEQ ID NO: 255 - DNA, 16 bp, synthetic construct
  source 1..16: mol_type = other DNA
  modified_base 1..16: mod_base = OTHER; note = phosphorothioate bond
  modified_base 1..2: mod_base = OTHER; note = modified LNA monomer with 5-methylcytosine base
  modified_base 3: mod_base = OTHER; note = 2'-O-[2-(N-methylcarbamoyl)ethyl]guanosine
  modified_base 14: mod_base = OTHER; note = 2'-O-[2-(N-methylcarbamoyl)ethyl]guanosine
  modified_base 15: mod_base = OTHER; note = modified LNA monomer with thymine base
  modified_base 16: mod_base = OTHER; note = modified LNA monomer with 5-methylcytosine base
ccgtgtagaagaggtc

SEQ ID NO: 256 - DNA, 16 bp, synthetic construct
  source 1..16: mol_type = other DNA
  modified_base 1..16: mod_base = OTHER; note = phosphorothioate bond
  modified_base 1: mod_base = OTHER; note = modified LNA monomer with guanine base
  modified_base 2: mod_base = OTHER; note = modified LNA monomer with 5-methylcytosine base
  modified_base 3: mod_base = OTHER; note = 2'-O-[2-(N-methylcarbamoyl)ethyl]adenosine
  modified_base 12: mod_base = m5c
  modified_base 14: mod_base = OTHER; note = 2'-O-[2-(N-methylcarbamoyl)ethyl]-5-methylcytidine
  modified_base 15: mod_base = OTHER; note = modified LNA monomer with adenine base
  modified_base 16: mod_base = OTHER; note = modified LNA monomer with thymine base
gcataagaaagctcat

SEQ ID NO: 257 - DNA, 16 bp, synthetic construct
  source 1..16: mol_type = other DNA
  modified_base 1..16: mod_base = OTHER; note = phosphorothioate bond
  modified_base 1..2: mod_base = OTHER; note = modified LNA monomer with guanine base
  modified_base 3: mod_base = OTHER; note = 2'-O-[2-(N-methylcarbamoyl)ethyl]-5-methylcytidine
  modified_base 13: mod_base = m5c
  modified_base 14: mod_base = OTHER; note = 2'-O-[2-(N-methylcarbamoyl)ethyl]-5-methyluridine
  modified_base 15: mod_base = OTHER; note = modified LNA monomer with 5-methylcytosine base
  modified_base 16: mod_base = OTHER; note = modified LNA monomer with adenine base
ggcataagaaagctca

SEQ ID NO: 258 - DNA, 16 bp, synthetic construct
  source 1..16: mol_type = other DNA
  modified_base 1..16: mod_base = OTHER; note = phosphorothioate bond
  modified_base 1: mod_base = OTHER; note = modified LNA monomer with 5-methylcytosine base
  modified_base 2: mod_base = OTHER; note = modified LNA monomer with guanine base
  modified_base 3: mod_base = OTHER; note = 2'-O-[2-(N-methylcarbamoyl)ethyl]guanosine
  modified_base 11..12: mod_base = m5c
  modified_base 14: mod_base = OTHER; note = 2'-O-[2-(N-methylcarbamoyl)ethyl]-5-methylcytidine
  modified_base 15: mod_base = OTHER; note = modified LNA monomer with adenine base
  modified_base 16: mod_base = OTHER; note = modified LNA monomer with thymine base
cggaaggtgacctcat

SEQ ID NO: 259 - DNA, 16 bp, synthetic construct
  source 1..16: mol_type = other DNA
  modified_base 1..16: mod_base = OTHER; note = phosphorothioate bond
  modified_base 1: mod_base = OTHER; note = modified LNA monomer with thymine base
  modified_base 2: mod_base = OTHER; note = modified LNA monomer with guanine base
  modified_base 3: mod_base = OTHER; note = 2'-O-[2-(N-methylcarbamoyl)ethyl]-5-methylcytidine
  modified_base 11: mod_base = m5c
  modified_base 13: mod_base = m5c
  modified_base 14: mod_base = OTHER; note = 2'-O-[2-(N-methylcarbamoyl)ethyl]-5-methylcytidine
  modified_base 15..16: mod_base = OTHER; note = modified LNA monomer with 5-methylcytosine base
tgcttggtgacacccc

SEQ ID NO: 260 - DNA, 16 bp, synthetic construct
  source 1..16: mol_type = other DNA
  modified_base 1..16: mod_base = OTHER; note = phosphorothioate bond
  modified_base 1: mod_base = OTHER; note = 2'-O-[2-(N-methylcarbamoyl)ethyl]guanosine
  modified_base 2: mod_base = OTHER; note = modified LNA monomer with thymine base
  modified_base 3: mod_base = OTHER; note = modified LNA monomer with guanine base
  modified_base 12: mod_base = m5c
  modified_base 13: mod_base = OTHER; note = 2'-O-[2-(N-methylcarbamoyl)ethyl]-5-methyluridine
  modified_base 14: mod_base = OTHER; note = modified LNA monomer with guanine base
  modified_base 15: mod_base = OTHER; note = modified LNA monomer with 5-methylcytosine base
  modified_base 16: mod_base = OTHER; note = 2'-O-[2-(N-methylcarbamoyl)ethyl]adenosine
gtgttgaaattctgca

SEQ ID NO: 261 - DNA, 16 bp, synthetic construct
  source 1..16: mol_type = other DNA
  modified_base 1..16: mod_base = OTHER; note = phosphorothioate bond
  modified_base 1: mod_base = OTHER; note = 2'-O-[2-(N-methylcarbamoyl)ethyl]guanosine
  modified_base 2..3: mod_base = OTHER; note = modified LNA monomer with guanine base
  modified_base 7..8: mod_base = m5c
  modified_base 13: mod_base = OTHER; note = 2'-O-[2-(N-methylcarbamoyl)ethyl]guanosine
  modified_base 14: mod_base = OTHER; note = modified LNA monomer with thymine base
  modified_base 15: mod_base = OTHER; note = modified LNA monomer with 5-methylcytosine base
  modified_base 16: mod_base = OTHER; note = 2'-O-[2-(N-methylcarbamoyl)ethyl]-5-methyluridine
gggagtccttgagtct

SEQ ID NO: 262 - DNA, 16 bp, synthetic construct
  source 1..16: mol_type = other DNA
  modified_base 1..16: mod_base = OTHER; note = phosphorothioate bond
  modified_base 1: mod_base = OTHER; note = 2'-O-[2-(N-methylcarbamoyl)ethyl]-5-methyluridine
  modified_base 2: mod_base = OTHER; note = modified LNA monomer with thymine base
  modified_base 3: mod_base = OTHER; note = modified LNA monomer with 5-methylcytosine base
  modified_base 13: mod_base = OTHER; note = 2'-O-[2-(N-methylcarbamoyl)ethyl]-5-methylcytidine
  modified_base 14: mod_base = OTHER; note = modified LNA monomer with 5-methylcytosine base
  modified_base 15: mod_base = OTHER; note = modified LNA monomer with thymine base
  modified_base 16: mod_base = OTHER; note = 2'-O-[2-(N-methylcarbamoyl)ethyl]-5-methylcytidine
ttcggaaggtgacctc

SEQ ID NO: 263 - DNA, 16 bp, synthetic construct
  source 1..16: mol_type = other DNA
  modified_base 1..16: mod_base = OTHER; note = phosphorothioate bond
  modified_base 1: mod_base = OTHER; note = 2'-O-[2-(N-methylcarbamoyl)ethyl]guanosine
  modified_base 2: mod_base = OTHER; note = modified LNA monomer with guanine base
  modified_base 3: mod_base = OTHER; note = modified LNA monomer with adenine base
  modified_base 6: mod_base = m5c
  modified_base 10: mod_base = m5c
  modified_base 13: mod_base = OTHER; note = 2'-O-[2-(N-methylcarbamoyl)ethyl]guanosine
  modified_base 14: mod_base = OTHER; note = modified LNA monomer with guanine base
  modified_base 15: mod_base = OTHER; note = modified LNA monomer with thymine base
  modified_base 16: mod_base = OTHER; note = 2'-O-[2-(N-methylcarbamoyl)ethyl]-5-methylcytidine
ggattcagtctgggtc

SEQ ID NO: 264 - DNA, 16 bp, synthetic construct
  source 1..16: mol_type = other DNA
  modified_base 1..16: mod_base = OTHER; note = phosphorothioate bond
  modified_base 1: mod_base = OTHER; note = 2'-O-[2-(N-methylcarbamoyl)ethyl]-5-methylcytidine
  modified_base 2: mod_base = OTHER; note = modified LNA monomer with guanine base
  modified_base 3: mod_base = OTHER; note = modified LNA monomer with thymine base
  modified_base 13: mod_base = OTHER; note = 2'-O-[2-(N-methylcarbamoyl)ethyl]-5-methylcytidine
  modified_base 14: mod_base = OTHER; note = modified LNA monomer with thymine base
  modified_base 15: mod_base = OTHER; note = modified LNA monomer with guanine base
  modified_base 16: mod_base = OTHER; note = 2'-O-[2-(N-methylcarbamoyl)ethyl]-5-methylcytidine
cgtgttgaaattctgc

SEQ ID NO: 265 - DNA, 16 bp, synthetic construct
  source 1..16: mol_type = other DNA
  modified_base 1..16: mod_base = OTHER; note = phosphorothioate bond
  modified_base 1: mod_base = OTHER; note = 2'-O-[2-(N-methylcarbamoyl)ethyl]guanosine
  modified_base 2: mod_base = OTHER; note = modified LNA monomer with 5-methylcytosine base
  modified_base 3: mod_base = OTHER; note = modified LNA monomer with guanine base
  modified_base 13: mod_base = OTHER; note = 2'-O-[2-(N-methylcarbamoyl)ethyl]-5-methyluridine
  modified_base 14: mod_base = OTHER; note = modified LNA monomer with 5-methylcytosine base
  modified_base 15: mod_base = OTHER; note = modified LNA monomer with thymine base
  modified_base 16: mod_base = OTHER; note = 2'-O-[2-(N-methylcarbamoyl)ethyl]guanosine
gcgtgttgaaattctg

SEQ ID NO: 266 - DNA, 16 bp, synthetic construct
  source 1..16: mol_type = other DNA
  modified_base 1..16: mod_base = OTHER; note = phosphorothioate bond
  modified_base 1: mod_base = OTHER; note = 2'-O-[2-(N-methylcarbamoyl)ethyl]guanosine
  modified_base 2: mod_base = OTHER; note = modified LNA monomer with adenine base
  modified_base 3: mod_base = OTHER; note = modified LNA monomer with guanine base
  modified_base 5..6: mod_base = m5c
  modified_base 13: mod_base = OTHER; note = 2'-O-[2-(N-methylcarbamoyl)ethyl]-5-methylcytidine
  modified_base 14: mod_base = OTHER; note = modified LNA monomer with thymine base
  modified_base 15: mod_base = OTHER; note = modified LNA monomer with guanine base
  modified_base 16: mod_base = OTHER; note = 2'-O-[2-(N-methylcarbamoyl)ethyl]guanosine
gagtccttgagtctgg

SEQ ID NO: 267 - DNA, 16 bp, synthetic construct
  source 1..16: mol_type = other DNA
  modified_base 1..16: mod_base = OTHER; note = phosphorothioate bond
  modified_base 1: mod_base = OTHER; note = 2'-O-[2-(N-methylcarbamoyl)ethyl]guanosine
  modified_base 2: mod_base = OTHER; note = modified LNA monomer with guanine base
  modified_base 3: mod_base = OTHER; note = modified LNA monomer with adenine base
  modified_base 6..7: mod_base = m5c
  modified_base 13: mod_base = OTHER; note = 2'-O-[2-(N-methylcarbamoyl)ethyl]-5-methyluridine
  modified_base 14: mod_base = OTHER; note = modified LNA monomer with 5-methylcytosine base
  modified_base 15: mod_base = OTHER; note = modified LNA monomer with thymine base
  modified_base 16: mod_base = OTHER; note = 2'-O-[2-(N-methylcarbamoyl)ethyl]guanosine
ggagtccttgagtctg

SEQ ID NO: 268 - DNA, 16 bp, synthetic construct
  source 1..16: mol_type = other DNA
  modified_base 1..16: mod_base = OTHER; note = phosphorothioate bond
  modified_base 1: mod_base = OTHER; note = 2'-O-[2-(N-methylcarbamoyl)ethyl]-5-methyluridine
  modified_base 2..3: mod_base = OTHER; note = modified LNA monomer with guanine base
  modified_base 8..9: mod_base = m5c
  modified_base 13: mod_base = OTHER; note = 2'-O-[2-(N-methylcarbamoyl)ethyl]adenosine
  modified_base 14: mod_base = OTHER; note = modified LNA monomer with guanine base
  modified_base 15: mod_base = OTHER; note = modified LNA monomer with thymine base
  modified_base 16: mod_base = OTHER; note = 2'-O-[2-(N-methylcarbamoyl)ethyl]-5-methylcytidine
tgggagtccttgagtc

SEQ ID NO: 269 - DNA, 16 bp, synthetic construct
  source 1..16: mol_type = other DNA
  modified_base 1..16: mod_base = OTHER; note = phosphorothioate bond
  modified_base 1: mod_base = OTHER; note = 2'-O-[2-(N-methylcarbamoyl)ethyl]guanosine
  modified_base 2..3: mod_base = OTHER; note = modified LNA monomer with thymine base
  modified_base 4: mod_base = m5c
  modified_base 7: mod_base = m5c
  modified_base 13: mod_base = OTHER; note = 2'-O-[2-(N-methylcarbamoyl)ethyl]-5-methyluridine
  modified_base 14: mod_base = OTHER; note = modified LNA monomer with adenine base
  modified_base 15: mod_base = OTHER; note = modified LNA monomer with guanine base
  modified_base 16: mod_base = OTHER; note = 2'-O-[2-(N-methylcarbamoyl)ethyl]guanosine
gttcagcttgggtagg

SEQ ID NO: 270 - DNA, 16 bp, synthetic construct
  source 1..16: mol_type = other DNA
  modified_base 1..16: mod_base = OTHER; note = phosphorothioate bond
  modified_base 1: mod_base = OTHER; note = 2'-O-[2-(N-methylcarbamoyl)ethyl]-5-methylcytidine
  modified_base 2: mod_base = OTHER; note = modified LNA monomer with 5-methylcytosine base
  modified_base 3: mod_base = OTHER; note = modified LNA monomer with guanine base
  modified_base 13: mod_base = OTHER; note = 2'-O-[2-(N-methylcarbamoyl)ethyl]guanosine
  modified_base 14: mod_base = OTHER; note = modified LNA monomer with guanine base
  modified_base 15: mod_base = OTHER; note = modified LNA monomer with thymine base
  modified_base 16: mod_base = OTHER; note = 2'-O-[2-(N-methylcarbamoyl)ethyl]-5-methylcytidine
ccgtgtagaagaggtc

SEQ ID NO: 271 - DNA, 16 bp, synthetic construct
  source 1..16: mol_type = other DNA
  modified_base 1..16: mod_base = OTHER; note = phosphorothioate bond
  modified_base 1: mod_base = OTHER; note = 2'-O-[2-(N-methylcarbamoyl)ethyl]guanosine
  modified_base 2: mod_base = OTHER; note = modified LNA monomer with 5-methylcytosine base
  modified_base 3: mod_base = OTHER; note = modified LNA monomer with adenine base
  modified_base 12: mod_base = m5c
  modified_base 13: mod_base = OTHER; note = 2'-O-[2-(N-methylcarbamoyl)ethyl]-5-methyluridine
  modified_base 14: mod_base = OTHER; note = modified LNA monomer with 5-methylcytosine base
  modified_base 15: mod_base = OTHER; note = modified LNA monomer with adenine base
  modified_base 16: mod_base = OTHER; note = 2'-O-[2-(N-methylcarbamoyl)ethyl]-5-methyluridine
gcataagaaagctcat

SEQ ID NO: 272 - DNA, 16 bp, synthetic construct
  source 1..16: mol_type = other DNA
  modified_base 1..16: mod_base = OTHER; note = phosphorothioate bond
  modified_base 1: mod_base = OTHER; note = 2'-O-[2-(N-methylcarbamoyl)ethyl]guanosine
  modified_base 2: mod_base = OTHER; note = modified LNA monomer with guanine base
  modified_base 3: mod_base = OTHER; note = modified LNA monomer with 5-methylcytosine base
  modified_base 13: mod_base = OTHER; note = 2'-O-[2-(N-methylcarbamoyl)ethyl]-5-methylcytidine
  modified_base 14: mod_base = OTHER; note = modified LNA monomer with thymine base
  modified_base 15: mod_base = OTHER; note = modified LNA monomer with 5-methylcytosine base
  modified_base 16: mod_base = OTHER; note = 2'-O-[2-(N-methylcarbamoyl)ethyl]adenosine
ggcataagaaagctca

SEQ ID NO: 273 - DNA, 16 bp, synthetic construct
  source 1..16: mol_type = other DNA
  modified_base 1..16: mod_base = OTHER; note = phosphorothioate bond
  modified_base 1: mod_base = OTHER; note = 2'-O-[2-(N-methylcarbamoyl)ethyl]-5-methylcytidine
  modified_base 2..3: mod_base = OTHER; note = modified LNA monomer with guanine base
  modified_base 11..12: mod_base = m5c
  modified_base 13: mod_base = OTHER; note = 2'-O-[2-(N-methylcarbamoyl)ethyl]-5-methyluridine
  modified_base 14: mod_base = OTHER; note = modified LNA monomer with 5-methylcytosine base
  modified_base 15: mod_base = OTHER; note = modified LNA monomer with adenine base
  modified_base 16: mod_base = OTHER; note = 2'-O-[2-(N-methylcarbamoyl)ethyl]-5-methyluridine
cggaaggtgacctcat

SEQ ID NO: 274 - DNA, 16 bp, synthetic construct
  source 1..16: mol_type = other DNA
  modified_base 1..16: mod_base = OTHER; note = phosphorothioate bond
  modified_base 1: mod_base = OTHER; note = 2'-O-[2-(N-methylcarbamoyl)ethyl]-5-methyluridine
  modified_base 2: mod_base = OTHER; note = modified LNA monomer with guanine base
  modified_base 3: mod_base = OTHER; note = modified LNA monomer with 5-methylcytosine base
  modified_base 11: mod_base = m5c
  modified_base 13: mod_base = OTHER; note = 2'-O-[2-(N-methylcarbamoyl)ethyl]-5-methylcytidine
  modified_base 14..15: mod_base = OTHER; note = modified LNA monomer with 5-methylcytosine base
  modified_base 16: mod_base = OTHER; note = 2'-O-[2-(N-methylcarbamoyl)ethyl]-5-methylcytidine
tgcttggtgacacccc

SEQ ID NO: 275 - DNA, 16 bp, synthetic construct
  source 1..16: mol_type = other DNA
  modified_base 1..16: mod_base = OTHER; note = phosphorothioate bond
  modified_base 1: mod_base = OTHER; note = 2'-O-[2-(N-methylcarbamoyl)ethyl]guanosine
  modified_base 2: mod_base = OTHER; note = modified LNA monomer with thymine base
  modified_base 3: mod_base = OTHER; note = modified LNA monomer with guanine base
  modified_base 4: mod_base = OTHER; note = 2'-O-[2-(N-methylcarbamoyl)ethyl]-5-methyluridine
  modified_base 12: mod_base = m5c
  modified_base 14: mod_base = OTHER; note = modified LNA monomer with guanine base
  modified_base 15: mod_base = OTHER; note = modified LNA monomer with 5-methylcytosine base
  modified_base 16: mod_base = OTHER; note = 2'-O-[2-(N-methylcarbamoyl)ethyl]adenosine
gtgttgaaattctgca

SEQ ID NO: 276 - DNA, 16 bp, synthetic construct
  source 1..16: mol_type = other DNA
  modified_base 1..16: mod_base = OTHER; note = phosphorothioate bond
  modified_base 1: mod_base = OTHER; note = 2'-O-[2-(N-methylcarbamoyl)ethyl]guanosine
  modified_base 2..3: mod_base = OTHER; note = modified LNA monomer with guanine base
  modified_base 4: mod_base = OTHER; note = 2'-O-[2-(N-methylcarbamoyl)ethyl]adenosine
  modified_base 7..8: mod_base = m5c
  modified_base 14: mod_base = OTHER; note = modified LNA monomer with thymine base
  modified_base 15: mod_base = OTHER; note = modified LNA monomer with 5-methylcytosine base
  modified_base 16: mod_base = OTHER; note = 2'-O-[2-(N-methylcarbamoyl)ethyl]-5-methyluridine
gggagtccttgagtct

SEQ ID NO: 277 - DNA, 16 bp, synthetic construct
  source 1..16: mol_type = other DNA
  modified_base 1..16: mod_base = OTHER; note = phosphorothioate bond
  modified_base 1: mod_base = OTHER; note = 2'-O-[2-(N-methylcarbamoyl)ethyl]-5-methyluridine
  modified_base 2: mod_base = OTHER; note = modified LNA monomer with thymine base
  modified_base 3: mod_base = OTHER; note = modified LNA monomer with 5-methylcytosine base
  modified_base 4: mod_base = OTHER; note = 2'-O-[2-(N-methylcarbamoyl)ethyl]guanosine
  modified_base 13: mod_base = m5c
  modified_base 14: mod_base = OTHER; note = modified LNA monomer with 5-methylcytosine base
  modified_base 15: mod_base = OTHER; note = modified LNA monomer with thymine base
  modified_base 16: mod_base = OTHER; note = 2'-O-[2-(N-methylcarbamoyl)ethyl]-5-methylcytidine
ttcggaaggtgacctc

SEQ ID NO: 278 - DNA, 16 bp, synthetic construct
  source 1..16: mol_type = other DNA
  modified_base 1..16: mod_base = OTHER; note = phosphorothioate bond
  modified_base 1: mod_base = OTHER; note = 2'-O-[2-(N-methylcarbamoyl)ethyl]guanosine
  modified_base 2: mod_base = OTHER; note = modified LNA monomer with guanine base
  modified_base 3: mod_base = OTHER; note = modified LNA monomer with adenine base
  modified_base 4: mod_base = OTHER; note = 2'-O-[2-(N-methylcarbamoyl)ethyl]-5-methyluridine
  modified_base 6: mod_base = m5c
  modified_base 10: mod_base = m5c
  modified_base 14: mod_base = OTHER; note = modified LNA monomer with guanine base
  modified_base 15: mod_base = OTHER; note = modified LNA monomer with thymine base
  modified_base 16: mod_base = OTHER; note = 2'-O-[2-(N-methylcarbamoyl)ethyl]-5-methylcytidine
ggattcagtctgggtc

SEQ ID NO: 279 - DNA, 16 bp, synthetic construct
  source 1..16: mol_type = other DNA
  modified_base 1..16: mod_base = OTHER; note = phosphorothioate bond
  modified_base 1: mod_base = OTHER; note = 2'-O-[2-(N-methylcarbamoyl)ethyl]-5-methylcytidine
  modified_base 2: mod_base = OTHER; note = modified LNA monomer with guanine base
  modified_base 3: mod_base = OTHER; note = modified LNA monomer with thymine base
  modified_base 4: mod_base = OTHER; note = 2'-O-[2-(N-methylcarbamoyl)ethyl]guanosine
  modified_base 13: mod_base = m5c
  modified_base 14: mod_base = OTHER; note = modified LNA monomer with thymine base
  modified_base 15: mod_base = OTHER; note = modified LNA monomer with guanine base
  modified_base 16: mod_base = OTHER; note = 2'-O-[2-(N-methylcarbamoyl)ethyl]-5-methylcytidine
cgtgttgaaattctgc

SEQ ID NO: 280 - DNA, 16 bp, synthetic construct
  source 1..16: mol_type = other DNA
  modified_base 1..16: mod_base = OTHER; note = phosphorothioate bond
  modified_base 1: mod_base = OTHER; note = 2'-O-[2-(N-methylcarbamoyl)ethyl]guanosine
  modified_base 2: mod_base = OTHER; note = modified LNA monomer with 5-methylcytosine base
  modified_base 3: mod_base = OTHER; note = modified LNA monomer with guanine base
  modified_base 4: mod_base = OTHER; note = 2'-O-[2-(N-methylcarbamoyl)ethyl]-5-methyluridine
  modified_base 14: mod_base = OTHER; note = modified LNA monomer with 5-methylcytosine base
  modified_base 15: mod_base = OTHER; note = modified LNA monomer with thymine base
  modified_base 16: mod_base = OTHER; note = 2'-O-[2-(N-methylcarbamoyl)ethyl]guanosine
gcgtgttgaaattctg

SEQ ID NO: 281 - DNA, 16 bp, synthetic construct
  source 1..16: mol_type = other DNA
  modified_base 1..16: mod_base = OTHER; note = phosphorothioate bond
  modified_base 1: mod_base = OTHER; note = 2'-O-[2-(N-methylcarbamoyl)ethyl]guanosine
  modified_base 2: mod_base = OTHER; note = modified LNA monomer with adenine base
  modified_base 3: mod_base = OTHER; note = modified LNA monomer with guanine base
  modified_base 4: mod_base = OTHER; note = 2'-O-[2-(N-methylcarbamoyl)ethyl]-5-methyluridine
  modified_base 5..6: mod_base = m5c
  modified_base 13: mod_base = m5c
  modified_base 14: mod_base = OTHER; note = modified LNA monomer with thymine base
  modified_base 15: mod_base = OTHER; note = modified LNA monomer with guanine base
  modified_base 16: mod_base = OTHER; note = 2'-O-[2-(N-methylcarbamoyl)ethyl]guanosine
gagtccttgagtctgg

SEQ ID NO: 282 - DNA, 16 bp, synthetic construct
  source 1..16: mol_type = other DNA
  modified_base 1..16: mod_base = OTHER; note = phosphorothioate bond
  modified_base 1: mod_base = OTHER; note = 2'-O-[2-(N-methylcarbamoyl)ethyl]guanosine
  modified_base 2: mod_base = OTHER; note = modified LNA monomer with guanine base
  modified_base 3: mod_base = OTHER; note = modified LNA monomer with adenine base
  modified_base 4: mod_base = OTHER; note = 2'-O-[2-(N-methylcarbamoyl)ethyl]guanosine
  modified_base 6..7: mod_base = m5c
  modified_base 14: mod_base = OTHER; note = modified LNA monomer with 5-methylcytosine base
  modified_base 15: mod_base = OTHER; note = modified LNA monomer with thymine base
  modified_base 16: mod_base = OTHER; note = 2'-O-[2-(N-methylcarbamoyl)ethyl]guanosine
ggagtccttgagtctg

SEQ ID NO: 283 - DNA, 16 bp, synthetic construct
  source 1..16: mol_type = other DNA
  modified_base 1..16: mod_base = OTHER; note = phosphorothioate bond
  modified_base 1: mod_base = OTHER; note = 2'-O-[2-(N-methylcarbamoyl)ethyl]-5-methyluridine
  modified_base 2..3: mod_base = OTHER; note = modified LNA monomer with guanine base
  modified_base 4: mod_base = OTHER; note = 2'-O-[2-(N-methylcarbamoyl)ethyl]guanosine
  modified_base 8..9: mod_base = m5c
  modified_base 14: mod_base = OTHER; note = modified LNA monomer with guanine base
  modified_base 15: mod_base = OTHER; note = modified LNA monomer with thymine base
  modified_base 16: mod_base = OTHER; note = 2'-O-[2-(N-methylcarbamoyl)ethyl]-5-methylcytidine
tgggagtccttgagtc

SEQ ID NO: 284 - DNA, 16 bp, synthetic construct
  source 1..16: mol_type = other DNA
  modified_base 1..16: mod_base = OTHER; note = phosphorothioate bond
  modified_base 1: mod_base = OTHER; note = 2'-O-[2-(N-methylcarbamoyl)ethyl]guanosine
  modified_base 2..3: mod_base = OTHER; note = modified LNA monomer with thymine base
  modified_base 4: mod_base = OTHER; note = 2'-O-[2-(N-methylcarbamoyl)ethyl]-5-methylcytidine
  modified_base 7: mod_base = m5c
  modified_base 14: mod_base = OTHER; note = modified LNA monomer with adenine base
  modified_base 15: mod_base = OTHER; note = modified LNA monomer with guanine base
  modified_base 16: mod_base = OTHER; note = 2'-O-[2-(N-methylcarbamoyl)ethyl]guanosine
gttcagcttgggtagg

SEQ ID NO: 285 - DNA, 16 bp, synthetic construct
  source 1..16: mol_type = other DNA
  modified_base 1..16: mod_base = OTHER; note = phosphorothioate bond
  modified_base 1: mod_base = OTHER; note = 2'-O-[2-(N-methylcarbamoyl)ethyl]-5-methylcytidine
  modified_base 2: mod_base = OTHER; note = modified LNA monomer with 5-methylcytosine base
  modified_base 3: mod_base = OTHER; note = modified LNA monomer with guanine base
  modified_base 4: mod_base = OTHER; note = 2'-O-[2-(N-methylcarbamoyl)ethyl]-5-methyluridine
  modified_base 14: mod_base = OTHER; note = modified LNA monomer with guanine base
  modified_base 15: mod_base = OTHER; note = modified LNA monomer with thymine base
  modified_base 16: mod_base = OTHER; note = 2'-O-[2-(N-methylcarbamoyl)ethyl]-5-methylcytidine
ccgtgtagaagaggtc

SEQ ID NO: 286 - DNA, 16 bp, synthetic construct
  source 1..16: mol_type = other DNA
  modified_base 1..16: mod_base = OTHER; note = phosphorothioate bond
  modified_base 1: mod_base = OTHER; note = 2'-O-[2-(N-methylcarbamoyl)ethyl]guanosine
  modified_base 2: mod_base = OTHER; note = modified LNA monomer with 5-methylcytosine base
  modified_base 3: mod_base = OTHER; note = modified LNA monomer with adenine base
  modified_base 4: mod_base = OTHER; note = 2'-O-[2-(N-methylcarbamoyl)ethyl]-5-methyluridine
  modified_base 12: mod_base = m5c
  modified_base 14: mod_base = OTHER; note = modified LNA monomer with 5-methylcytosine base
  modified_base 15: mod_base = OTHER; note = modified LNA monomer with adenine base
  modified_base 16: mod_base = OTHER; note = 2'-O-[2-(N-methylcarbamoyl)ethyl]-5-methyluridine
gcataagaaagctcat

SEQ ID NO: 287 - DNA, 16 bp, synthetic construct
  source 1..16: mol_type = other DNA
  modified_base 1..16: mod_base = OTHER; note = phosphorothioate bond
  modified_base 1: mod_base = OTHER; note = 2'-O-[2-(N-methylcarbamoyl)ethyl]guanosine
  modified_base 2: mod_base = OTHER; note = modified LNA monomer with guanine base
  modified_base 3: mod_base = OTHER; note = modified LNA monomer with 5-methylcytosine base
  modified_base 4: mod_base = OTHER; note = 2'-O-[2-(N-methylcarbamoyl)ethyl]adenosine
  modified_base 13: mod_base = m5c
  modified_base 14: mod_base = OTHER; note = modified LNA monomer with thymine base
  modified_base 15: mod_base = OTHER; note = modified LNA monomer with 5-methylcytosine base
  modified_base 16: mod_base = OTHER; note = 2'-O-[2-(N-methylcarbamoyl)ethyl]adenosine
ggcataagaaagctca

SEQ ID NO: 288 - DNA, 16 bp, synthetic construct
  source 1..16: mol_type = other DNA
  modified_base 1..16: mod_base = OTHER; note = phosphorothioate bond
  modified_base 1: mod_base = OTHER; note = 2'-O-[2-(N-methylcarbamoyl)ethyl]-5-methylcytidine
  modified_base 2..3: mod_base = OTHER; note = modified LNA monomer with guanine base
  modified_base 4: mod_base = OTHER; note = 2'-O-[2-(N-methylcarbamoyl)ethyl]adenosine
  modified_base 11..12: mod_base = m5c
  modified_base 14: mod_base = OTHER; note = modified LNA monomer with 5-methylcytosine base
  modified_base 15: mod_base = OTHER; note = modified LNA monomer with adenine base
  modified_base 16: mod_base = OTHER; note = 2'-O-[2-(N-methylcarbamoyl)ethyl]-5-methyluridine
cggaaggtgacctcat

SEQ ID NO: 289 - DNA, 16 bp, synthetic construct
  source 1..16: mol_type = other DNA
  modified_base 1: mod_base = OTHER; note = 2'-O-[2-(N-methylcarbamoyl)ethyl]-5-methyluridine
  modified_base 1..16: mod_base = OTHER; note = phosphorothioate bond
  modified_base 2: mod_base = OTHER; note = modified LNA monomer with guanine base
  modified_base 3: mod_base = OTHER; note = modified LNA monomer with 5-methylcytosine base
  modified_base 4: mod_base = OTHER; note = 2'-O-[2-(N-methylcarbamoyl)ethyl]-5-methyluridine
  modified_base 11: mod_base = m5c
  modified_base 13: mod_base = m5c
  modified_base 14..15: mod_base = OTHER; note = modified LNA monomer with 5-methylcytosine base
  modified_base 16: mod_base = OTHER; note = 2'-O-[2-(N-methylcarbamoyl)ethyl]-5-methylcytidine
tgcttggtgacacccc

SEQ ID NO: 290 - DNA, 16 bp, synthetic construct
  source 1..16: mol_type = other DNA
  modified_base 1..16: mod_base = OTHER; note = phosphorothioate bond
  modified_base 1: mod_base = OTHER; note = 2'-O-[2-(N-methylcarbamoyl)ethyl]guanosine
  modified_base 2: mod_base = OTHER; note = modified LNA monomer with thymine base
  modified_base 3: mod_base = OTHER; note = modified LNA monomer with guanine base
  modified_base 4..5: mod_base = OTHER; note = 2'-O-[2-(N-methylcarbamoyl)ethyl]-5-methyluridine
  modified_base 12: mod_base = m5c
  modified_base 14: mod_base = OTHER; note = modified LNA monomer with guanine base
  modified_base 15: mod_base = OTHER; note = modified LNA monomer with 5-methylcytosine base
  modified_base 16: mod_base = OTHER; note = 2'-O-[2-(N-methylcarbamoyl)ethyl]adenosine
gtgttgaaattctgca

SEQ ID NO: 291 - DNA, 16 bp, synthetic construct
  source 1..16: mol_type = other DNA
  modified_base 1..16: mod_base = OTHER; note = phosphorothioate bond
  modified_base 1: mod_base = OTHER; note = 2'-O-[2-(N-methylcarbamoyl)ethyl]guanosine
  modified_base 2..3: mod_base = OTHER; note = modified LNA monomer with guanine base
  modified_base 4: mod_base = OTHER; note = 2'-O-[2-(N-methylcarbamoyl)ethyl]adenosine
  modified_base 5: mod_base = OTHER; note = 2'-O-[2-(N-methylcarbamoyl)ethyl]guanosine
  modified_base 7..8: mod_base = m5c
  modified_base 14: mod_base = OTHER; note = modified LNA monomer with thymine base
  modified_base 15: mod_base = OTHER; note = modified LNA monomer with 5-methylcytosine base
  modified_base 16: mod_base = OTHER; note = 2'-O-[2-(N-methylcarbamoyl)ethyl]-5-methyluridine
gggagtccttgagtct

SEQ ID NO: 292 - DNA, 16 bp, synthetic construct
  source 1..16: mol_type = other DNA
  modified_base 1..16: mod_base = OTHER; note = phosphorothioate bond
  modified_base 1: mod_base = OTHER; note = 2'-O-[2-(N-methylcarbamoyl)ethyl]-5-methyluridine
  modified_base 2: mod_base = OTHER; note = modified LNA monomer with thymine base
  modified_base 3: mod_base = OTHER; note = modified LNA monomer with 5-methylcytosine base
  modified_base 4..5: mod_base = OTHER; note = 2'-O-[2-(N-methylcarbamoyl)ethyl]guanosine
  modified_base 13: mod_base = m5c
  modified_base 14: mod_base = OTHER; note = modified LNA monomer with 5-methylcytosine base
  modified_base 15: mod_base = OTHER; note = modified LNA monomer with thymine base
  modified_base 16: mod_base = OTHER; note = 2'-O-[2-(N-methylcarbamoyl)ethyl]-5-methylcytidine
ttcggaaggtgacctc

SEQ ID NO: 293 - DNA, 16 bp, synthetic construct
  source 1..16: mol_type = other DNA
  modified_base 1..16: mod_base = OTHER; note = phosphorothioate bond
  modified_base 1: mod_base = OTHER; note = 2'-O-[2-(N-methylcarbamoyl)ethyl]guanosine
  modified_base 2: mod_base = OTHER; note = modified LNA monomer with guanine base
  modified_base 3: mod_base = OTHER; note = modified LNA monomer with adenine base
  modified_base 4..5: mod_base = OTHER; note = 2'-O-[2-(N-methylcarbamoyl)ethyl]-5-methyluridine
  modified_base 6: mod_base = m5c
  modified_base 10: mod_base = m5c
  modified_base 14: mod_base = OTHER; note = modified LNA monomer with guanine base
  modified_base 15: mod_base = OTHER; note = modified LNA monomer with thymine base
  modified_base 16: mod_base = OTHER; note = 2'-O-[2-(N-methylcarbamoyl)ethyl]-5-methylcytidine
ggattcagtctgggtc

SEQ ID NO: 294 - DNA, 16 bp, synthetic construct
  source 1..16: mol_type = other DNA
  modified_base 1..16: mod_base = OTHER; note = phosphorothioate bond
  modified_base 1: mod_base = OTHER; note = 2'-O-[2-(N-methylcarbamoyl)ethyl]-5-methylcytidine
  modified_base 2: mod_base = OTHER; note = modified LNA monomer with guanine base
  modified_base 3: mod_base = OTHER; note = modified LNA monomer with thymine base
  modified_base 4: mod_base = OTHER; note = 2'-O-[2-(N-methylcarbamoyl)ethyl]guanosine
  modified_base 5: mod_base = OTHER; note = 2'-O-[2-(N-methylcarbamoyl)ethyl]-5-methyluridine
  modified_base 13: mod_base = m5c
  modified_base 14: mod_base = OTHER; note = modified LNA monomer with thymine base
  modified_base 15: mod_base = OTHER; note = modified LNA monomer with guanine base
  modified_base 16: mod_base = OTHER; note = 2'-O-[2-(N-methylcarbamoyl)ethyl]-5-methylcytidine
cgtgttgaaattctgc

SEQ ID NO: 295 - DNA, 16 bp, synthetic construct
  source 1..16: mol_type = other DNA
  modified_base 1..16: mod_base = OTHER; note = phosphorothioate bond
  modified_base 1: mod_base = OTHER; note = 2'-O-[2-(N-methylcarbamoyl)ethyl]guanosine
  modified_base 2: mod_base = OTHER; note = modified LNA monomer with 5-methylcytosine base
  modified_base 3: mod_base = OTHER; note = modified LNA monomer with guanine base
  modified_base 4: mod_base = OTHER; note = 2'-O-[2-(N-methylcarbamoyl)ethyl]-5-methyluridine
  modified_base 5: mod_base = OTHER; note = 2'-O-[2-(N-methylcarbamoyl)ethyl]guanosine
  modified_base 14: mod_base = OTHER; note = modified LNA monomer with 5-methylcytosine base
  modified_base 15: mod_base = OTHER; note = modified LNA monomer with thymine base
  modified_base 16: mod_base = OTHER; note = 2'-O-[2-(N-methylcarbamoyl)ethyl]guanosine
gcgtgttgaaattctg

SEQ ID NO: 296 - DNA, 16 bp, synthetic construct
  source 1..16: mol_type = other DNA
  modified_base 1..16: mod_base = OTHER; note = phosphorothioate bond
  modified_base 1: mod_base = OTHER; note = 2'-O-[2-(N-methylcarbamoyl)ethyl]guanosine
  modified_base 2: mod_base = OTHER; note = modified LNA monomer with adenine base
  modified_base 3: mod_base = OTHER; note = modified LNA monomer with guanine base
  modified_base 4: mod_base = OTHER; note = 2'-O-[2-(N-methylcarbamoyl)ethyl]-5-methyluridine
  modified_base 5: mod_base = OTHER; note = 2'-O-[2-(N-methylcarbamoyl)ethyl]-5-methylcytidine
  modified_base 6: mod_base = m5c
  modified_base 13: mod_base = m5c
  modified_base 14: mod_base = OTHER; note = modified LNA monomer with thymine base
  modified_base 15: mod_base = OTHER; note = modified LNA monomer with guanine base
  modified_base 16: mod_base = OTHER; note = 2'-O-[2-(N-methylcarbamoyl)ethyl]guanosine
gagtccttgagtctgg

SEQ ID NO: 297 - DNA, 16 bp, synthetic construct
  source 1..16: mol_type = other DNA
  modified_base 1..16: mod_base = OTHER; note = phosphorothioate bond
  modified_base 1: mod_base = OTHER; note = 2'-O-[2-(N-methylcarbamoyl)ethyl]guanosine
  modified_base 2: mod_base = OTHER; note = modified LNA monomer with guanine base
  modified_base 3: mod_base = OTHER; note = modified LNA monomer with adenine base
  modified_base 4: mod_base = OTHER; note = 2'-O-[2-(N-methylcarbamoyl)ethyl]guanosine
  modified_base 5: mod_base = OTHER; note = 2'-O-[2-(N-methylcarbamoyl)ethyl]-5-methyluridine
  modified_base 6..7: mod_base = m5c
  modified_base 14: mod_base = OTHER; note = modified LNA monomer with 5-methylcytosine base
  modified_base 15: mod_base = OTHER; note = modified LNA monomer with thymine base
  modified_base 16: mod_base = OTHER; note = 2'-O-[2-(N-methylcarbamoyl)ethyl]guanosine
ggagtccttgagtctg

SEQ ID NO: 298 - DNA, 16 bp, synthetic construct
  source 1..16: mol_type = other DNA
  modified_base 1..16: mod_base = OTHER; note = phosphorothioate bond
  modified_base 1: mod_base = OTHER; note = 2'-O-[2-(N-methylcarbamoyl)ethyl]-5-methyluridine
  modified_base 2..3: mod_base = OTHER; note = modified LNA monomer with guanine base
  modified_base 4: mod_base = OTHER; note = 2'-O-[2-(N-methylcarbamoyl)ethyl]guanosine
  modified_base 5: mod_base = OTHER; note = 2'-O-[2-(N-methylcarbamoyl)ethyl]adenosine
  modified_base 8..9: mod_base = m5c
  modified_base 14: mod_base = OTHER; note = modified LNA monomer with guanine base
  modified_base 15: mod_base = OTHER; note = modified LNA monomer with thymine base
  modified_base 16: mod_base = OTHER; note = 2'-O-[2-(N-methylcarbamoyl)ethyl]-5-methylcytidine
tgggagtccttgagtc

SEQ ID NO: 299 - DNA, 16 bp, synthetic construct
  source 1..16: mol_type = other DNA
  modified_base 1..16: mod_base = OTHER; note = phosphorothioate bond
  modified_base 1: mod_base = OTHER; note = 2'-O-[2-(N-methylcarbamoyl)ethyl]guanosine
  modified_base 2..3: mod_base = OTHER; note = modified LNA monomer with thymine base
  modified_base 4: mod_base = OTHER; note = 2'-O-[2-(N-methylcarbamoyl)ethyl]-5-methylcytidine
  modified_base 5: mod_base = OTHER; note = 2'-O-[2-(N-methylcarbamoyl)ethyl]adenosine
  modified_base 7: mod_base = m5c
  modified_base 14: mod_base = OTHER; note = modified LNA monomer with adenine base
  modified_base 15: mod_base = OTHER; note = modified LNA monomer with guanine base
  modified_base 16: mod_base = OTHER; note = 2'-O-[2-(N-methylcarbamoyl)ethyl]guanosine
gttcagcttgggtagg

SEQ ID NO: 300 - DNA, 16 bp, synthetic construct
  source 1..16: mol_type = other DNA
  modified_base 1..16: mod_base = OTHER; note = phosphorothioate bond
  modified_base 1: mod_base = OTHER; note = 2'-O-[2-(N-methylcarbamoyl)ethyl]-5-methylcytidine
  modified_base 2: mod_base = OTHER; note = modified LNA monomer with 5-methylcytosine base
  modified_base 3: mod_base = OTHER; note = modified LNA monomer with guanine base
  modified_base 4: mod_base = OTHER; note = 2'-O-[2-(N-methylcarbamoyl)ethyl]-5-methyluridine
  modified_base 5: mod_base = OTHER; note = 2'-O-[2-(N-methylcarbamoyl)ethyl]guanosine
  modified_base 14: mod_base = OTHER; note = modified LNA monomer with guanine base
  modified_base 15: mod_base = OTHER; note = modified LNA monomer with thymine base
  modified_base 16: mod_base = OTHER; note = 2'-O-[2-(N-methylcarbamoyl)ethyl]-5-methylcytidine
ccgtgtagaagaggtc

SEQ ID NO: 301 - DNA, 16 bp, synthetic construct
  source 1..16: mol_type = other DNA
  modified_base 1..16: mod_base = OTHER; note = phosphorothioate bond
  modified_base 1: mod_base = OTHER; note = 2'-O-[2-(N-methylcarbamoyl)ethyl]guanosine
  modified_base 2: mod_base = OTHER; note = modified LNA monomer with 5-methylcytosine base
  modified_base 3: mod_base = OTHER; note = modified LNA monomer with adenine base
  modified_base 4: mod_base = OTHER; note = 2'-O-[2-(N-methylcarbamoyl)ethyl]-5-methyluridine
  modified_base 5: mod_base = OTHER; note = 2'-O-[2-(N-methylcarbamoyl)ethyl]adenosine
  modified_base 12: mod_base = m5c
  modified_base 14: mod_base = OTHER; note = modified LNA monomer with 5-methylcytosine base
  modified_base 15: mod_base = OTHER; note = modified LNA monomer with adenine base
  modified_base 16: mod_base = OTHER; note = 2'-O-[2-(N-methylcarbamoyl)ethyl]-5-methyluridine
gcataagaaagctcat

SEQ ID NO: 302 - DNA, 16 bp, synthetic construct
  source 1..16: mol_type = other DNA
  modified_base 1..16: mod_base = OTHER; note = phosphorothioate bond
  modified_base 1: mod_base = OTHER; note = 2'-O-[2-(N-methylcarbamoyl)ethyl]guanosine
  modified_base 2: mod_base = OTHER; note = modified LNA monomer with guanine base
  modified_base 3: mod_base = OTHER; note = modified LNA monomer with 5-methylcytosine base
  modified_base 4: mod_base = OTHER; note = 2'-O-[2-(N-methylcarbamoyl)ethyl]adenosine
  modified_base 5: mod_base = OTHER; note = 2'-O-[2-(N-methylcarbamoyl)ethyl]-5-methyluridine
  modified_base 13: mod_base = m5c
  modified_base 14: mod_base = OTHER; note = modified LNA monomer with thymine base
  modified_base 15: mod_base = OTHER; note = modified LNA monomer with 5-methylcytosine base
  modified_base 16: mod_base = OTHER; note = 2'-O-[2-(N-methylcarbamoyl)ethyl]adenosine
ggcataagaaagctca

SEQ ID NO: 303 - DNA, 16 bp, synthetic construct
  source 1..16: mol_type = other DNA
  modified_base 1..16: mod_base = OTHER; note = phosphorothioate bond
  modified_base 1: mod_base = OTHER; note = 2'-O-[2-(N-methylcarbamoyl)ethyl]-5-methylcytidine
  modified_base 2..3: mod_base = OTHER; note = modified LNA monomer with guanine base
  modified_base 4..5: mod_base = OTHER; note = 2'-O-[2-(N-methylcarbamoyl)ethyl]adenosine
  modified_base 11..12: mod_base = m5c
  modified_base 14: mod_base = OTHER; note = modified LNA monomer with 5-methylcytosine base
  modified_base 15: mod_base = OTHER; note = modified LNA monomer with adenine base
  modified_base 16: mod_base = OTHER; note = 2'-O-[2-(N-methylcarbamoyl)ethyl]-5-methyluridine
cggaaggtgacctcat

SEQ ID NO: 304 - DNA, 16 bp, synthetic construct
  source 1..16: mol_type = other DNA
  modified_base 1..16: mod_base = OTHER; note = phosphorothioate bond
  modified_base 1: mod_base = OTHER; note = 2'-O-[2-(N-methylcarbamoyl)ethyl]-5-methyluridine
  modified_base 2: mod_base = OTHER; note = modified LNA monomer with guanine base
  modified_base 3: mod_base = OTHER; note = modified LNA monomer with 5-methylcytosine base
  modified_base 4..5: mod_base = OTHER; note = 2'-O-[2-(N-methylcarbamoyl)ethyl]-5-methyluridine
  modified_base 11: mod_base = m5c
  modified_base 13: mod_base = m5c
  modified_base 14..15: mod_base = OTHER; note = modified LNA monomer with 5-methylcytosine base
  modified_base 16: mod_base = OTHER; note = 2'-O-[2-(N-methylcarbamoyl)ethyl]-5-methylcytidine
tgcttggtgacacccc

SEQ ID NO: 305 - DNA, 16 bp, synthetic construct
  source 1..16: mol_type = other DNA
  modified_base 1..2: mod_base = OTHER; note = phosphorothioate bond
  modified_base 4..14: mod_base = OTHER; note = phosphorothioate bond
  modified_base 15..16: mod_base = OTHER; note = phosphorothioate bond
  modified_base 1: mod_base = OTHER; note = 2'-O-[2-(N-methylcarbamoyl)ethyl]guanosine
  modified_base 2: mod_base = OTHER; note = modified LNA monomer with thymine base
  modified_base 3: mod_base = OTHER; note = modified LNA monomer with guanine base
  modified_base 12: mod_base = m5c
  modified_base 14: mod_base = OTHER; note = modified LNA monomer with guanine base
  modified_base 15: mod_base = OTHER; note = modified LNA monomer with 5-methylcytosine base
  modified_base 16: mod_base = OTHER; note = 2'-O-[2-(N-methylcarbamoyl)ethyl]adenosine
gtgttgaaattctgca

SEQ ID NO: 306 - DNA, 16 bp, synthetic construct
  source 1..16: mol_type = other DNA
  modified_base 1..2: mod_base = OTHER; note = phosphorothioate bond
  modified_base 4..14: mod_base = OTHER; note = phosphorothioate bond
  modified_base 15..16: mod_base = OTHER; note = phosphorothioate bond
  modified_base 1: mod_base = OTHER; note = 2'-O-[2-(N-methylcarbamoyl)ethyl]guanosine
  modified_base 2..3: mod_base = OTHER; note = modified LNA monomer with guanine base
  modified_base 7..8: mod_base = m5c
  modified_base 14: mod_base = OTHER; note = modified LNA monomer with thymine base
  modified_base 15: mod_base = OTHER; note = modified LNA monomer with 5-methylcytosine base
  modified_base 16: mod_base = OTHER; note = 2'-O-[2-(N-methylcarbamoyl)ethyl]-5-methyluridine
gggagtccttgagtct

SEQ ID NO: 307 - DNA, 16 bp, synthetic construct
  source 1..16: mol_type = other DNA
  modified_base 1..2: mod_base = OTHER; note = phosphorothioate bond
  modified_base 4..14: mod_base = OTHER; note = phosphorothioate bond
  modified_base 15..16: mod_base = OTHER; note = phosphorothioate bond
  modified_base 1: mod_base = OTHER; note = 2'-O-[2-(N-methylcarbamoyl)ethyl]-5-methyluridine
  modified_base 2: mod_base = OTHER; note = modified LNA monomer with thymine base
  modified_base 3: mod_base = OTHER; note = modified LNA monomer with 5-methylcytosine base
  modified_base 13: mod_base = m5c
  modified_base 14: mod_base = OTHER; note = modified LNA monomer with 5-methylcytosine base
  modified_base 15: mod_base = OTHER; note = modified LNA monomer with thymine base
  modified_base 16: mod_base = OTHER; note = 2'-O-[2-(N-methylcarbamoyl)ethyl]-5-methylcytidine
ttcggaaggtgacctc

SEQ ID NO: 308 - DNA, 16 bp, synthetic construct
  source 1..16: mol_type = other DNA
  modified_base 1..2: mod_base = OTHER; note = phosphorothioate bond
  modified_base 4..14: mod_base = OTHER; note = phosphorothioate bond
  modified_base 15..16: mod_base = OTHER; note = phosphorothioate bond
  modified_base 1: mod_base = OTHER; note = 2'-O-[2-(N-methylcarbamoyl)ethyl]guanosine
  modified_base 3: mod_base = OTHER; note = modified LNA monomer with adenine base
  modified_base 2: mod_base = OTHER; note = modified LNA monomer with guanine base
  modified_base 6: mod_base = m5c
  modified_base 10: mod_base = m5c
  modified_base 14: mod_base = OTHER; note = modified LNA monomer with guanine base
  modified_base 15: mod_base = OTHER; note = modified LNA monomer with thymine base
  modified_base 16: mod_base = OTHER; note = 2'-O-[2-(N-methylcarbamoyl)ethyl]-5-methylcytidine
ggattcagtctgggtc

SEQ ID NO: 309 - DNA, 16 bp, synthetic construct
  source 1..16: mol_type = other DNA
  modified_base 1..2: mod_base = OTHER; note = phosphorothioate bond
  modified_base 4..14: mod_base = OTHER; note = phosphorothioate bond
  modified_base 15..16: mod_base = OTHER; note = phosphorothioate bond
  modified_base 1: mod_base = OTHER; note = 2'-O-[2-(N-methylcarbamoyl)ethyl]-5-methylcytidine
  modified_base 2: mod_base = OTHER; note = modified LNA monomer with guanine base
  modified_base 3: mod_base = OTHER; note = modified LNA monomer with thymine base
  modified_base 13: mod_base = m5c
  modified_base 14: mod_base = OTHER; note = modified LNA monomer with thymine base
  modified_base 15: mod_base = OTHER; note = modified LNA monomer with guanine base
  modified_base 16: mod_base = OTHER; note = 2'-O-[2-(N-methylcarbamoyl)ethyl]-5-methylcytidine
cgtgttgaaattctgc

SEQ ID NO: 310 - DNA, 16 bp, synthetic construct
  source 1..16: mol_type = other DNA
  modified_base 1..2: mod_base = OTHER; note = phosphorothioate bond
  modified_base 4..14: mod_base = OTHER; note = phosphorothioate bond
  modified_base 15..16: mod_base = OTHER; note = phosphorothioate bond
  modified_base 1: mod_base = OTHER; note = 2'-O-[2-(N-methylcarbamoyl)ethyl]guanosine
  modified_base 2: mod_base = OTHER; note = modified LNA monomer with 5-methylcytosine base
  modified_base 3: mod_base = OTHER; note = modified LNA monomer with guanine base
  modified_base 14: mod_base = OTHER; note = modified LNA monomer with 5-methylcytosine base
  modified_base 15: mod_base = OTHER; note = modified LNA monomer with thymine base
  modified_base 16: mod_base = OTHER; note = 2'-O-[2-(N-methylcarbamoyl)ethyl]guanosine
gcgtgttgaaattctg

SEQ ID NO: 311 - DNA, 16 bp, synthetic construct
  source 1..16: mol_type = other DNA
  modified_base 1..2: mod_base = OTHER; note = phosphorothioate bond
  modified_base 4..14: mod_base = OTHER; note = phosphorothioate bond
  modified_base 15..16: mod_base = OTHER; note = phosphorothioate bond
  modified_base 1: mod_base = OTHER; note = 2'-O-[2-(N-methylcarbamoyl)ethyl]guanosine
  modified_base 2: mod_base = OTHER; note = modified LNA monomer with adenine base
  modified_base 3: mod_base = OTHER; note = modified LNA monomer with guanine base
  modified_base 5..6: mod_base = m5c
  modified_base 13: mod_base = m5c
  modified_base 14: mod_base = OTHER; note = modified LNA monomer with thymine base
  modified_base 15: mod_base = OTHER; note = modified LNA monomer with guanine base
  modified_base 16: mod_base = OTHER; note = 2'-O-[2-(N-methylcarbamoyl)ethyl]guanosine
gagtccttgagtctgg

SEQ ID NO: 312 - DNA, 16 bp, synthetic construct
  source 1..16: mol_type = other DNA
  modified_base 1..2: mod_base = OTHER; note = phosphorothioate bond
  modified_base 4..14: mod_base = OTHER; note = phosphorothioate bond
  modified_base 15..16: mod_base = OTHER; note = phosphorothioate bond
  modified_base 1: mod_base = OTHER; note = 2'-O-[2-(N-methylcarbamoyl)ethyl]guanosine
  modified_base 2: mod_base = OTHER; note = modified LNA monomer with guanine base
  modified_base 3: mod_base = OTHER; note = modified LNA monomer with adenine base
  modified_base 6..7: mod_base = m5c
  modified_base 14: mod_base = OTHER; note = modified LNA monomer with 5-methylcytosine base
  modified_base 15: mod_base = OTHER; note = modified LNA monomer with thymine base
  modified_base 16: mod_base = OTHER; note = 2'-O-[2-(N-methylcarbamoyl)ethyl]guanosine
ggagtccttgagtctg

SEQ ID NO: 313 - DNA, 16 bp, synthetic construct
  source 1..16: mol_type = other DNA
  modified_base 1..2: mod_base = OTHER; note = phosphorothioate bond
  modified_base 4..14: mod_base = OTHER; note = phosphorothioate bond
  modified_base 15..16: mod_base = OTHER; note = phosphorothioate bond
  modified_base 1: mod_base = OTHER; note = 2'-O-[2-(N-methylcarbamoyl)ethyl]-5-methyluridine
  modified_base 2..3: mod_base = OTHER; note = modified LNA monomer with guanine base
  modified_base 8..9: mod_base = m5c
  modified_base 14: mod_base = OTHER; note = modified LNA monomer with guanine base
  modified_base 15: mod_base = OTHER; note = modified LNA monomer with thymine base
  modified_base 16: mod_base = OTHER; note = 2'-O-[2-(N-methylcarbamoyl)ethyl]-5-methylcytidine
tgggagtccttgagtc

SEQ ID NO: 314 - DNA, 16 bp, synthetic construct
  source 1..16: mol_type = other DNA
  modified_base 1..2: mod_base = OTHER; note = phosphorothioate bond
  modified_base 4..14: mod_base = OTHER; note = phosphorothioate bond
  modified_base 15..16: mod_base = OTHER; note = phosphorothioate bond
  modified_base 1: mod_base = OTHER; note = 2'-O-[2-(N-methylcarbamoyl)ethyl]guanosine
  modified_base 2..3: mod_base = OTHER; note = modified LNA monomer with thymine base
  modified_base 4: mod_base = m5c
  modified_base 7: mod_base = m5c
  modified_base 14: mod_base = OTHER; note = modified LNA monomer with adenine base
  modified_base 15: mod_base = OTHER; note = modified LNA monomer with guanine base
  modified_base 16: mod_base = OTHER; note = 2'-O-[2-(N-methylcarbamoyl)ethyl]guanosine
gttcagcttgggtagg

SEQ ID NO: 315 - DNA, 16 bp, synthetic construct
  source 1..16: mol_type = other DNA
  modified_base 1..2: mod_base = OTHER; note = phosphorothioate bond
  modified_base 4..14: mod_base = OTHER; note = phosphorothioate bond
  modified_base 15..16: mod_base = OTHER; note = phosphorothioate bond
  modified_base 1: mod_base = OTHER; note = 2'-O-[2-(N-methylcarbamoyl)ethyl]-5-methylcytidine
  modified_base 2: mod_base = OTHER; note = modified LNA monomer with 5-methylcytosine base
  modified_base 3: mod_base = OTHER; note = modified LNA monomer with guanine base
  modified_base 14: mod_base = OTHER; note = modified LNA monomer with guanine base
  modified_base 15: mod_base = OTHER; note = modified LNA monomer with thymine base
  modified_base 16: mod_base = OTHER; note = 2'-O-[2-(N-methylcarbamoyl)ethyl]-5-methylcytidine
ccgtgtagaagaggtc

SEQ ID NO: 316 - DNA, 16 bp, synthetic construct
  source 1..16: mol_type = other DNA
  modified_base 1..2: mod_base = OTHER; note = phosphorothioate bond
  modified_base 4..14: mod_base = OTHER; note = phosphorothioate bond
  modified_base 15..16: mod_base = OTHER; note = phosphorothioate bond
  modified_base 1: mod_base = OTHER; note = 2'-O-[2-(N-methylcarbamoyl)ethyl]guanosine
  modified_base 2: mod_base = OTHER; note = modified LNA monomer with 5-methylcytosine base
  modified_base 3: mod_base = OTHER; note = modified LNA monomer with adenine base
  modified_base 12: mod_base = m5c
  modified_base 14: mod_base = OTHER; note = modified LNA monomer with 5-methylcytosine base
  modified_base 15: mod_base = OTHER; note = modified LNA monomer with adenine base
  modified_base 16: mod_base = OTHER; note = 2'-O-[2-(N-methylcarbamoyl)ethyl]-5-methyluridine
gcataagaaagctcat

SEQ ID NO: 317 - DNA, 16 bp, synthetic construct
  source 1..16: mol_type = other DNA
  modified_base 1..2: mod_base = OTHER; note = phosphorothioate bond
  modified_base 4..14: mod_base = OTHER; note = phosphorothioate bond
  modified_base 15..16: mod_base = OTHER; note = phosphorothioate bond
  modified_base 1: mod_base = OTHER; note = 2'-O-[2-(N-methylcarbamoyl)ethyl]guanosine
  modified_base 2: mod_base = OTHER; note = modified LNA monomer with guanine base
  modified_base 3: mod_base = OTHER; note = modified LNA monomer with 5-methylcytosine base
  modified_base 13: mod_base = m5c
  modified_base 14: mod_base = OTHER; note = modified LNA monomer with thymine base
  modified_base 15: mod_base = OTHER; note = modified LNA monomer with 5-methylcytosine base
  modified_base 16: mod_base = OTHER; note = 2'-O-[2-(N-methylcarbamoyl)ethyl]adenosine
ggcataagaaagctca

SEQ ID NO: 318 - DNA, 16 bp, synthetic construct
  source 1..16: mol_type = other DNA
  modified_base 1..2: mod_base = OTHER; note = phosphorothioate bond
  modified_base 4..14: mod_base = OTHER; note = phosphorothioate bond
  modified_base 15..16: mod_base = OTHER; note = phosphorothioate bond
  modified_base 1: mod_base = OTHER; note = 2'-O-[2-(N-methylcarbamoyl)ethyl]-5-methylcytidine
  modified_base 2..3: mod_base = OTHER; note = modified LNA monomer with guanine base
  modified_base 11..12: mod_base = m5c
  modified_base 14: mod_base = OTHER; note = modified LNA monomer with 5-methylcytosine base
  modified_base 15: mod_base = OTHER; note = modified LNA monomer with adenine base
  modified_base 16: mod_base = OTHER; note = 2'-O-[2-(N-methylcarbamoyl)ethyl]-5-methyluridine
cggaaggtgacctcat

SEQ ID NO: 319 - DNA, 16 bp, synthetic construct
  source 1..16: mol_type = other DNA
  modified_base 1..2: mod_base = OTHER; note = phosphorothioate bond
  modified_base 4..14: mod_base = OTHER; note = phosphorothioate bond
  modified_base 15..16: mod_base = OTHER; note = phosphorothioate bond
  modified_base 1: mod_base = OTHER; note = 2'-O-[2-(N-methylcarbamoyl)ethyl]-5-methyluridine
  modified_base 2: mod_base = OTHER; note = modified LNA monomer with guanine base
  modified_base 3: mod_base = OTHER; note = modified LNA monomer with 5-methylcytosine base
  modified_base 11: mod_base = m5c
  modified_base 13: mod_base = m5c
  modified_base 14..15: mod_base = OTHER; note = modified LNA monomer with 5-methylcytosine base
  modified_base 16: mod_base = OTHER; note = 2'-O-[2-(N-methylcarbamoyl)ethyl]-5-methylcytidine
tgcttggtgacacccc

SEQ ID NO: 320 - DNA, 16 bp, synthetic construct
  source 1..16: mol_type = other DNA
  modified_base 1..16: mod_base = OTHER; note = phosphorothioate bond
  modified_base 1: mod_base = OTHER; note = 2'-O-[2-(N-methylcarbamoyl)ethyl]guanosine
  modified_base 2: mod_base = OTHER; note = modified LNA monomer with thymine base
  modified_base 3: mod_base = OTHER; note = modified LNA monomer with guanine base
  modified_base 4: mod_base = OTHER; note = 2'-O-[2-[N-(2-morpholinoethyl)carbamoyl]ethyl]-5-methyluridine
  modified_base 12: mod_base = m5c
  modified_base 14: mod_base = OTHER; note = modified LNA monomer with guanine base
  modified_base 15: mod_base = OTHER; note = modified LNA monomer with 5-methylcytosine base
  modified_base 16: mod_base = OTHER; note = 2'-O-[2-(N-methylcarbamoyl)ethyl]adenosine
gtgttgaaattctgca

SEQ ID NO: 321 - DNA, 16 bp, synthetic construct
  source 1..16: mol_type = other DNA
  modified_base 1..16: mod_base = OTHER; note = phosphorothioate bond
  modified_base 1: mod_base = OTHER; note = 2'-O-[2-(N-methylcarbamoyl)ethyl]guanosine
  modified_base 2..3: mod_base = OTHER; note = modified LNA monomer with guanine base
  modified_base 4: mod_base = OTHER; note = 2'-O-[2-[N-(2-morpholinoethyl)carbamoyl]ethyl]adenosine
  modified_base 7..8: mod_base = m5c
  modified_base 14: mod_base = OTHER; note = modified LNA monomer with thymine base
  modified_base 15: mod_base = OTHER; note = modified LNA monomer with 5-methylcytosine base
  modified_base 16: mod_base = OTHER; note = 2'-O-[2-(N-methylcarbamoyl)ethyl]-5-methyluridine
gggagtccttgagtct

SEQ ID NO: 322 - DNA, 16 bp, synthetic construct
  source 1..16: mol_type = other DNA
  modified_base 1..16: mod_base = OTHER; note = phosphorothioate bond
  modified_base 1: mod_base = OTHER; note = 2'-O-[2-(N-methylcarbamoyl)ethyl]-5-methyluridine
  modified_base 2: mod_base = OTHER; note = modified LNA monomer with thymine base
  modified_base 3: mod_base = OTHER; note = modified LNA monomer with 5-methylcytosine base
  modified_base 4: mod_base = OTHER; note = 2'-O-[2-[N-(2-morpholinoethyl)carbamoyl]ethyl]guanosine
  modified_base 13: mod_base = m5c
  modified_base 14: mod_base = OTHER; note = modified LNA monomer with 5-methylcytosine base
  modified_base 15: mod_base = OTHER; note = modified LNA monomer with thymine base
  modified_base 16: mod_base = OTHER; note = 2'-O-[2-(N-methylcarbamoyl)ethyl]-5-methylcytidine
ttcggaaggtgacctc

SEQ ID NO: 323 - DNA, 16 bp, synthetic construct
  source 1..16: mol_type = other DNA
  modified_base 1..16: mod_base = OTHER; note = phosphorothioate bond
  modified_base 1: mod_base = OTHER; note = 2'-O-[2-(N-methylcarbamoyl)ethyl]guanosine
  modified_base 2: mod_base = OTHER; note = modified LNA monomer with guanine base
  modified_base 3: mod_base = OTHER; note = modified LNA monomer with adenine base
  modified_base 4: mod_base = OTHER; note = 2'-O-[2-[N-(2-morpholinoethyl)carbamoyl]ethyl]-5-methyluridine
  modified_base 6: mod_base = m5c
  modified_base 10: mod_base = m5c
  modified_base 14: mod_base = OTHER; note = modified LNA monomer with guanine base
  modified_base 15: mod_base = OTHER; note = modified LNA monomer with thymine base
  modified_base 16: mod_base = OTHER; note = 2'-O-[2-(N-methylcarbamoyl)ethyl]-5-methylcytidine
ggattcagtctgggtc

SEQ ID NO: 324 - DNA, 16 bp, synthetic construct
  source 1..16: mol_type = other DNA
  modified_base 1..16: mod_base = OTHER; note = phosphorothioate bond
  modified_base 1: mod_base = OTHER; note = 2'-O-[2-(N-methylcarbamoyl)ethyl]-5-methylcytidine
  modified_base 2: mod_base = OTHER; note = modified LNA monomer with guanine base
  modified_base 3: mod_base = OTHER; note = modified LNA monomer with thymine base
  modified_base 4: mod_base = OTHER; note = 2'-O-[2-[N-(2-morpholinoethyl)carbamoyl]ethyl]guanosine
  modified_base 13: mod_base = m5c
  modified_base 14: mod_base = OTHER; note = modified LNA monomer with thymine base
  modified_base 15: mod_base = OTHER; note = modified LNA monomer with guanine base
  modified_base 16: mod_base = OTHER; note = 2'-O-[2-(N-methylcarbamoyl)ethyl]-5-methylcytidine
cgtgttgaaattctgc

SEQ ID NO: 325 - DNA, 16 bp, synthetic construct
  source 1..16: mol_type = other DNA
  modified_base 1..16: mod_base = OTHER; note = phosphorothioate bond
  modified_base 1: mod_base = OTHER; note = 2'-O-[2-(N-methylcarbamoyl)ethyl]guanosine
  modified_base 2: mod_base = OTHER; note = modified LNA monomer with 5-methylcytosine base
  modified_base 3: mod_base = OTHER; note = modified LNA monomer with guanine base
  modified_base 4: mod_base = OTHER; note = 2'-O-[2-[N-(2-morpholinoethyl)carbamoyl]ethyl]-5-methyluridine
  modified_base 14: mod_base = OTHER; note = modified LNA monomer with 5-methylcytosine base
  modified_base 15: mod_base = OTHER; note = modified LNA monomer with thymine base
  modified_base 16: mod_base = OTHER; note = 2'-O-[2-(N-methylcarbamoyl)ethyl]guanosine
gcgtgttgaaattctg

SEQ ID NO: 326 - DNA, 16 bp, synthetic construct
  source 1..16: mol_type = other DNA
  modified_base 1..16: mod_base = OTHER; note = phosphorothioate bond
  modified_base 1: mod_base = OTHER; note = 2'-O-[2-(N-methylcarbamoyl)ethyl]guanosine
  modified_base 2: mod_base = OTHER; note = modified LNA monomer with adenine base
  modified_base 3: mod_base = OTHER; note = modified LNA monomer with guanine base
  modified_base 4: mod_base = OTHER; note = 2'-O-[2-[N-(2-morpholinoethyl)carbamoyl]ethyl]-5-methyluridine
  modified_base 5..6: mod_base = m5c
  modified_base 13: mod_base = m5c
  modified_base 14: mod_base = OTHER; note = modified LNA monomer with thymine base
  modified_base 15: mod_base = OTHER; note = modified LNA monomer with guanine base
  modified_base 16: mod_base = OTHER; note = 2'-O-[2-(N-methylcarbamoyl)ethyl]guanosine
gagtccttgagtctgg

SEQ ID NO: 327 - DNA, 16 bp, synthetic construct
  source 1..16: mol_type = other DNA
  modified_base 1..16: mod_base = OTHER; note = phosphorothioate bond
  modified_base 1: mod_base = OTHER; note = 2'-O-[2-(N-methylcarbamoyl)ethyl]guanosine
  modified_base 2: mod_base = OTHER; note = modified LNA monomer with guanine base
  modified_base 3: mod_base = OTHER; note = modified LNA monomer with adenine base
  modified_base 4: mod_base = OTHER; note = 2'-O-[2-[N-(2-morpholinoethyl)carbamoyl]ethyl]guanosine
  modified_base 6..7: mod_base = m5c
  modified_base 14: mod_base = OTHER; note = modified LNA monomer with 5-methylcytosine base
  modified_base 15: mod_base = OTHER; note = modified LNA monomer with thymine base
  modified_base 16: mod_base = OTHER; note = 2'-O-[2-(N-methylcarbamoyl)ethyl]guanosine
ggagtccttgagtctg

SEQ ID NO: 328 - DNA, 16 bp, synthetic construct
  source 1..16: mol_type = other DNA
  modified_base 1..16: mod_base = OTHER; note = phosphorothioate bond
  modified_base 1: mod_base = OTHER; note = 2'-O-[2-(N-methylcarbamoyl)ethyl]-5-methyluridine
  modified_base 2..3: mod_base = OTHER; note = modified LNA monomer with guanine base
  modified_base 4: mod_base = OTHER; note = 2'-O-[2-[N-(2-morpholinoethyl)carbamoyl]ethyl]guanosine
  modified_base 8..9: mod_base = m5c
  modified_base 14: mod_base = OTHER; note = modified LNA monomer with guanine base
  modified_base 15: mod_base = OTHER; note = modified LNA monomer with thymine base
  modified_base 16: mod_base = OTHER; note = 2'-O-[2-(N-methylcarbamoyl)ethyl]-5-methylcytidine
tgggagtccttgagtc

SEQ ID NO: 329 - DNA, 16 bp, synthetic construct
  source 1..16: mol_type = other DNA
  modified_base 1..16: mod_base = OTHER; note = phosphorothioate bond
  modified_base 1: mod_base = OTHER; note = 2'-O-[2-(N-methylcarbamoyl)ethyl]guanosine
  modified_base 2..3: mod_base = OTHER; note = modified LNA monomer with thymine base
  modified_base 4: mod_base = OTHER; note = 2'-O-[2-[N-(2-morpholinoethyl)carbamoyl]ethyl]-5-methylcytidine
  modified_base 7: mod_base = m5c
  modified_base 14: mod_base = OTHER; note = modified LNA monomer with adenine base
  modified_base 15: mod_base = OTHER; note = modified LNA monomer with guanine base
  modified_base 16: mod_base = OTHER; note = 2'-O-[2-(N-methylcarbamoyl)ethyl]guanosine
gttcagcttgggtagg

SEQ ID NO: 330 - DNA, 16 bp, synthetic construct
  source 1..16: mol_type = other DNA
  modified_base 1..16: mod_base = OTHER; note = phosphorothioate bond
  modified_base 1: mod_base = OTHER; note = 2'-O-[2-(N-methylcarbamoyl)ethyl]-5-methylcytidine
  modified_base 2: mod_base = OTHER; note = modified LNA monomer with 5-methylcytosine base
  modified_base 3: mod_base = OTHER; note = modified LNA monomer with guanine base
  modified_base 4: mod_base = OTHER; note = 2'-O-[2-[N-(2-morpholinoethyl)carbamoyl]ethyl]-5-methyluridine
  modified_base 14: mod_base = OTHER; note = modified LNA monomer with guanine base
  modified_base 15: mod_base = OTHER; note = modified LNA monomer with thymine base
  modified_base 16: mod_base = OTHER; note = 2'-O-[2-(N-methylcarbamoyl)ethyl]-5-methylcytidine
ccgtgtagaagaggtc

SEQ ID NO: 331 - DNA, 16 bp, synthetic construct
  source 1..16: mol_type = other DNA
  modified_base 1..16: mod_base = OTHER; note = phosphorothioate bond
  modified_base 1: mod_base = OTHER; note = 2'-O-[2-(N-methylcarbamoyl)ethyl]guanosine
  modified_base 2: mod_base = OTHER; note = modified LNA monomer with 5-methylcytosine base
  modified_base 3: mod_base = OTHER; note = modified LNA monomer with adenine base
  modified_base 4: mod_base = OTHER; note = 2'-O-[2-[N-(2-morpholinoethyl)carbamoyl]ethyl]-5-methyluridine
  modified_base 12: mod_base = m5c
  modified_base 14: mod_base = OTHER; note = modified LNA monomer with 5-methylcytosine base
  modified_base 15: mod_base = OTHER; note = modified LNA monomer with adenine base
  modified_base 16: mod_base = OTHER; note = 2'-O-[2-(N-methylcarbamoyl)ethyl]-5-methyluridine
gcataagaaagctcat

SEQ ID NO: 332 - DNA, 16 bp, synthetic construct
  source 1..16: mol_type = other DNA
  modified_base 1..16: mod_base = OTHER; note = phosphorothioate bond
  modified_base 1: mod_base = OTHER; note = 2'-O-[2-(N-methylcarbamoyl)ethyl]guanosine
  modified_base 2: mod_base = OTHER; note = modified LNA monomer with guanine base
  modified_base 3: mod_base = OTHER; note = modified LNA monomer with 5-methylcytosine base
  modified_base 4: mod_base = OTHER; note = 2'-O-[2-[N-(2-morpholinoethyl)carbamoyl]ethyl]adenosine
  modified_base 13: mod_base = m5c
  modified_base 14: mod_base = OTHER; note = modified LNA monomer with thymine base
  modified_base 15: mod_base = OTHER; note = modified LNA monomer with 5-methylcytosine base
  modified_base 16: mod_base = OTHER; note = 2'-O-[2-(N-methylcarbamoyl)ethyl]adenosine
ggcataagaaagctca

SEQ ID NO: 333 - DNA, 16 bp, synthetic construct
  source 1..16: mol_type = other DNA
  modified_base 1..16: mod_base = OTHER; note = phosphorothioate bond
  modified_base 1: mod_base = OTHER; note = 2'-O-[2-(N-methylcarbamoyl)ethyl]-5-methylcytidine
  modified_base 2..3: mod_base = OTHER; note = modified LNA monomer with guanine base
  modified_base 4: mod_base = OTHER; note = 2'-O-[2-[N-(2-morpholinoethyl)carbamoyl]ethyl]adenosine
  modified_base 11..12: mod_base = m5c
  modified_base 14: mod_base = OTHER; note = modified LNA monomer with 5-methylcytosine base
  modified_base 15: mod_base = OTHER; note = modified LNA monomer with adenine base
  modified_base 16: mod_base = OTHER; note = 2'-O-[2-(N-methylcarbamoyl)ethyl]-5-methyluridine
cggaaggtgacctcat

SEQ ID NO: 334 - DNA, 16 bp, synthetic construct
  source 1..16: mol_type = other DNA
  modified_base 1..16: mod_base = OTHER; note = phosphorothioate bond
  modified_base 1: mod_base = OTHER; note = 2'-O-[2-(N-methylcarbamoyl)ethyl]-5-methyluridine
  modified_base 2: mod_base = OTHER; note = modified LNA monomer with guanine base
  modified_base 3: mod_base = OTHER; note = modified LNA monomer with 5-methylcytosine base
  modified_base 4: mod_base = OTHER; note = 2'-O-[2-[N-(2-morpholinoethyl)carbamoyl]ethyl]-5-methyluridine
  modified_base 11: mod_base = m5c
  modified_base 13: mod_base = m5c
  modified_base 14..15: mod_base = OTHER; note = modified LNA monomer with 5-methylcytosine base
  modified_base 16: mod_base = OTHER; note = 2'-O-[2-(N-methylcarbamoyl)ethyl]-5-methylcytidine
tgcttggtgacacccc

SEQ ID NO: 335 - DNA, 16 bp, synthetic construct
  source 1..16: mol_type = other DNA
  modified_base 1..16: mod_base = OTHER; note = phosphorothioate bond
  modified_base 1: mod_base = OTHER; note = 2'-O-[2-(N-methylcarbamoyl)ethyl]guanosine
  modified_base 2: mod_base = OTHER; note = modified LNA monomer with thymine base
  modified_base 3: mod_base = OTHER; note = modified LNA monomer with guanine base
  modified_base 4..5: mod_base = OTHER; note = 2'-O-[2-[N-(2-morpholinoethyl)carbamoyl]ethyl]-5-methyluridine
  modified_base 12: mod_base = m5c
  modified_base 14: mod_base = OTHER; note = modified LNA monomer with guanine base
  modified_base 15: mod_base = OTHER; note = modified LNA monomer with 5-methylcytosine base
  modified_base 16: mod_base = OTHER; note = 2'-O-[2-(N-methylcarbamoyl)ethyl]adenosine
gtgttgaaattctgca

SEQ ID NO: 336 - DNA, 16 bp, synthetic construct
  source 1..16: mol_type = other DNA
  modified_base 1..16: mod_base = OTHER; note = phosphorothioate bond
  modified_base 1: mod_base = OTHER; note = 2'-O-[2-(N-methylcarbamoyl)ethyl]guanosine
  modified_base 2..3: mod_base = OTHER; note = modified LNA monomer with guanine base
  modified_base 4: mod_base = OTHER; note = 2'-O-[2-[N-(2-morpholinoethyl)carbamoyl]ethyl]adenosine
  modified_base 5: mod_base = OTHER; note = 2'-O-[2-[N-(2-morpholinoethyl)carbamoyl]ethyl]guanosine
  modified_base 7..8: mod_base = m5c
  modified_base 14: mod_base = OTHER; note = modified LNA monomer with thymine base
  modified_base 15: mod_base = OTHER; note = modified LNA monomer with 5-methylcytosine base
  modified_base 16: mod_base = OTHER; note = 2'-O-[2-(N-methylcarbamoyl)ethyl]-5-methyluridine
gggagtccttgagtct

SEQ ID NO: 337 - DNA, 16 bp, synthetic construct
  source 1..16: mol_type = other DNA
  modified_base 1..16: mod_base = OTHER; note = phosphorothioate bond
  modified_base 1: mod_base = OTHER; note = 2'-O-[2-(N-methylcarbamoyl)ethyl]-5-methyluridine
  modified_base 2: mod_base = OTHER; note = modified LNA monomer with thymine base
  modified_base 3: mod_base = OTHER; note = modified LNA monomer with 5-methylcytosine base
  modified_base 4..5: mod_base = OTHER; note = 2'-O-[2-[N-(2-morpholinoethyl)carbamoyl]ethyl]guanosine
  modified_base 13: mod_base = m5c
  modified_base 14: mod_base = OTHER; note = modified LNA monomer with 5-methylcytosine base
  modified_base 15: mod_base = OTHER; note = modified LNA monomer with thymine base
  modified_base 16: mod_base = OTHER; note = 2'-O-[2-(N-methylcarbamoyl)ethyl]-5-methylcytidine
ttcggaaggtgacctc

SEQ ID NO: 338 - DNA, 16 bp, synthetic construct
  source 1..16: mol_type = other DNA
  modified_base 1..16: mod_base = OTHER; note = phosphorothioate bond
  modified_base 1: mod_base = OTHER; note = 2'-O-[2-(N-methylcarbamoyl)ethyl]guanosine
  modified_base 2: mod_base = OTHER; note = modified LNA monomer with guanine base
  modified_base 3: mod_base = OTHER; note = modified LNA monomer with adenine base
  modified_base 4..5: mod_base = OTHER; note = 2'-O-[2-[N-(2-morpholinoethyl)carbamoyl]ethyl]-5-methyluridine
  modified_base 6: mod_base = m5c
  modified_base 10: mod_base = m5c
  modified_base 14: mod_base = OTHER; note = modified LNA monomer with guanine base
  modified_base 15: mod_base = OTHER; note = modified LNA monomer with thymine base
  modified_base 16: mod_base = OTHER; note = 2'-O-[2-(N-methylcarbamoyl)ethyl]-5-methylcytidine
ggattcagtctgggtc

SEQ ID NO: 339 - DNA, 16 bp, synthetic construct
  source 1..16: mol_type = other DNA
  modified_base 1..16: mod_base = OTHER; note = phosphorothioate bond
  modified_base 1: mod_base = OTHER; note = 2'-O-[2-(N-methylcarbamoyl)ethyl]-5-methylcytidine
  modified_base 2: mod_base = OTHER; note = modified LNA monomer with guanine base
  modified_base 3: mod_base = OTHER; note = modified LNA monomer with thymine base
  modified_base 4: mod_base = OTHER; note = 2'-O-[2-[N-(2-morpholinoethyl)carbamoyl]ethyl]guanosine
  modified_base 5: mod_base = OTHER; note = 2'-O-[2-[N-(2-morpholinoethyl)carbamoyl]ethyl]-5-methyluridine
  modified_base 13: mod_base = m5c
  modified_base 14: mod_base = OTHER; note = modified LNA monomer with thymine base
  modified_base 15: mod_base = OTHER; note = modified LNA monomer with guanine base
  modified_base 16: mod_base = OTHER; note = 2'-O-[2-(N-methylcarbamoyl)ethyl]-5-methylcytidine
cgtgttgaaattctgc

SEQ ID NO: 340 - DNA, 16 bp, synthetic construct
  source 1..16: mol_type = other DNA
  modified_base 1..16: mod_base = OTHER; note = phosphorothioate bond
  modified_base 1: mod_base = OTHER; note = 2'-O-[2-(N-methylcarbamoyl)ethyl]guanosine
  modified_base 2: mod_base = OTHER; note = modified LNA monomer with 5-methylcytosine base
  modified_base 3: mod_base = OTHER; note = modified LNA monomer with guanine base
  modified_base 4: mod_base = OTHER; note = 2'-O-[2-[N-(2-morpholinoethyl)carbamoyl]ethyl]-5-methyluridine
  modified_base 5: mod_base = OTHER; note = 2'-O-[2-[N-(2-morpholinoethyl)carbamoyl]ethyl]guanosine
  modified_base 14: mod_base = OTHER; note = modified LNA monomer with 5-methylcytosine base
  modified_base 15: mod_base = OTHER; note = modified LNA monomer with thymine base
  modified_base 16: mod_base = OTHER; note = 2'-O-[2-(N-methylcarbamoyl)ethyl]guanosine
gcgtgttgaaattctg

SEQ ID NO: 341 - DNA, 16 bp, synthetic construct
  source 1..16: mol_type = other DNA
  modified_base 1..16: mod_base = OTHER; note = phosphorothioate bond
  modified_base 1: mod_base = OTHER; note = 2'-O-[2-(N-methylcarbamoyl)ethyl]guanosine
  modified_base 2: mod_base = OTHER; note = modified LNA monomer with adenine base
  modified_base 3: mod_base = OTHER; note = modified LNA monomer with guanine base
  modified_base 4: mod_base = OTHER; note = 2'-O-[2-[N-(2-morpholinoethyl)carbamoyl]ethyl]-5-methyluridine
  modified_base 5: mod_base = OTHER; note = 2'-O-[2-[N-(2-morpholinoethyl)carbamoyl]ethyl]-5-methylcytidine
  modified_base 6: mod_base = m5c
  modified_base 13: mod_base = m5c
  modified_base 14: mod_base = OTHER; note = modified LNA monomer with thymine base
  modified_base 15: mod_base = OTHER; note = modified LNA monomer with guanine base
  modified_base 16: mod_base = OTHER; note = 2'-O-[2-(N-methylcarbamoyl)ethyl]guanosine
gagtccttgagtctgg

SEQ ID NO: 342 - DNA, 16 bp, synthetic construct
  source 1..16: mol_type = other DNA
  modified_base 1..16: mod_base = OTHER; note = phosphorothioate bond
  modified_base 1: mod_base = OTHER; note = 2'-O-[2-(N-methylcarbamoyl)ethyl]guanosine
  modified_base 2: mod_base = OTHER; note = modified LNA monomer with guanine base
  modified_base 3: mod_base = OTHER; note = modified LNA monomer with adenine base
  modified_base 4: mod_base = OTHER; note = 2'-O-[2-[N-(2-morpholinoethyl)carbamoyl]ethyl]guanosine
  modified_base 5: mod_base = OTHER; note = 2'-O-[2-[N-(2-morpholinoethyl)carbamoyl]ethyl]-5-methyluridine
  modified_base 6..7: mod_base = m5c
  modified_base 14: mod_base = OTHER; note = modified LNA monomer with 5-methylcytosine base
  modified_base 15: mod_base = OTHER; note = modified LNA monomer with thymine base
  modified_base 16: mod_base = OTHER; note = 2'-O-[2-(N-methylcarbamoyl)ethyl]guanosine
ggagtccttgagtctg

SEQ ID NO: 343 - DNA, 16 bp, synthetic construct
  source 1..16: mol_type = other DNA
  modified_base 1..16: mod_base = OTHER; note = phosphorothioate bond
  modified_base 1: mod_base = OTHER; note = 2'-O-[2-(N-methylcarbamoyl)ethyl]-5-methyluridine
  modified_base 2..3: mod_base = OTHER; note = modified LNA monomer with guanine base
  modified_base 4: mod_base = OTHER; note = 2'-O-[2-[N-(2-morpholinoethyl)carbamoyl]ethyl]guanosine
  modified_base 5: mod_base = OTHER; note = 2'-O-[2-[N-(2-morpholinoethyl)carbamoyl]ethyl]adenosine
  modified_base 8..9: mod_base = m5c
  modified_base 14: mod_base = OTHER; note = modified LNA monomer with guanine base
  modified_base 15: mod_base = OTHER; note = modified LNA monomer with thymine base
  modified_base 16: mod_base = OTHER; note = 2'-O-[2-(N-methylcarbamoyl)ethyl]-5-methylcytidine
tgggagtccttgagtc

SEQ ID NO: 344 - DNA, 16 bp, synthetic construct
  source 1..16: mol_type = other DNA
  modified_base 1..16: mod_base = OTHER; note = phosphorothioate bond
  modified_base 1: mod_base = OTHER; note = 2'-O-[2-(N-methylcarbamoyl)ethyl]guanosine
  modified_base 2..3: mod_base = OTHER; note = modified LNA monomer with thymine base
  modified_base 4: mod_base = OTHER; note = 2'-O-[2-[N-(2-morpholinoethyl)carbamoyl]ethyl]-5-methylcytidine
  modified_base 5: mod_base = OTHER; note = 2'-O-[2-[N-(2-morpholinoethyl)carbamoyl]ethyl]adenosine
  modified_base 7: mod_base = m5c
  modified_base 14: mod_base = OTHER; note = modified LNA monomer with adenine base
  modified_base 15: mod_base = OTHER; note = modified LNA monomer with guanine base
  modified_base 16: mod_base = OTHER; note = 2'-O-[2-(N-methylcarbamoyl)ethyl]guanosine
gttcagcttgggtagg

SEQ ID NO: 345 - DNA, 16 bp, synthetic construct
  source 1..16: mol_type = other DNA
  modified_base 1..16: mod_base = OTHER; note = phosphorothioate bond
  modified_base 1: mod_base = OTHER; note = 2'-O-[2-(N-methylcarbamoyl)ethyl]-5-methylcytidine
  modified_base 2: mod_base = OTHER; note = modified LNA monomer with 5-methylcytosine base
  modified_base 3: mod_base = OTHER; note = modified LNA monomer with guanine base
  modified_base 4: mod_base = OTHER; note = 2'-O-[2-[N-(2-morpholinoethyl)carbamoyl]ethyl]-5-methyluridine
  modified_base 5: mod_base = OTHER; note = 2'-O-[2-[N-(2-morpholinoethyl)carbamoyl]ethyl]guanosine
  modified_base 14: mod_base = OTHER; note = modified LNA monomer with guanine base
  modified_base 15: mod_base = OTHER; note = modified LNA monomer with thymine base
  modified_base 16: mod_base = OTHER; note = 2'-O-[2-(N-methylcarbamoyl)ethyl]-5-methylcytidine
ccgtgtagaagaggtc

SEQ ID NO: 346 - DNA, 16 bp, synthetic construct
  source 1..16: mol_type = other DNA
  modified_base 1..16: mod_base = OTHER; note = phosphorothioate bond
  modified_base 1: mod_base = OTHER; note = 2'-O-[2-(N-methylcarbamoyl)ethyl]guanosine
  modified_base 2: mod_base = OTHER; note = modified LNA monomer with 5-methylcytosine base
  modified_base 3: mod_base = OTHER; note = modified LNA monomer with adenine base
  modified_base 4: mod_base = OTHER; note = 2'-O-[2-[N-(2-morpholinoethyl)carbamoyl]ethyl]-5-methyluridine
  modified_base 5: mod_base = OTHER; note = 2'-O-[2-[N-(2-morpholinoethyl)carbamoyl]ethyl]adenosine
  modified_base 12: mod_base = m5c
  modified_base 14: mod_base = OTHER; note = modified LNA monomer with 5-methylcytosine base
  modified_base 15: mod_base = OTHER; note = modified LNA monomer with adenine base
  modified_base 16: mod_base = OTHER; note = 2'-O-[2-(N-methylcarbamoyl)ethyl]-5-methyluridine
gcataagaaagctcat

SEQ ID NO: 347 - DNA, 16 bp, synthetic construct
  source 1..16: mol_type = other DNA
  modified_base 1..16: mod_base = OTHER; note = phosphorothioate bond
  modified_base 1: mod_base = OTHER; note = 2'-O-[2-(N-methylcarbamoyl)ethyl]guanosine
  modified_base 2: mod_base = OTHER; note = modified LNA monomer with guanine base
  modified_base 3: mod_base = OTHER; note = modified LNA monomer with 5-methylcytosine base
  modified_base 4: mod_base = OTHER; note = 2'-O-[2-[N-(2-morpholinoethyl)carbamoyl]ethyl]adenosine
  modified_base 5: mod_base = OTHER; note = 2'-O-[2-[N-(2-morpholinoethyl)carbamoyl]ethyl]-5-methyluridine
  modified_base 13: mod_base = m5c
  modified_base 14: mod_base = OTHER; note = modified LNA monomer with thymine base
  modified_base 15: mod_base = OTHER; note = modified LNA monomer with 5-methylcytosine base
  modified_base 16: mod_base = OTHER; note = 2'-O-[2-(N-methylcarbamoyl)ethyl]adenosine
ggcataagaaagctca

SEQ ID NO: 348 - DNA, 16 bp, synthetic construct
  source 1..16: mol_type = other DNA
  modified_base 1..16: mod_base = OTHER; note = phosphorothioate bond
  modified_base 1: mod_base = OTHER; note = 2'-O-[2-(N-methylcarbamoyl)ethyl]-5-methylcytidine
  modified_base 2..3: mod_base = OTHER; note = modified LNA monomer with guanine base
  modified_base 4..5: mod_base = OTHER; note = 2'-O-[2-[N-(2-morpholinoethyl)carbamoyl]ethyl]adenosine
  modified_base 11..12: mod_base = m5c
  modified_base 14: mod_base = OTHER; note = modified LNA monomer with 5-methylcytosine base
  modified_base 15: mod_base = OTHER; note = modified LNA monomer with adenine base
  modified_base 16: mod_base = OTHER; note = 2'-O-[2-(N-methylcarbamoyl)ethyl]-5-methyluridine
cggaaggtgacctcat

SEQ ID NO: 349 - DNA, 16 bp, synthetic construct
  source 1..16: mol_type = other DNA
  modified_base 1..16: mod_base = OTHER; note = phosphorothioate bond
  modified_base 1: mod_base = OTHER; note = 2'-O-[2-(N-methylcarbamoyl)ethyl]-5-methyluridine
  modified_base 2: mod_base = OTHER; note = modified LNA monomer with guanine base
  modified_base 3: mod_base = OTHER; note = modified LNA monomer with 5-methylcytosine base
  modified_base 4..5: mod_base = OTHER; note = 2'-O-[2-[N-(2-morpholinoethyl)carbamoyl]ethyl]-5-methyluridine
  modified_base 11: mod_base = m5c
  modified_base 13: mod_base = m5c
  modified_base 14..15: mod_base = OTHER; note = modified LNA monomer with 5-methylcytosine base
  modified_base 16: mod_base = OTHER; note = 2'-O-[2-(N-methylcarbamoyl)ethyl]-5-methylcytidine
tgcttggtgacacccc

SEQ ID NO: 350 - DNA, 16 bp, synthetic construct
  source 1..16: mol_type = other DNA
  modified_base 1..16: mod_base = OTHER; note = phosphorothioate bond
  modified_base 1: mod_base = OTHER; note = 2'-O-[2-(N-methylcarbamoyl)ethyl]guanosine
  modified_base 2: mod_base = OTHER; note = modified LNA monomer with guanine base
  modified_base 3: mod_base = OTHER; note = modified LNA monomer with 5-methylcytosine base
  modified_base 4: mod_base = m5c
  modified_base 6: mod_base = m5c
  modified_base 9: mod_base = m5c
  modified_base 13: mod_base = m5c
  modified_base 14: mod_base = OTHER; note = modified LNA monomer with adenine base
  modified_base 15: mod_base = OTHER; note = modified LNA monomer with thymine base
  modified_base 16: mod_base = OTHER; note = 2'-O-[2-(N-methylcarbamoyl)ethyl]-5-methyluridine
  modified_base 1: mod_base = OTHER; note = bonded to 6-[N-(hexadecanoyl)amino]hexyl group via phosphodiester bond
ggcctcttcttacatt

SEQ ID NO: 351 - DNA, 16 bp, synthetic construct
  source 1..16: mol_type = other DNA
  modified_base 1..16: mod_base = OTHER; note = phosphorothioate bond
  modified_base 1: mod_base = OTHER; note = modified LNA monomer with thymine base
  modified_base 2: mod_base = OTHER; note = modified LNA monomer with guanine base
  modified_base 3: mod_base = OTHER; note = 2'-O-[2-(N-methylcarbamoyl)ethyl]guanosine
  modified_base 4..5: mod_base = m5c
  modified_base 7: mod_base = m5c
  modified_base 13: mod_base = m5c
  modified_base 14: mod_base = OTHER; note = 2'-O-[2-(N-methylcarbamoyl)ethyl]-5-methyluridine
  modified_base 15: mod_base = OTHER; note = modified LNA monomer with 5-methylcytosine base
  modified_base 16: mod_base = OTHER; note = modified LNA monomer with adenine base
tggcctctttaactca

SEQ ID NO: 352 - DNA, 16 bp, synthetic construct
  source 1..16: mol_type = other DNA
  modified_base 1..16: mod_base = OTHER; note = phosphorothioate bond
  modified_base 1: mod_base = OTHER; note = 2'-O-[2-(N-methylcarbamoyl)ethyl]-5-methyluridine
  modified_base 2..3: mod_base = OTHER; note = modified LNA monomer with guanine base
  modified_base 4..5: mod_base = m5c
  modified_base 7: mod_base = m5c
  modified_base 13: mod_base = OTHER; note = 2'-O-[2-(N-methylcarbamoyl)ethyl]-5-methylcytidine
  modified_base 14: mod_base = OTHER; note = modified LNA monomer with thymine base
  modified_base 15: mod_base = OTHER; note = modified LNA monomer with 5-methylcytosine base
  modified_base 16: mod_base = OTHER; note = 2'-O-[2-(N-methylcarbamoyl)ethyl]adenosine
tggcctctttaactca

SEQ ID NO: 353 - DNA, 16 bp, synthetic construct
  source 1..16: mol_type = other DNA
  modified_base 1..16: mod_base = OTHER; note = phosphorothioate bond
  modified_base 1: mod_base = OTHER; note = 2'-O-[2-(N-methylcarbamoyl)ethyl]-5-methyluridine
  modified_base 2..3: mod_base = OTHER; note = modified LNA monomer with guanine base
  modified_base 4: mod_base = OTHER; note = 2'-O-[2-(N-methylcarbamoyl)ethyl]-5-methylcytidine
  modified_base 5: mod_base = m5c
  modified_base 7: mod_base = m5c
  modified_base 13: mod_base = m5c
  modified_base 14: mod_base = OTHER; note = modified LNA monomer with thymine base
  modified_base 15: mod_base = OTHER; note = modified LNA monomer with 5-methylcytosine base
  modified_base 16: mod_base = OTHER; note = 2'-O-[2-(N-methylcarbamoyl)ethyl]adenosine
tggcctctttaactca

SEQ ID NO: 354 - DNA, 16 bp, synthetic construct
  source 1..16: mol_type = other DNA
  modified_base 1..16: mod_base = OTHER; note = phosphorothioate bond
  modified_base 1: mod_base = OTHER; note = 2'-O-[2-(N-methylcarbamoyl)ethyl]-5-methyluridine
  modified_base 2..3: mod_base = OTHER; note = modified LNA monomer with guanine base
  modified_base 4..5: mod_base = OTHER; note = 2'-O-[2-(N-methylcarbamoyl)ethyl]-5-methylcytidine
  modified_base 7: mod_base = m5c
  modified_base 13: mod_base = m5c
  modified_base 14: mod_base = OTHER; note = modified LNA monomer with thymine base
  modified_base 15: mod_base = OTHER; note = modified LNA monomer with 5-methylcytosine base
  modified_base 16: mod_base = OTHER; note = 2'-O-[2-(N-methylcarbamoyl)ethyl]adenosine
tggcctctttaactca

SEQ ID NO: 355 - DNA, 16 bp, synthetic construct
  source 1..16: mol_type = other DNA
  modified_base 1..16: mod_base = OTHER; note = phosphorothioate bond
  modified_base 1: mod_base = OTHER; note = 2'-O-[2-(N-methylcarbamoyl)ethyl]-5-methyluridine
  modified_base 2..3: mod_base = OTHER; note = modified LNA monomer with guanine base
  modified_base 4: mod_base = OTHER; note = 2'-O-[2-[N-(2-morpholinoethyl)carbamoyl]ethyl]-5-methylcytidine
  modified_base 5: mod_base = m5c
  modified_base 7: mod_base = m5c
  modified_base 13: mod_base = m5c
  modified_base 14: mod_base = OTHER; note = modified LNA monomer with thymine base
  modified_base 15: mod_base = OTHER; note = modified LNA monomer with 5-methylcytosine base
  modified_base 16: mod_base = OTHER; note = 2'-O-[2-(N-methylcarbamoyl)ethyl]adenosine
tggcctctttaactca

SEQ ID NO: 356 - DNA, 16 bp, synthetic construct
  source 1..16: mol_type = other DNA
  modified_base 1..16: mod_base = OTHER; note = phosphorothioate bond
  modified_base 1: mod_base = OTHER; note = 2'-O-[2-(N-methylcarbamoyl)ethyl]-5-methyluridine
  modified_base 2..3: mod_base = OTHER; note = modified LNA monomer with guanine base
  modified_base 4..5: mod_base = OTHER; note = 2'-O-[2-[N-(2-morpholinoethyl)carbamoyl]ethyl]-5-methylcytidine
  modified_base 7: mod_base = m5c
  modified_base 13: mod_base = m5c
  modified_base 14: mod_base = OTHER; note = modified LNA monomer with thymine base
  modified_base 15: mod_base = OTHER; note = modified LNA monomer with 5-methylcytosine base
  modified_base 16: mod_base = OTHER; note = 2'-O-[2-(N-methylcarbamoyl)ethyl]adenosine
tggcctctttaactca

SEQ ID NO: 357 - DNA, 16 bp, synthetic construct
  source 1..16: mol_type = other DNA
  modified_base 1..2: mod_base = OTHER; note = phosphorothioate bond
  modified_base 4..14: mod_base = OTHER; note = phosphorothioate bond
  modified_base 15..16: mod_base = OTHER; note = phosphorothioate bond
  modified_base 1: mod_base = OTHER; note = 2'-O-[2-(N-methylcarbamoyl)ethyl]-5-methyluridine
  modified_base 2..3: mod_base = OTHER; note = modified LNA monomer with guanine base
  modified_base 4..5: mod_base = m5c
  modified_base 7: mod_base = m5c
  modified_base 13: mod_base = m5c
  modified_base 14: mod_base = OTHER; note = modified LNA monomer with thymine base
  modified_base 15: mod_base = OTHER; note = modified LNA monomer with 5-methylcytosine base
  modified_base 16: mod_base = OTHER; note = 2'-O-[2-(N-methylcarbamoyl)ethyl]adenosine
tggcctctttaactca

SEQ ID NO: 358 - DNA, 16 bp, synthetic construct
  source 1..16: mol_type = other DNA
  modified_base 1..16: mod_base = OTHER; note = phosphorothioate bond
  modified_base 1: mod_base = OTHER; note = bonded to 6-[N-(hexadecanoyl)amino]hexyl group via phosphodiester bond
  modified_base 1: mod_base = OTHER; note = 2'-O-[2-(N-methylcarbamoyl)ethyl]-5-methylcytidine
  modified_base 2: mod_base = OTHER; note = modified LNA monomer with 5-methylcytosine base
  modified_base 3: mod_base = OTHER; note = modified LNA monomer with guanine base
  modified_base 6: mod_base = m5c
  modified_base 14: mod_base = OTHER; note = modified LNA monomer with adenine base
  modified_base 15: mod_base = OTHER; note = modified LNA monomer with guanine base
  modified_base 16: mod_base = OTHER; note = 2'-O-[2-(N-methylcarbamoyl)ethyl]-5-methylcytidine
ccgggcataagaaagc

SEQ ID NO: 359 - DNA, 16 bp, synthetic construct
  source 1..16: mol_type = other DNA
  modified_base 1..16: mod_base = OTHER; note = phosphorothioate bond
  modified_base 1: mod_base = OTHER; note = bonded to 6-[N-(hexadecanoyl)amino]hexyl group via phosphodiester bond
  modified_base 1: mod_base = OTHER; note = 2'-O-[2-(N-methylcarbamoyl)ethyl]-5-methyluridine
  modified_base 2: mod_base = OTHER; note = modified LNA monomer with thymine base
  modified_base 3: mod_base = OTHER; note = modified LNA monomer with 5-methylcytosine base
  modified_base 13: mod_base = m5c
  modified_base 14: mod_base = OTHER; note = modified LNA monomer with 5-methylcytosine base
  modified_base 15: mod_base = OTHER; note = modified LNA monomer with thymine base
  modified_base 16: mod_base = OTHER; note = 2'-O-[2-(N-methylcarbamoyl)ethyl]-5-methylcytidine
ttcggaaggtgacctc

SEQ ID NO: 360 - DNA, 16 bp, synthetic construct
  source 1..16: mol_type = other DNA
  modified_base 1..16: mod_base = OTHER; note = phosphorothioate bond
  modified_base 1: mod_base = OTHER; note = bonded to 6-[N-(hexadecanoyl)amino]hexyl group via phosphodiester bond
  modified_base 1: mod_base = OTHER; note = 2'-O-[2-(N-methylcarbamoyl)ethyl]guanosine
  modified_base 2: mod_base = OTHER; note = modified LNA monomer with guanine base
  modified_base 3: mod_base = OTHER; note = modified LNA monomer with 5-methylcytosine base
  modified_base 4: mod_base = OTHER; note = 2'-O-[2-(N-methylcarbamoyl)ethyl]adenosine
  modified_base 5: mod_base = OTHER; note = 2'-O-[2-(N-methylcarbamoyl)ethyl]-5-methyluridine
  modified_base 13: mod_base = m5c
  modified_base 14: mod_base = OTHER; note = modified LNA monomer with thymine base
  modified_base 15: mod_base = OTHER; note = modified LNA monomer with 5-methylcytosine base
  modified_base 16: mod_base = OTHER; note = 2'-O-[2-(N-methylcarbamoyl)ethyl]adenosine
ggcataagaaagctca

SEQ ID NO: 361 - DNA, 16 bp, synthetic construct
  source 1..16: mol_type = other DNA
  modified_base 1..2: mod_base = OTHER; note = phosphorothioate bond
  modified_base 4..14: mod_base = OTHER; note = phosphorothioate bond
  modified_base 15..16: mod_base = OTHER; note = phosphorothioate bond
  modified_base 1: mod_base = OTHER; note = bonded to 6-[N-(hexadecanoyl)amino]hexyl group via phosphodiester bond
  modified_base 1: mod_base = OTHER; note = 2'-O-[2-(N-methylcarbamoyl)ethyl]guanosine
  modified_base 2: mod_base = OTHER; note = modified LNA monomer with guanine base
  modified_base 3: mod_base = OTHER; note = modified LNA monomer with 5-methylcytosine base
  modified_base 13: mod_base = m5c
  modified_base 14: mod_base = OTHER; note = modified LNA monomer with thymine base
  modified_base 15: mod_base = OTHER; note = modified LNA monomer with 5-methylcytosine base
  modified_base 16: mod_base = OTHER; note = 2'-O-[2-(N-methylcarbamoyl)ethyl]adenosine
ggcataagaaagctca

SEQ ID NO: 362 - DNA, 16 bp, synthetic construct
  source 1..16: mol_type = other DNA
  modified_base 1..16: mod_base = OTHER; note = phosphorothioate bond
  modified_base 1: mod_base = OTHER; note = bonded to 6-[N-(hexadecanoyl)amino]hexyl group via phosphodiester bond
  modified_base 1: mod_base = OTHER; note = 2'-O-[2-(N-methylcarbamoyl)ethyl]guanosine
  modified_base 2: mod_base = OTHER; note = modified LNA monomer with guanine base
  modified_base 3: mod_base = OTHER; note = modified LNA monomer with 5-methylcytosine base
  modified_base 4: mod_base = OTHER; note = 2'-O-[2-[N-(2-morpholinoethyl)carbamoyl]ethyl]adenosine
  modified_base 13: mod_base = m5c
  modified_base 14: mod_base = OTHER; note = modified LNA monomer with thymine base
  modified_base 15: mod_base = OTHER; note = modified LNA monomer with 5-methylcytosine base
  modified_base 16: mod_base = OTHER; note = 2'-O-[2-(N-methylcarbamoyl)ethyl]adenosine
ggcataagaaagctca

SEQ ID NO: 363 - DNA, 16 bp, synthetic construct
  source 1..16: mol_type = other DNA
  modified_base 1..16: mod_base = OTHER; note = phosphorothioate bond
  modified_base 1: mod_base = OTHER; note = bonded to 6-[N-(hexadecanoyl)amino]hexyl group via phosphodiester bond
  modified_base 1: mod_base = OTHER; note = 2'-O-[2-(N-methylcarbamoyl)ethyl]guanosine
  modified_base 2: mod_base = OTHER; note = modified LNA monomer with guanine base
  modified_base 3: mod_base = OTHER; note = modified LNA monomer with 5-methylcytosine base
  modified_base 6: mod_base = m5c
  modified_base 9: mod_base = m5c
  modified_base 11..12: mod_base = m5c
  modified_base 14: mod_base = OTHER; note = modified LNA monomer with thymine base
  modified_base 15: mod_base = OTHER; note = modified LNA monomer with 5-methylcytosine base
  modified_base 16: mod_base = OTHER; note = 2'-O-[2-(N-methylcarbamoyl)ethyl]adenosine
ggctactacgccgtca